European Patent Specification EP 3 802 807 B1, published November 20, 2024. Title: RNA-GUIDED NUCLEASES AND ACTIVE FRAGMENTS AND VARIANTS THEREOF AND METHODS OF USE. Applicant: LIFEEDIT, INC. The sequence listing filed with the application follows.

SEQUENCE LISTING (651 sequences)

SEQ ID NO: 1 - protein, 1070 aa, Bacillus sp.
  source: /note="APG05083.1"
MRELDYRIGLDIGTNSIGWGIIELSWNKDREQYEKARIVDKGVRMFDKAEIPKTGASLAEPRRIARSSRRRLNRKSQRKKDIRNLLVQHEIISQKELASLYPLTKSSMDIWDIRLDGLDRLLDRFEWTRLLIHLAQRRGFKSNRKSELKDVETGKVLSSIQANEKRLSLYRTVGEMWMKNEDFSKYDKRRNSSNEYVFSVSRADLEKEIVTLFEAQRKFQSSYASADLQKTYLQIWAHQLPFASGNAIVNKVGYCSLLKGKEKRVPKATYTFQYFSTLDQINRTRLGPNFQPFTKEQRDVILDEMFNRTDYYKKKTIPEVTYYDIRKWLALDETIQFKGLTYDPNEELKKIELKSFINLKPFYEIKKVVTNYAKKTNEAFSTLDYDTFAYALTVYKTDKDIRSYLKKSNNLSKCCYDDQLIEELLTLSYTKFGHLSFKAINHVLPIMQEGRTYQEAIHQLGYDATNLKKENRSMFLPLFPDEITNPIVKRALTQARKVVNAIIRRYGSPNSVHIELARELSKSHDERTKIMKAHDENYKKNKGAISILIENGILNPTGYDIVRYKLWKEQGERCAYSLKQIPANTFFNEMKKERSGSPVLEIDHILPYSQSFIDSYHNKVLVYGDENQKKGNRIPYTYFLEGNKDWESFESYVRLNSFFSKKKRGYLLKKAYLPRESNMIKERHLNDTRYASSYLKNFIEKNLKFKEVEGSTRKKHVQTVNGIITAHLRKRWGLEKDRQETYLHHAMDAIIVACTDHHMVTKVTEYYQIKESNKSIRKPYFPLPWVGFREEILSHLARQPIARKISEELKIGYQSFDYILVSRMPKRSVTGAAHEQTIMKKGGIDKKGKTIIIKRVYLKDIKFDENGDFKMVGKEQDLATYEAIKQRYIEYGKESKKAFETPLYKPSKKGKGNLIKKIKVEVQTKSFVREVNGGVAQNGDLVRVDLFEKDNRYYMIPIYVMDTVHSELPNKAVTSSKGYEQWLTIDNSFTFKFSLYPYDLVRLVKGNEDRFLYFSTLDINSDRLNFKDVNKPSKQAENRYSLKTIENLEKYEVGVLGDLRFVRQEIRKNF

SEQ ID NO: 2 - RNA, 19 nt, Bacillus sp.
  source: /note="crRNA"
gucauaguuccauuauugc

SEQ ID NO: 3 - RNA, 84 nt, Bacillus sp.
  source: /note="tracrRNA"
gcuuugauguuucuaugauaagggcuuaggcccguggcguuggggaucgccugcccauuuuaaugggcuucuccccaucuauuu

SEQ ID NO: 4 - RNA, 137 nt, Artificial Sequence
  source: /note="Description of Artificial Sequence: Synthetic polynucleotide"
  source: /note="sgRNA L1"
gagcggacagcagcuuccuauaucucguacgucauaguuccauuauugcaaaggcuuugauguuucuaugauaagggcuuaggcccguggcguuggggaucgccugcccauuuuaaugggcuucuccccaucuauuu

SEQ ID NO: 5 - RNA, 137 nt, Artificial Sequence
  source: /note="Description of Artificial Sequence: Synthetic polynucleotide"
  source: /note="sgRNA L2"
ccaugauauagacguuguggcuguuguagugucauaguuccauuauugcaaaggcuuugauguuucuaugauaagggcuuaggcccguggcguuggggaucgccugcccauuuuaaugggcuucuccccaucuauuu

SEQ ID NO: 6 - DNA, 6 bp, Artificial Sequence
  source: /note="Description of Artificial Sequence: Synthetic oligonucleotide"
  source: /note="PAM"
  modified_base (1)..(4): a, c, t, g, unknown or other
nnnncc

SEQ ID NO: 7 - DNA, 6 bp, Artificial Sequence
  source: /note="Description of Artificial Sequence: Synthetic oligonucleotide"
  source: /note="PAM examplary"
  modified_base (1)..(2): a, c, t, g, unknown or other
  modified_base (4)..(4): a, c, t, g, unknown or other
nnrncc

SEQ ID NO: 8 - DNA, 38 bp, Artificial Sequence
  source: /note="Description of Artificial Sequence: Synthetic oligonucleotide"
  source: /note="Target seq and PAM region of plasmid library 1"
  modified_base (31)..(38): a, c, t, g, unknown or other
gagcggacagcagcttcctatatctcgtacnnnnnnnn

SEQ ID NO: 9 - DNA, 38 bp, Artificial Sequence
  source: /note="Description of Artificial Sequence: Synthetic oligonucleotide"
  source: /note="Target seq and PAM region of plasmid library 2"
  modified_base (31)..(38): a, c, t, g, unknown or other
ccatgatatagacgttgtggctgttgtagtnnnnnnnn

SEQ ID NO: 10 - RNA, 132 nt, Artificial Sequence
  source: /note="Description of Artificial Sequence: Synthetic polynucleotide"
  source: /note="sgRNA with N's"
  modified_base (1)..(25): a, c, u, g, unknown or other
nnnnnnnnnnnnnnnnnnnnnnnnngucauaguuccauuauugcaaaggcuuugauguuucuaugauaagggcuuaggcccguggcguuggggaucgccugcccauuuuaaugggcuucuccccaucuauuu

SEQ ID NO: 11 - protein, 1071 aa, Bacillus sp.
  source: /note="APG07433.1"
MRELDYRIGLDIGTNSIGWGVIELSWNKDRERYEKVRIVDQGVRMFDRAEMPKTGASLAEPRRIARSSRRRLNRKSQRKKNIRNLLVQHGVITQEELDSLYPLSKKSMDIWGIRLDGLDRLLNHFEWARLLIHLAQRRGFKSNRKSELKDTETGKVLSSIQLNEKRLSLYRTVGEMWMKDPDFSKYDRKRNSPNEYVFSVSRAELEKEIVTLFAAQRRFQSPYASKDLQETYLQIWTHQLPFASGNAILNKVGYCSLLKGKERRIPKATYTFQYFSALDQVNRTRLGPDFQPFTKEQREIILNNMFQRTDYYKKKTIPEVTYYDIRKWLELDETIQFKGLNYDPNEELKKIEKKPFINLKAFYEINKVVANYSERTNETFSTLDYDGIGYALTVYKTDKDIRSYLKSSHNLPKRCYDDQLIEELLSLSYTKFGHLSLKAINHVLSIMQKGNTYKEAVDQLGYDTSGLKKEKRSKFLPPISDEITNPIVKRALTQARKVVNAIIRRHGSPHSVHIELARELSKNHDERTKIVSAQDENYKKNKGAISILSEHGILNPTGYDIVRYKLWKEQGERCAYSLKEIPADTFFNELKKERNGAPILEVDHILPYSQSFIDSYHNKVLVYSDENRKKGNRIPYTYFLETNKDWEAFERYVRSNKFFSKKKREYLLKRAYLPRESELIKERHLNDTRYASTFLKNFIEQNLQFKEAEDNPRKRRVQTVNGVITAHFRKRWGLEKDRQETYLHHAMDAIIVACTDHHMVTRVTEYYQIKESNKSVKKPYFPMPWEGFRDELLSHLASQPIAKKISEELKAGYQSLDYIFVSRMPKRSITGAAHKQTIMRKGGIDKKGKTIIIERLHLKDIKFDENGDFKMVGKEQDMATYEAIKQRYLEHGKNSKKAFETPLYKPSKKGTGNLIKRVKVEGQAKSFVREVNGGVAQNGDLVRVDLFEKDDKYYMVPIYVPDTVCSELPKKVVASSKGYEQWLTLDNSFTFKFSLYPYDLVRLVKGDEDRFLYFGTLDIDSDRLNFKDVNKPSKKNEYRYSLKTIEDLEKYEVGVLGDLRLVRKETRRNFH

SEQ ID NO: 12 - RNA, 21 nt, Bacillus sp.
  source: /note="crRNA"
gucauaguuccauuaaagcca

SEQ ID NO: 13 - RNA, 85 nt, Bacillus sp.
  source: /note="tracrRNA"
uggcuuugauguuucuaugauaaggguuucgacccguggcgucggggaucgccugcccauugaaaugggcuucuccccauuuauu

SEQ ID NO: 14 - RNA, 140 nt, Artificial Sequence
  source: /note="Description of Artificial Sequence: Synthetic polynucleotide"
  source: /note="sgRNA L1"
gagcggacagcagcuuccuauaucucguacgucauaguuccauuaaagccagaaauggcuuugauguuucuaugauaaggguuucgacccguggcgucggggaucgccugcccauugaaaugggcuucuccccauuuauu

SEQ ID NO: 15 - RNA, 140 nt, Artificial Sequence
  source: /note="Description of Artificial Sequence: Synthetic polynucleotide"
  source: /note="sgRNA L2"
ccaugauauagacguuguggcuguuguagugucauaguuccauuaaagccagaaauggcuuugauguuucuaugauaaggguuucgacccguggcgucggggaucgccugcccauugaaaugggcuucuccccauuuauu

SEQ ID NO: 16 - DNA, 38 bp, Artificial Sequence; identical to SEQ ID NO: 8
  source: /note="Description of Artificial Sequence: Synthetic oligonucleotide"
  source: /note="Target seq and PAM region of plasmid library 1"
  modified_base (31)..(38): a, c, t, g, unknown or other

SEQ ID NO: 17 - DNA, 38 bp, Artificial Sequence; identical to SEQ ID NO: 9
  source: /note="Description of Artificial Sequence: Synthetic oligonucleotide"
  source: /note="Target seq and PAM region of plasmid library 2"
  modified_base (31)..(38): a, c, t, g, unknown or other

SEQ ID NO: 18 - RNA, 135 nt, Artificial Sequence
  source: /note="Description of Artificial Sequence: Synthetic polynucleotide"
  source: /note="sgRNA with N's"
  modified_base (1)..(25): a, c, u, g, unknown or other
nnnnnnnnnnnnnnnnnnnnnnnnngucauaguuccauuaaagccaaaaguggcuuugauguuucuaugauaaggguuucgacccguggcgucggggaucgccugcccauugaaaugggcuucuccccauuuauu

SEQ ID NO: 19 - protein, 1071 aa, Bacillus sp.
  source: /note="APG07513.1"
MRELDYRIGLDIGTNSIGWGVIELSWNKDREQYEKTRIVDKGVRMFDKAEIPKTGASLAEPRRIARSSRRRLNRKSQRKKDIRNLLVQHEIISQKELTSLYPLSKSSMDIWDIRLDGLDRLLDRFEWARLLIHLAQRRGFKSNRKSELKDVETGKVLSSIQVNEKRLSLYRTVGEMWMKNADCSKYGKRRNSPNEYVFSVSRADLEKEIVTLFEAQRKFHSSYASVDLQKTYIQIWAHQLPFASGNAIVNKVGYCSLLKGKEKRVPKATYTFQYFNTLDQINRTRLGPNFQPFTKEQRDIILDKMFQRTDYYKKKTIPEVTYYDIRKWLALDETIQFKGLTYDPNEELKKIEMKPFINLKPFYEIKKVVTNYAKKTNEVFSALDYDTVAYALTVYKTDKDIRSYLKRSNNLSKRCYDDQLIEELLTLSYTKFGHLSFKAINHVLPIMQEGRTYQEAIHQLGYDTTNLKKENRSMFLPIIPDEITNPIVKRALTQARKVVNAIIRRYGSPNSVHIELARELSKSHDERKKIMTAHDENYKKNKGAVSILIDNGILNPTGYDIVRYKLWKEQGERCAYSLKKIPANTFFNELKKERSGPPVLEVDHILPYSQSFIDSYHNKVLVYGDENQKKGNRIPYTFFSEEDKEWESFESYVRSNSFFSKKKRGYLLKKAYLPRESNLIKERHLNDTRYASSYLKNFIEKNLKFKEAVGITRKKYVQTVNGVITAHLRKRWGLEKDRQETYLHHAMDAIIVACTDHHMVTKVTEYYQIKEGNKSIKKPYFPLPWMGFREEILSHLESQPIARKISEELKIGYQSPDYILVSRMPKRSVTGSAHDQTVMKKGDIDKKGKTIIIKRVHLKDIKFDENGDFKMVGKEQDLATYEAIKQRYLEYRKESKKAFETPLYKPSKKGKGNLIKKIKVEVQTKSFVREINGGVAQNGDLVRVDLFEKDNRYYMVPIYVVDTVRSELPNKAVTSSKGYEQWLSIDNSFTFKFSLYPYDLVRLVKGDEDRFLYFSTLDINSDRLNFKDVNKPSKQAEYRYSLKTIENLEKYEIGVLGDLRLVRQETRKIFK

SEQ ID NO: 20 - RNA, 27 nt, Bacillus sp.
  source: /note="crRNA"
gucauaguuccauuaaagccauugcug

SEQ ID NO: 21 - RNA, 93 nt, Bacillus sp.
  source: /note="tracrRNA"
acagcaauggcuuugauguuucuaugauaagggcuucggcccguggcguuggggaucgccugcccauuuuaaugggcuucuccccaucuauuu

SEQ ID NO: 22 - RNA, 154 nt, Artificial Sequence
  source: /note="Description of Artificial Sequence: Synthetic polynucleotide"
  source: /note="sgRNA L1"
gagcggacagcagcuuccuauaucucguacgucauaguuccauuaaagccauugcugaaagacagcaauggcuuugauguuucuaugauaagggcuucggcccguggcguuggggaucgccugcccauuuuaaugggcuucuccccaucuauuu

SEQ ID NO: 23 - RNA, 154 nt, Artificial Sequence
  source: /note="Description of Artificial Sequence: Synthetic polynucleotide"
  source: /note="sgRNA L2"
ccaugauauagacguuguggcuguuguagugucauaguuccauuaaagccauugcugaaagacagcaauggcuuugauguuucuaugauaagggcuucggcccguggcguuggggaucgccugcccauuuuaaugggcuucuccccaucuauuu

SEQ ID NO: 24 - DNA, 38 bp, Artificial Sequence; identical to SEQ ID NO: 8
  source: /note="Description of Artificial Sequence: Synthetic oligonucleotide"
  source: /note="Target seq and PAM region of plasmid library 1"
  modified_base (31)..(38): a, c, t, g, unknown or other

SEQ ID NO: 25 - DNA, 38 bp, Artificial Sequence; identical to SEQ ID NO: 9
  source: /note="Description of Artificial Sequence: Synthetic oligonucleotide"
  source: /note="Target seq and PAM region of plasmid library 2"
  modified_base (31)..(38): a, c, t, g, unknown or other

SEQ ID NO: 26 - RNA, 149 nt, Artificial Sequence
  source: /note="Description of Artificial Sequence: Synthetic polynucleotide"
  source: /note="sgRNA with N's"
  modified_base (1)..(25): a, c, u, g, unknown or other
nnnnnnnnnnnnnnnnnnnnnnnnngucauaguuccauuaaagccauugcugaaagacagcaauggcuuugauguuucuaugauaagggcuucggcccguggcguuggggaucgccugcccauuuuaaugggcuucuccccaucuauuu

SEQ ID NO: 27 - protein, 1072 aa, Bacillus sp.
  source: /note="APG08290.1"
MSELDYRIGLDIGTNSIGWGVIELFWNKDRERYEKVRIVDKGVRMFDKAEIPNKGASLAEPRRIARSSRRRLNRKSQRKKEIRNLLVQHGMITQEELDLLYPLSKKSIDIWDIRLDGLDRLLNHLEWARLLIHLAQRRGFKSNRKSELKDAETGKVLSSIQVNEKRLFLYRTVGEMWIKDAEFSKYDRRRNSPNEYVFSVSRADLEKEIVTLFEAQRKFQSSYASKNLQETYLQIWAHQLPFASGNAILNKVGYCSLLKGKERRIPKATYTFQYFSALDQVNRTRLGPDFQPFTQEQKEIILDKMFQRTDYYKKKTIPEVSYYDIRKWLELDETIQFKGLNYDPNEELKKIEKKPFINLKAFYEIKKVVANYAERTNEAFSTLDYDAIAYALTVYKTDKDIRSYLKKSNNLSKRCYDDQLIEELFTLSYTKFGHLSFKAINHVLPIMQEGRTYQEAIHQLGYDTTNLKKENRSMFLPLIPDEITNPIVKRAITQARKVVNAIIRRYGSPNSVHIELARELSKSHDERKKIMTAHDENYKKNKGAISILIENGILNPTGYDIVRYKLWKEQGERCAYSLKEIPPDTFFNELKKERNGSPILEVDHILPYSQSFIDSYHNKVLVYSDENRNKGNRIPYTYFLETNKDWEAFERYVRSNKLFSKKKREYLLKKTYLPRESELIKERHLNDTRYASTFLKNFIEQNLQFKEVEVNLRKKRVQTVNGVITAHLRKRWGLEKNRQETYLHHAMDAIIVACTDHHMVTRITEYYQIKESNKSVKKPYFPMPWEGFRDELLSHLASQPIAKKISEELKAGYQSSDYIFVSRMPKRSVTGAAHDQTIRRKGGIDKKGKTIIIKRVRLKDIKFDENGDFKMVGKEQDLATYEAIKQRYLEHRKNSKKAFETPLYKPSKKGTGNLIKRVKIEGQTKAFVREVNGGVAQNSDLVRVDLFEKDDKYYMVPIYVPDTVCSELPKKVVKSGKGYEQWLTLDNSFTFKSSLYPYDLVRLVKGNEDRFLYFGTLDIDSDRLNFKDVNKPSKQNEYRYSLKTIENLEKYEVGVLGDLRLVKQETRRIFNR

SEQ ID NO: 28 - RNA, 21 nt, Bacillus sp.
  source: /note="crRNA"
gucauaguuccaugaaagcca

SEQ ID NO: 29 - RNA, 85 nt, Bacillus sp.
  source: /note="tracrRNA"
uggcuuugauguuucuaugauaaggguuucggcccguggcgucggggaucgccugcccauuccgaugggcuucuccccauuuauu

SEQ ID NO: 30 - RNA, 140 nt, Artificial Sequence
  source: /note="Description of Artificial Sequence: Synthetic polynucleotide"
  source: /note="sgRNA L1"
gagcggacagcagcuuccuauaucucguacgucauaguuccaugaaagccaaaaguggcuuugauguuucuaugauaaggguuucggcccguggcgucggggaucgccugcccauuccgaugggcuucuccccauuuauu

SEQ ID NO: 31 - RNA, 140 nt, Artificial Sequence
  source: /note="Description of Artificial Sequence: Synthetic polynucleotide"
  source: /note="sgRNA L2"
ccaugauauagacguuguggcuguuguagugucauaguuccaugaaagccaaaaguggcuuugauguuucuaugauaaggguuucggcccguggcgucggggaucgccugcccauuccgaugggcuucuccccauuuauu

SEQ ID NO: 32 - DNA, 6 bp, Artificial Sequence
  source: /note="Description of Artificial Sequence: Synthetic oligonucleotide"
  source: /note="PAM"
  modified_base (1)..(2): a, c, t, g, unknown or other
  modified_base (4)..(4): a, c, t, g, unknown or other
nnrncc

SEQ ID NO: 33 - DNA, 38 bp, Artificial Sequence; identical to SEQ ID NO: 8
  source: /note="Description of Artificial Sequence: Synthetic oligonucleotide"
  source: /note="Target seq and PAM region of plasmid library 1"
  modified_base (31)..(38): a, c, t, g, unknown or other

SEQ ID NO: 34 - DNA, 38 bp, Artificial Sequence; identical to SEQ ID NO: 9
  source: /note="Description of Artificial Sequence: Synthetic oligonucleotide"
  source: /note="Target seq and PAM region of plasmid library 2"
  modified_base (31)..(38): a, c, t, g, unknown or other

SEQ ID NO: 35 - RNA, 135 nt, Artificial Sequence
  source: /note="Description of Artificial Sequence: Synthetic polynucleotide"
  source: /note="sgRNA with N's"
  modified_base (1)..(25): a, c, u, g, unknown or other
nnnnnnnnnnnnnnnnnnnnnnnnngucauaguuccaugaaagccaaaaguggcuuugauguuucuaugauaaggguuucggcccguggcgucggggaucgccugcccauuccgaugggcuucuccccauuuauu

SEQ ID NO: 36 - protein, 1337 aa, Enterococcus sp.
  source: /note="APG05459.1"
MKKDYVIGLDIGTNSVGWAVMTEDYQLVKKKMPIYGNTEKKKIKKNFWGVRLFEEGHTAEDRRLKRTARRRISRRRNRLRYLQAFFEEAMTALDENFFARLQESFLVPEDKKWHRHPIFAKLEDEVAYHETYPTIYHLRKKLADSSEQADLRLIYLALAHIVKYRGHFLIEGKLSTENISVKEQFQQFMIIYNQTFVNGESRLVSAPLPESVLIEEELTEKASRTKKSEKVLQQFPQEKANGLFGQFLKLMVGNKADFKKVFGLEEEAKITYASESYEEDLEGILAKVGDEYSDVFLAAKNVYDAVELSTILADSDKKSHAKLSSSMIVRFTEHQEDLKKFKRFIRENCPDEYDNLFKNEQKDGYAGYIAHAGKVSQLKFYQYVKKIIQDIAGAEYFLEKIAQENFLRKQRTFDNGVIPHQIHLAELQAIIHRQAAYYPFLKENQEKIEQLVTFRIPYYVGPLSKGDASTFAWLKRQSEEPIRPWNLQETVDLDQSATAFIERMTNFDTYLPSEKVLPKHSLLYEKFMVFNELTKISYTDDRGIKANFSGKEKEKIFDYLFKTRRKVKKKDIIQFYRNEYNTEIVTLSGLEEDQFNASFSTYQDLLKCGLTRAELDHPDNAEKLEDIIKILTIFEDRQRIRTQLSTFKGQFSAEVLKKLERKHYTGWGRLSKKLINGIYDKESGKTILDYLIKDDGVSKHYNRNFMQLINDSQLSFKNAIQKAQSSEHEETLSETVNELAGSPAIKKGIYQSLKIVDELVAIMGYAPKRIVVEMARENQTTSTGKRRSIQRLKIVEKAMAEIGSNLLKEQPTTNEQLRDTRLFLYYMQNGKDMYTGDELSLHRLSHYDIDHIIPQSFMKDDSLDNLVLVGSTENRGKSDDVPSKEVVKDMKAYWEKLYAAGLISQRKFQRLTKGEQGGLTLEDKAHFIQRQLVETRQITKNVAGILDQRYNANSKEKKVQIITLKASLTSQFRSIFGLYKVREVNDYHHGQDAYLNCVVATTLLKVYPNLAPEFVYGEYPKFQAFKENKATAKTIIYTNLMRFFTEDEPRFMKDGEILWSNSYLKNIKKELNYHQMNIVKKVEVQKGGFSKESIKPKGPSNKLIPVKNGLDPQKYGGFDSPVVAYTVLFTHEKGKKPLIKQEILGITIMEKTRFEQNPILFLEEKGFLRPRVLMKLPKYTLYEFPEGRRRLLASAKEAQKGNQMVLPEHLLTLLYHAKQCLLPNQSESLAYVEQHQPEFQEILERVVDFAEVHTLAKSKVQQIVKLFEANQTADVKEIAASFIQLMQFNAMGAPSTFKFFQKDIERARYTSIKEIFDATIIYQSTTGLYETRRKVVD

SEQ ID NO: 37 - RNA, 16 nt, Enterococcus sp.
  source: /note="crRNA"
guuuuagagucauguu

SEQ ID NO: 38 - RNA, 74 nt, Enterococcus sp.
  source: /note="tracrRNA"
aacauagcaaguuaaaauaagguuuuaaccguaaucaacuguaaaguggcgcuguuucggcgcuuuuuuuguuu

SEQ ID NO: 39 - RNA, 124 nt, Artificial Sequence
  source: /note="Description of Artificial Sequence: Synthetic polynucleotide"
  source: /note="sgRNA L1"
gagcggacagcagcuuccuauaucucguacguuuuagagucauguuaaagaacauagcaaguuaaaauaagguuuuaaccguaaucaacuguaaaguggcgcuguuucggcgcuuuuuuuguuu

SEQ ID NO: 40 - RNA, 124 nt, Artificial Sequence
  source: /note="Description of Artificial Sequence: Synthetic polynucleotide"
  source: /note="sgRNA L2"
ccaugauauagacguuguggcuguuguaguguuuuagagucauguuaaagaacauagcaaguuaaaauaagguuuuaaccguaaucaacuguaaaguggcgcuguuucggcgcuuuuuuuguuu

SEQ ID NO: 41 - DNA, 3 bp, Artificial Sequence
  source: /note="Description of Artificial Sequence: Synthetic oligonucleotide"
  source: /note="PAM"
  modified_base (1)..(1): a, c, t, g, unknown or other
ngg

SEQ ID NO: 42 - DNA, 38 bp, Artificial Sequence; identical to SEQ ID NO: 8
  source: /note="Description of Artificial Sequence: Synthetic oligonucleotide"
  source: /note="Target seq and PAM region of plasmid library 1"
  modified_base (31)..(38): a, c, t, g, unknown or other

SEQ ID NO: 43 - DNA, 38 bp, Artificial Sequence; identical to SEQ ID NO: 9
  source: /note="Description of Artificial Sequence: Synthetic oligonucleotide"
  source: /note="Target seq and PAM region of plasmid library 2"
  modified_base (31)..(38): a, c, t, g, unknown or other

SEQ ID NO: 44 - RNA, 119 nt, Artificial Sequence
  source: /note="Description of Artificial Sequence: Synthetic polynucleotide"
  source: /note="sgRNA with N's"
  modified_base (1)..(25): a, c, u, g, unknown or other
nnnnnnnnnnnnnnnnnnnnnnnnnguuuuagagucauguuaaagaacauagcaaguuaaaauaagguuuuaaccguaaucaacuguaaaguggcgcuguuucggcgcuuuuuuuguuu

SEQ ID NO: 45 - protein, 1436 aa, Enterococcus sp.
  source: /note="APG04583.1"
MAKNILGLDLGTNSIGWALVQQDFENKEGNILGMGSRIIPMSQDILGEFGKGNSISQTAERTGYRGVRRLRERHLLRRERLHRVLHLLGFLPKHYDEKIDFTQRFGKFINQAEPKLAFDSEFLFKDSFHEMLADFKQNQPEFLKDKNGEDCLVPYDWTIYYLRKKALTQKIEKYELAWLILNFNQKRGYYQLRGEEEKENPNKLVGFHSLKIVDVIPDAETNKKGETWYSLHLENGWVYRRSSKISLADWKDKVRDFIVTTDLNDDGSEKLDKDGIVKRSFRAPSADDWTLLKKKTEKDIDNSNKTVGTYIYDNLLLNPKQKIKGKMVRTIERKFYKQELEQILKTQKEFHSELQSENLLQDCVRELYRNNEQHQQMLEAKDFVHLFLNDIIFYQRPLRSQKSSISNCTLEFRKSKNENGEEVIHRLKVIAKSNPYYQEFRLLQWVQNLAIYTKDDDKNVTNEFLKSTQDWEDLLRWLHSKKEIKQDALIKFLIEKKGLKGKALTIEVAKYRWNYVQDKDYPGNETRYLIQSRLDKVEYAPKDFLTYENEMALWHIIYSINDKIEYEKALKSFANKKGLDEVTFVEAFKKFPPFKSDYGSFSEKAIKKLLPLMRFGTQWNWDNIDQNSKERIGKILTGEYDENIKGRVREKARHLNSETDFQALPLWLAQYVVYGRHSEADIAGKWNSVDDLKQFLDDFKQHSLRNPIVEQVITETLRAVKDIWNFYGKGAKDFFSEIHIELGREMKNTADERKRITTMVTDNENTNLRIKALLAEMALDQNVDNVRPYSPMQQEILKIYEEGVLNAEENIDDDILKISKTAQPSATDLKRYKLWLEQKYRSPYTGQMIPLNKLFTPEYEIEHIIPQSRYFDDSMSNKVICEAAVNKLKDNQIGLVFIKNHHGEVVDFGMGKQVKILEVSDYEDFVKQNYNKNRGKRNKLLLEDIPEKMIERQLNDTRYISKYITQVLSNIVRDDKEGSKDDGVNSKNIVPGNGKITTRLKQDWGLNDVWNDLVLPRFERMNTLTNSNDFTSKNTHGKTIPTVPIELSKGFSKKRIDHRHHAMDALVIACATRDHVNLLNNESSKSDTKRYDLNRKLRKYEKVAYNDPKTGERIEKEVPKDFIKPWETFTEDTRTLLENIVISFKQNLRVINKATNYYEKIENGKKVKVEQKGINWAVRKALHKETVSGQVHLDRIKVAKGKILTATRKTLDASFNEKTIESITDTGIQKILLNYLKSKDNNPEVAFSPEGIEELNKNIRLYNDGKAHQPILKVRVFEQGSKFTLGETGNKTTKFVEAAKGTNLFFGIYEDKSGKRSYETIPLNIVIERQKQGLQAVPETNEKGKQLLFTLSPNDLVYVPEEGVFDENNIKVDRIYKVVSFSTYQCFFVRNDVSTSVVNKVEYSALNKMEKSIDNIMIKENCVKLNVDRLGKISKA

SEQ ID NO: 46 - RNA, 16 nt, Enterococcus sp.
  source: /note="crRNA"
guugugaguuccuuuc

SEQ ID NO: 47 - RNA, 78 nt, Enterococcus sp.
  source: /note="tracrRNA"
gaaaggaacucacaauaaggauuauuccguugugaaaacauuuagcgccucgacuaucuucggggcuuuuuuauuuuu

SEQ ID NO: 48 - RNA, 128 nt, Artificial Sequence
  source: /note="Description of Artificial Sequence: Synthetic polynucleotide"
  source: /note="sgRNA L1"
gagcggacagcagcuuccuauaucucguacguugugaguuccuuucacuugaaaggaacucacaauaaggauuauuccguugugaaaacauuuagcgccucgacuaucuucggggcuuuuuuauuuuu

SEQ ID NO: 49 - RNA, 128 nt, Artificial Sequence
  source: /note="Description of Artificial Sequence: Synthetic polynucleotide"
  source: /note="sgRNA L2"
ccaugauauagacguuguggcuguuguaguguugugaguuccuuucacuugaaaggaacucacaauaaggauuauuccguugugaaaacauuuagcgccucgacuaucuucggggcuuuuuuauuuuu

SEQ ID NO: 50 - DNA, 7 bp, Artificial Sequence
  source: /note="Description of Artificial Sequence: Synthetic oligonucleotide"
  source: /note="PAM"
  modified_base (1)..(2): a, c, t, g, unknown or other
nnraaty

SEQ ID NO: 51 - DNA, 38 bp, Artificial Sequence; identical to SEQ ID NO: 8
  source: /note="Description of Artificial Sequence: Synthetic oligonucleotide"
  source: /note="Target seq and PAM region of plasmid library 1"
  modified_base (31)..(38): a, c, t, g, unknown or other

SEQ ID NO: 52 - DNA, 38 bp, Artificial Sequence; identical to SEQ ID NO: 9
  source: /note="Description of Artificial Sequence: Synthetic oligonucleotide"
  source: /note="Target seq and PAM region of plasmid library 2"
  modified_base (31)..(38): a, c, t, g, unknown or other

SEQ ID NO: 53 - RNA, 123 nt, Artificial Sequence
  source: /note="Description of Artificial Sequence: Synthetic polynucleotide"
  source: /note="sgRNA with N's"
  modified_base (1)..(25): a, c, u, g, unknown or other
nnnnnnnnnnnnnnnnnnnnnnnnnguugugaguuccuuucaaaggaaaggaacucacaauaaggauuauuccguugugaaaacauuuagcgccucgacuaucuucggggcuuuuuuauuuuu

SEQ ID NO: 54 - protein, 1456 aa, Empedobacter sp.
  source: /note="APG01688.1"
MMIKNILGLDLGTNSIGWALIKQDFENKHGEILGMGSRIIPMSQDILGDFGKGNSISQTADRTKYRSVRRLRERFLLRRERLHRVLHLLNFLPQHYASQIDFEKKFGKFKSETEPKLAWENWGGKFSFLFQNSFNEMLEDFKAAGQGLKIPYDWTIYYLRKKALSQKIEKEELAWILLNFNQKRGYYQLRGEEEEENPNKLVEFYSLKIVDVVADEPQKGKSDIWYSLILENGWVYRRASKIPLFDWKDKTRDFIVTTDLNDDRSVKTDKEGNEKRSFRAPSENDWTLVKKKTEQEIDQSHKTVGTYIYETLLLNPKQKIKGKLVRTIERKFYKDELKQILEKQKEFHQELKNDDLYNDCIRELYRNNEAHQLTLSKKDFVHLLMDDLIFYQRPLRSQKSSISNCTLEFRKYKDENGIEHTQYLKAIPKSNPYYQEFRLWQWMYNLNIYRKDDEANVTKEFLNTNKDFESLFEFLNNRKEIEQKPLIKFLLEQKDINKKLLNAEAEKYRWNYVEDKKYPCNETKTMISSRLDKVENISDDFLTRDIEQKIWHIIYSVNDKIEYEKALKSFATRNDLDENSFIEAFKKFSPFKSEYGSFSEKAIKKLLPLMRLGKYWYEDEIVKHSDIYFKNIENLLGDFSNRDKKISEEDKEKWNKSINLKLQEELKDFQTAEIDLFQGLRLHIAQYLVYGRHSEASMIGKWNSAEDLEEFLKDFKQHSLRNPIVEQVITETLRVVKDIWLKYGNGAKDFFNEIHIELGREMKLPADDRKKLTNQISENENTNFRIKALLAEMMNDSSVENVRPFSPMQQEILKIYEDDVLKSDIEIEDDILKISKTAQPSPSDLKRYKLWLEQKYKSPYTGQIIPLNKLFTPEYEIEHIIPQSRYFDDSFSNKVICESAVNKLKDNYIGLEFIKQFGGTIIELGFGKSIKVFETKEYEDFVKKHYANNQGKRNKLLMEDIPEKMIERQMNDTRYISKYISGVLSNIVRVEDGSDEGVNSKNIVPGNGKITTQLKQDWGLNDVWNDLILPRFERMNQLTNSKVFTAWNENYQKFLPTVPIEYSKGFSKKRIDHRHHALDALVIACATKDHVNLLNNQSAKSDTKRYDLKKKSMKFEKVVYNDAKTGEKIEREVPKQFLKPWENFTLDVKHNLETIIVSFKQNLRVINKATNYYEKYVEKDGTKNKERVEQTGTNWAIRKPMHKDTVSGKVDLPWVKVPKGKILTATRKSLDSSFDLKSIGSITDTGIQKILKNYLAFKDGNPELAFSPEGIDDLNKNIEKYNDGKPHQPINKVRVFELGSKFQVGQSGNKKDKYVEAAKGTNLFFAVYEDEKGKRNYETIPLNEVIERQKQGLSVVDLKGTNDFYLCPNDFVYIPSGDELENINNVDFKDIKKEINERIYKVVSFTGNRLSCIPYMVATTIVNKLEFTQLNKIEFTKEKEICIKLNVDRLGNISKA

SEQ ID NO: 55 - RNA, 18 nt, Empedobacter sp.
  source: /note="crRNA"
guugugaauugcuuucaa

SEQ ID NO: 56 - RNA, 75 nt, Empedobacter sp.
  source: /note="tracrRNA"
uugaaaagcaauucacaauaaggauuauuccguugugaaaacauucaaggcggggcaacucgucuuuuuucuuuu

SEQ ID NO: 57 - RNA, 127 nt, Artificial Sequence
  source: /note="Description of Artificial Sequence: Synthetic polynucleotide"
  source: /note="sgRNA L1"
gagcggacagcagcuuccuauaucucguacguugugaauugcuuucaaaaaguugaaaagcaauucacaauaaggauuauuccguugugaaaacauucaaggcggggcaacucgucuuuuuucuuuu

SEQ ID NO: 58 - RNA, 127 nt, Artificial Sequence
  source: /note="Description of Artificial Sequence: Synthetic polynucleotide"
  source: /note="sgRNA L2"
ccaugauauagacguuguggcuguuguaguguugugaauugcuuucaaaaaguugaaaagcaauucacaauaaggauuauuccguugugaaaacauucaaggcggggcaacucgucuuuuuucuuuu

SEQ ID NO: 59 - DNA, 6 bp, Artificial Sequence
  source: /note="Description of Artificial Sequence: Synthetic oligonucleotide"
  source: /note="PAM"
  modified_base (1)..(2): a, c, t, g, unknown or other
  modified_base (4)..(5): a, c, t, g, unknown or other
nnrnnc

SEQ ID NO: 60 - DNA, 38 bp, Artificial Sequence; identical to SEQ ID NO: 8
  source: /note="Description of Artificial Sequence: Synthetic oligonucleotide"
  source: /note="Target seq and PAM region of plasmid library 1"
  modified_base (31)..(38): a, c, t, g, unknown or other

SEQ ID NO: 61 - DNA, 38 bp, Artificial Sequence; identical to SEQ ID NO: 9
  source: /note="Description of Artificial Sequence: Synthetic oligonucleotide"
  source: /note="Target seq and PAM region of plasmid library 2"
  modified_base (31)..(38): a, c, t, g, unknown or other

SEQ ID NO: 62 - RNA, 122 nt, Artificial Sequence
  source: /note="Description of Artificial Sequence: Synthetic polynucleotide"
  source: /note="sgRNA with N's"
  modified_base (1)..(25): a, c, u, g, unknown or other
nnnnnnnnnnnnnnnnnnnnnnnnnguugugaauugcuuucaaaaaguugaaaagcaauucacaauaaggauuauuccguugugaaaacauucaaggcggggcaacucgucuuuuuucuuuu

SEQ ID NO: 63 - RNA, 4 nt, Artificial Sequence
  source: /note="Description of Artificial Sequence: Synthetic oligonucleotide"
  source: /note="4bp linker"
aaag

SEQ ID NO: 64 - RNA, 4 nt, Artificial Sequence
  source: /note="Description of Artificial Sequence: Synthetic oligonucleotide"
  source: /note="4bp linker"
gaaa

SEQ ID NO: 65 - RNA, 4 nt, Artificial Sequence
  source: /note="Description of Artificial Sequence: Synthetic oligonucleotide"
  source: /note="4bp linker"
acuu

SEQ ID NO: 66 - RNA, 6 nt, Artificial Sequence
  source: /note="Description of Artificial Sequence: Synthetic oligonucleotide"
  source: /note="6bp linker"
caaagg

SEQ ID NO: 67 - protein, 7 aa, Artificial Sequence
  source: /note="Description of Artificial Sequence: Synthetic peptide"
  source: /note="NLS"
PKKKRKV

SEQ ID NO: 68 - RNA, 6 nt, Artificial Sequence
  source: /note="Description of Artificial Sequence: Synthetic oligonucleotide"
  source: /note="conserved sequence in base of hairpin stem of tracrRNA"
  modified_base (2)..(2): a, c, u, g, unknown or other
  modified_base (4)..(5): a, c, u, g, unknown or other
unanng

SEQ ID NO: 69 - DNA, 6 bp, Artificial Sequence
  source: /note="Description of Artificial Sequence: Synthetic oligonucleotide"
  source: /note="APG05083.1/exemplary PAM"
  modified_base (1)..(2): a, c, t, g, unknown or other
  modified_base (4)..(4): a, c, t, g, unknown or other
nnrncc

SEQ ID NO: 70 - DNA, 7 bp, Artificial Sequence
  source: /note="Description of Artificial Sequence: Synthetic oligonucleotide"
  source: /note="APG07433.1/exemplary PAM"
  modified_base (1)..(4): a, c, t, g, unknown or other
nnnnccr

SEQ ID NO: 71 - DNA, 6 bp, Artificial Sequence
  source: /note="Description of Artificial Sequence: Synthetic oligonucleotide"
  source: /note="APG07513.1/exemplary PAM"
  modified_base (1)..(2): a, c, t, g, unknown or other
  modified_base (4)..(4): a, c, t, g, unknown or other
nnrncc

SEQ ID NO: 72 - DNA, 6 bp, Artificial Sequence
  source: /note="Description of Artificial Sequence: Synthetic oligonucleotide"
  source: /note="APG01688.1/exemplary PAM"
  modified_base (1)..(2): a, c, t, g, unknown or other
  modified_base (5)..(5): a, c, t, g, unknown or other
nnranc

SEQ ID NO: 73 - DNA, 30 bp, Artificial Sequence
  source: /note="Description of Artificial Sequence: Synthetic oligonucleotide"
  source: /note="mismatch repair Table 4"
gagcggacagcagcttcctatatctcgtac

SEQ ID NO: 74 - DNA, 30 bp, Artificial Sequence
  source: /note="Description of Artificial Sequence: Synthetic oligonucleotide"
  source: /note="mismatch repair Table 4"
gagcggacagcagcttcctatatctcgtag

SEQ ID NO: 75 - DNA, 30 bp, Artificial Sequence
  source: /note="Description of Artificial Sequence: Synthetic oligonucleotide"
  source: /note="mismatch repair Table 4"
gagcggacagcagcttcctatatctcgttc

SEQ ID NO: 76 - DNA, 30 bp, Artificial Sequence
  source: /note="Description of Artificial Sequence: Synthetic oligonucleotide"
  source: /note="mismatch repair Table 4"
gagcggacagcagcttcctatatctcgaac

SEQ ID NO: 77 - DNA, 30 bp, Artificial Sequence
  source: /note="Description of Artificial Sequence: Synthetic oligonucleotide"
  source: /note="mismatch repair Table 4"
gagcggacagcagcttcctatatctcctac

SEQ ID NO: 78 - DNA, 30 bp, Artificial Sequence
  source: /note="Description of Artificial Sequence: Synthetic oligonucleotide"
  source: /note="mismatch repair Table 4"
gagcggacagcagcttcctatatctggtac

SEQ ID NO: 79 - DNA, 30 bp, Artificial Sequence
  source: /note="Description of Artificial Sequence: Synthetic oligonucleotide"
  source: /note="mismatch repair Table 4"
gagcggacagcagcttcctatatcacgtac

SEQ ID NO: 80 - DNA, 30 bp, Artificial Sequence
  source: /note="Description of Artificial Sequence: Synthetic oligonucleotide"
  source: /note="mismatch repair Table 4"
gagcggacagcagcttcctatatgtcgtac

SEQ ID NO: 81 - DNA, 30 bp, Artificial Sequence
  source: /note="Description of Artificial Sequence: Synthetic oligonucleotide"
  source: /note="mismatch repair Table 4"
gagcggacagcagcttcctataactcgtac

SEQ ID NO: 82 - DNA, 30 bp, Artificial Sequence
  source: /note="Description of Artificial Sequence: Synthetic oligonucleotide"
  source: /note="mismatch repair Table 4"
gagcggacagcagcttcctatttctcgtac

SEQ ID NO: 83 - DNA, 30 bp, Artificial Sequence
  source: /note="Description of Artificial Sequence: Synthetic oligonucleotide"
  source: /note="mismatch repair Table 4"
gagcggacagcagcttcctaaatctcgtac

SEQ ID NO: 84 - DNA, 30 bp, Artificial Sequence
  source: /note="Description of Artificial Sequence: Synthetic oligonucleotide"
  source: /note="mismatch repair Table 4"
gagcggacagcagcttcctttatctcgtac

SEQ ID NO: 85 - DNA, 30 bp, Artificial Sequence
  source: /note="Description of Artificial Sequence: Synthetic oligonucleotide"
  source: /note="mismatch repair Table 4"
gagcggacagcagcttccaatatctcgtac

SEQ ID NO: 86 - DNA, 30 bp, Artificial Sequence
  source: /note="Description of Artificial Sequence: Synthetic oligonucleotide"
  source: /note="mismatch repair Table 4"
gagcggacagcagcttcgtatatctcgtac

SEQ ID NO: 87 - DNA, 30 bp, Artificial Sequence
  source: /note="Description of Artificial Sequence: Synthetic oligonucleotide"
  source: /note="mismatch repair Table 4"
gagcggacagcagcttgctatatctcgtac

SEQ ID NO: 88 - DNA, 30 bp, Artificial Sequence
  source: /note="Description of Artificial Sequence: Synthetic oligonucleotide"
  source: /note="mismatch repair Table 4"
gagcggacagcagctacctatatctcgtac

SEQ ID NO: 89 - DNA, 30 bp, Artificial Sequence
  source: /note="Description of Artificial Sequence: Synthetic oligonucleotide"
  source: /note="mismatch repair Table 4"
gagcggacagcagcatcctatatctcgtac

SEQ ID NO: 90 - DNA, 30 bp, Artificial Sequence
  source: /note="Description of Artificial Sequence: Synthetic oligonucleotide"
  source: /note="mismatch repair Table 4"
gagcggacagcaggttcctatatctcgtac

SEQ ID NO: 91 - DNA, 30 bp, Artificial Sequence
  source: /note="Description of Artificial Sequence: Synthetic oligonucleotide"
  source: /note="mismatch repair Table 4"
gagcggacagcaccttcctatatctcgtac

SEQ ID NO: 92 - DNA, 30 bp, Artificial Sequence
  source: /note="Description of Artificial Sequence: Synthetic oligonucleotide"
  source: /note="mismatch repair Table 4"
gagcggacagctgcttcctatatctcgtac

SEQ ID NO: 93 - DNA, 30 bp, Artificial Sequence
  source: /note="Description of Artificial Sequence: Synthetic oligonucleotide"
  source: /note="mismatch repair Table 4"
gagcggacaggagcttcctatatctcgtac

SEQ ID NO: 94 - DNA, 30 bp, Artificial Sequence
  source: /note="Description of Artificial Sequence: Synthetic oligonucleotide"
  source: /note="mismatch repair Table 4"
gagcggacaccagcttcctatatctcgtac

SEQ ID NO: 95 - DNA, 30 bp, Artificial Sequence
  source: /note="Description of Artificial Sequence: Synthetic oligonucleotide"
  source: /note="mismatch repair Table 4"
gagcggactgcagcttcctatatctcgtac

SEQ ID NO: 96 - DNA, 30 bp, Artificial Sequence
  source: /note="Description of Artificial Sequence: Synthetic oligonucleotide"
  source: /note="mismatch repair Table 4"
gagcggagagcagcttcctatatctcgtac

SEQ ID NO: 97 - DNA, 30 bp, Artificial Sequence
  source: /note="Description of Artificial Sequence: Synthetic oligonucleotide"
  source: /note="mismatch repair Table 4"
gagcggtcagcagcttcctatatctcgtac

SEQ ID NO: 98 - DNA, 30 bp, Artificial Sequence
  source: /note="Description of Artificial Sequence: Synthetic oligonucleotide"
  source: /note="mismatch repair Table 4"
gagcgcacagcagcttcctatatctcgtac

SEQ ID NO: 99 - DNA, 30 bp, Artificial Sequence
  source: /note="Description of Artificial Sequence: Synthetic oligonucleotide"
  source: /note="mismatch repair Table 4"
gagccgacagcagcttcctatatctcgtac

SEQ ID NO: 100 - DNA, 30 bp, Artificial Sequence
  source: /note="Description of Artificial Sequence: Synthetic oligonucleotide"
  source: /note="mismatch repair Table 4"
gaggggacagcagcttcctatatctcgtac

SEQ ID NO: 101 - DNA, 30 bp, Artificial Sequence
  source: /note="Description of Artificial Sequence: Synthetic oligonucleotide"
  source: /note="mismatch repair Table 4"
gaccggacagcagcttcctatatctcgtac

SEQ ID NO: 102 - DNA, 30 bp, Artificial Sequence
  source: /note="Description of Artificial Sequence: Synthetic oligonucleotide"
  source: /note="mismatch repair Table 4"
gtgcggacagcagcttcctatatctcgtac

SEQ ID NO: 103 - DNA, 30 bp, Artificial Sequence
  source: /note="Description of Artificial Sequence: Synthetic oligonucleotide"
  source: /note="mismatch repair Table 4"
cagcggacagcagcttcctatatctcgtac

SEQ ID NO: 104 - DNA, 30 bp, Artificial Sequence
  source: /note="Description of Artificial Sequence: Synthetic oligonucleotide"
  source: /note="mismatch repair Table 6"
gagcggacagcagcttcctatatctcgtat

SEQ ID NO: 105 - DNA, 30 bp, Artificial Sequence
  source: /note="Description of Artificial Sequence: Synthetic oligonucleotide"
  source: /note="mismatch repair Table 6"
gagcggacagcagcttcctatatctcgtgc

SEQ ID NO: 106 - DNA, 30 bp, Artificial Sequence
  source: /note="Description of Artificial Sequence: Synthetic oligonucleotide"
  source: /note="mismatch repair Table 6"
gagcggacagcagcttcctatatctcgcac

SEQ ID NO: 107 - DNA, 30 bp, Artificial Sequence
  source: /note="Description of Artificial Sequence: Synthetic oligonucleotide"
  source: /note="mismatch repair Table 6"
gagcggacagcagcttcctatatctcatac

SEQ ID NO: 108 - DNA, 30 bp, Artificial Sequence
  source: /note="Description of Artificial Sequence: Synthetic oligonucleotide"
  source: /note="mismatch repair Table 6"
gagcggacagcagcttcctatatcttgtac

SEQ ID NO: 109 - DNA, 30 bp, Artificial Sequence
  source: /note="Description of Artificial Sequence: Synthetic oligonucleotide"
  source: /note="mismatch repair Table 6"
gagcggacagcagcttcctatatcccgtac

SEQ ID NO: 110 - DNA, 30 bp, Artificial Sequence
  source: /note="Description of Artificial Sequence: Synthetic oligonucleotide"
  source: /note="mismatch repair Table 6"
gagcggacagcagcttcctatatttcgtac

SEQ ID NO: 111 - DNA, 30 bp, Artificial Sequence
  source: /note="Description of Artificial Sequence: Synthetic oligonucleotide"
  source: /note="mismatch repair Table 6"
gagcggacagcagcttcctatacctcgtac

SEQ ID NO: 112 - DNA, 30 bp, Artificial Sequence
  source: /note="Description of Artificial Sequence: Synthetic oligonucleotide"
  source: /note="mismatch repair Table 6"
gagcggacagcagcttcctatgtctcgtac

SEQ ID NO: 113 - DNA, 30 bp, Artificial Sequence
  source: /note="Description of Artificial Sequence: Synthetic oligonucleotide"
  source: /note="mismatch repair Table 6"
gagcggacagcagcttcctacatctcgtac

SEQ ID NO: 114 - DNA, 30 bp, Artificial Sequence
  source: /note="Description of Artificial Sequence: Synthetic oligonucleotide"
  source: /note="mismatch repair Table 6"
gagcggacagcagcttcctgtatctcgtac

SEQ ID NO: 115 - DNA, 30 bp, Artificial Sequence
  source: /note="Description of Artificial Sequence: Synthetic oligonucleotide"
  source: /note="mismatch repair Table 6"
gagcggacagcagcttcccatatctcgtac

SEQ ID NO: 116 - DNA, 30 bp, Artificial Sequence
  source: /note="Description of Artificial Sequence: Synthetic oligonucleotide"
  source: /note="mismatch repair Table 6"
gagcggacagcagcttcttatatctcgtac

SEQ ID NO: 117 - DNA, 30 bp, Artificial Sequence
  source: /note="Description of Artificial Sequence: Synthetic oligonucleotide"
  source: /note="mismatch repair Table 6"
gagcggacagcagctttctatatctcgtac

SEQ ID NO: 118 - DNA, 30 bp, Artificial Sequence
  source: /note="Description of Artificial Sequence: Synthetic oligonucleotide"
  source: /note="mismatch repair Table 6"
gagcggacagcagctccctatatctcgtac

SEQ ID NO: 119 - DNA, 30 bp, Artificial Sequence
  source: /note="Description of Artificial Sequence: Synthetic oligonucleotide"
  source: /note="mismatch repair Table 6"
gagcggacagcagcctcctatatctcgtac

SEQ ID NO: 120 - DNA, 30 bp, Artificial Sequence
  source: /note="Description of Artificial Sequence: Synthetic oligonucleotide"
  source: /note="mismatch repair Table 6"
gagcggacagcagtttcctatatctcgtac

SEQ ID NO: 121 - DNA, 30 bp, Artificial Sequence
  source: /note="Description of Artificial Sequence: Synthetic oligonucleotide"
  source: /note="mismatch repair Table 6"
gagcggacagcaacttcctatatctcgtac

SEQ ID NO: 122 - DNA, 30 bp, Artificial Sequence
  source: /note="Description of Artificial Sequence: Synthetic oligonucleotide"
  source: /note="mismatch repair Table 6"
gagcggacagcggcttcctatatctcgtac

SEQ ID NO: 123 - DNA, 30 bp, Artificial Sequence
  source: /note="Description of Artificial Sequence: Synthetic oligonucleotide"
  source: /note="mismatch repair Table 6"
gagcggacagtagcttcctatatctcgtac

SEQ ID NO: 124 - DNA, 30 bp, Artificial Sequence
  source: /note="Description of Artificial Sequence: Synthetic oligonucleotide"
  source: /note="mismatch repair Table 6"
gagcggacaacagcttcctatatctcgtac

SEQ ID NO: 125 - DNA, 30 bp, Artificial Sequence
  source: /note="Description of Artificial Sequence: Synthetic oligonucleotide"
  source: /note="mismatch repair Table 6"
gagcggacggcagcttcctatatctcgtac

SEQ ID NO: 126 - DNA, 30 bp, Artificial Sequence
  source: /note="Description of Artificial Sequence: Synthetic oligonucleotide"
  source: /note="mismatch repair Table 6"
gagcggatagcagcttcctatatctcgtac

SEQ ID NO: 127 - DNA, 3210 bp, Artificial Sequence
  source: /note="Description of Artificial Sequence: Synthetic polynucleotide"
  source: /note="APG05083.1 mammalian codon optimized sequence"
atgagagagctggattaccggatcggcctggatatcgggaccaactccattggatggggcatcatcgagctgtcttggaacaaagacagagaacagtacgagaaggcaagaatcgtggacaagggcgtgagaatgttcgacaaggccgaaatacccaagaccggagccagcctggccgagcctagaagaattgccagatcaagcagaagacggctcaacagaaagtctcagagaaaaaaagatattcggaacctgctggtccagcacgagatcatcagccaaaaggaactcgctagcctgtatcctctgaccaagagcagcatggacatttgggacatcagactggacggcctggacagactgctggatagattcgagtggaccagattgctgatccacctggctcagcggagaggcttcaaaagcaaccggaagagcgagctgaaggacgtggaaaccggcaaggtgctctccagcatccaggctaatgagaagcggctgtccctgtacagaactgtgggcgagatgtggatgaagaatgaagattttagcaagtacgacaaaagaagaaatagtagcaacgaatacgtgttctctgtgtcccgggccgacctggaaaaggaaatcgtgacactgtttgaagctcagcggaagttccagagcagctatgccagcgccgatcttcaaaaaacctacctccagatctgggcccatcaactgcctttcgcctctggcaacgccatcgttaacaaggtgggctactgcagcctactgaaaggcaaggagaagagagttcctaaggccacctacaccttccaatacttcagcaccctggatcagatcaacagaaccagactgggcccaaacttccagcccttcaccaaggaacagagagatgtgatcctggacgagatgtttaaccggaccgattattacaagaagaagaccatccctgaggtgacgtactacgatatcagaaaatggctggccctggacgagacaatccagttcaagggcctgacctacgaccctaatgaagaactgaagaaaattgagctaaagtcttttatcaatctgaagcctttctacgagataaagaaggtggtgacaaactacgccaagaagacaaatgaggcctttagcacactggactatgacacctttgcctacgccctgacagtgtacaagaccgacaaggacatccgctcctacctgaaaaagagtaacaacctgtccaaatgctgctacgacgaccaactgatcgaggaattgctgacactgagctacaccaaattcggccacctgagcttcaaggctatcaaccacgttctgcctatcatgcaggagggcagaacctaccaggaggccattcaccagctcggctacgatgccacaaacctcaaaaaagagaaccggtctatgttcctgcctctgttccctgacgagatcaccaaccccatcgtgaagagggccctgacccaggccaggaaggtggtcaacgccatcatcagacgatacgggtctccaaacagcgtgcacatcgagctggccagagagctgagcaagagccacgacgagagaacaaagatcatgaaagctcatgatgaaaactacaaaaagaacaagggcgctatcagcatcctgatcgagaacggtattctgaatcctacaggttatgacatcgtccggtacaagctgtggaaggaacagggcgagagatgcgcctattctctgaaacagatccccgccaacaccttcttcaacgaaatgaagaaggagcggtccggcagccctgtgctggaaatcgatcacatcctgccctacagccagagcttcatcgacagctaccacaacaaagtgctggtgtacggggatgagaaccagaaaaagggcaatagaatcccgtacacctacttcctggaaggcaacaaggactgggagtctttcgagagctatgtgcgcctgaactcctttttcagcaagaaaaagcgaggatatctgctgaagaaggcttacctgccaagagagagtaacatgatcaaggaacggcacctcaacgacacccggtacgccagctcctacctgaagaacttcatcgagaagaatctgaagttcaaggaggtggaaggctctacccggaagaagcacgtgcaaaccgtgaacggcataatcacagcccacctgagaaagagatggggcctggaaaaggaccgccaggagacatatcttcatcacgctatggacgccatcatcgtggcatgcaccgaccaccacatggtgacaaaggtgaccgagtactaccagatcaaagaaagcaataaatctattagaaagccttacttccccctgccttgggtgggctttagagaggaaattctgtcccacctggctcggcagcctatcgccagaaagatctctgaagagctgaagatcggataccagagcttcgattacatcctcgtgtctagaatgcctaaaagatcagtgaccggcgccgcccacgagcagaccattatgaaaaagggaggcatcgacaaaaaaggaaaaaccatcatcattaagcgggtctacctgaaggatatcaagttcgacgagaatggcgatttcaagatggttggaaaggaacaggacctggctacctacgaggccatcaagcagagatacatcgagtacggcaaggaatccaagaaggccttcgagacccctctgtataagcccagcaagaaaggcaaaggcaacctgatcaagaagatcaaagtggaagtgcaaaccaagagctttgtgagagaagtcaacggcggagtggcccagaacggcgatctggtgcgggttgacctgttcgagaaggataatagatactacatgatccccatctacgtgatggataccgtgcacagcgaacttcctaacaaggccgtgaccagcagcaaaggctatgagcaatggctgaccatcgacaacagcttcaccttcaagttcagcctatacccctacgacctggtgcggctggtcaagggtaacgaggacagattcctgtacttttccaccctggatattaacagtgatagactcaacttcaaagacgtcaacaagcccagcaagcaggccgagaacagatatagcctgaagacaatcgaaaacctggaaaaatacgaggtgggcgtcctgggcgacctcagatttgtgagacaggagatcagaaagaacttc

SEQ ID NO: 128 - DNA, 3213 bp, Artificial Sequence
  source: /note="Description of Artificial Sequence: Synthetic polynucleotide"
  source: /note="APG07433.1 mammalian codon optimized sequence"
atgagagagctggactacagaattggcctggacatcggcaccaacagcatcggatggggcgtgatcgagctgtcctggaacaaagaccgggagagatacgagaaggtcagaatcgtggatcaaggcgtgagaatgttcgacagagccgagatgcccaagacaggcgccagcttagctgaacccagaagaatcgccagatccagcagacggagactgaatcgcaagtcccagagaaagaaaaacatccggaacctgctggtgcaacacggcgtgatcacacaggaggaactggatagcctgtaccccctgagcaaaaagagcatggacatctggggcattcggctcgacggcctggacagactcctcaatcatttcgagtgggccagactgctgatccacctggctcagagacggggctttaagtccaacagaaagagtgaactgaaagatacagagacaggcaaggtgctgagcagcatccaactgaacgagaaacggctgagcttgtatagaaccgtgggcgagatgtggatgaaggaccccgacttctctaaatacgataggaagagaaatagccccaacgaatacgtgttcagcgtgtctagagccgagctggaaaaggaaatcgtgaccctgttcgccgcccagcggagattccagagcccttacgccagcaaagatctgcaggagacatatctgcagatctggacccaccaactgcctttcgccagcggcaatgccatcctgaacaaggtcggatactgctccctgttgaaaggcaaagaaagaaggattcccaaggctacatacaccttccaatacttctctgctctggaccaggtgaatcggaccagactgggacctgatttccagcccttcaccaaggagcaacgggaaattatcttgaacaacatgttccagaggacagattactacaagaagaaaaccatccccgaggtgacctactatgacatacggaagtggctggaattggacgagacaattcagttcaagggcctgaactacgaccctaacgaggaactgaagaagatcgagaagaagccttttatcaatctgaaggccttctacgagatcaacaaggtggtggccaactacagcgaaagaaccaacgagaccttctccaccctggactacgacggcatcggctacgccctgaccgtgtacaaaaccgacaaggatatccgcagctacctgaagagcagtcacaacctacctaagagatgctacgacgaccaactgatcgaggaactgctgagcctgagctacacaaagttcggccacctgtccctgaaagccatcaaccacgtgctgtctatcatgcagaagggcaatacctacaaggaagccgtggaccaactgggctacgacaccagcggccttaagaaggagaagaggtccaagttcctgccacctatttctgatgaaatcacgaatccaatcgtgaaaagggccctgacccaggccagaaaagtggtgaacgccataattagaagacacggatctcctcactccgtgcacatcgagctggccagagagctgagcaagaaccacgacgagcggacaaagatcgtcagcgcccaggatgaaaactacaagaaaaacaagggcgctatcagcatcctgtctgagcacggcatcctgaaccctacaggctacgacatcgtgagatacaaactgtggaaggagcagggcgaacggtgcgcctacagcctgaaggaaatccctgccgatacatttttcaacgagctgaagaaggaacgcaacggcgcccctatccttgaagtggaccacatcctgccctacagccagtccttcatcgactcctaccacaacaaggtcctggtgtacagcgacgaaaaccggaaaaagggcaacagaatcccttatacctacttcctggaaaccaacaaggattgggaggcctttgagcggtacgtgcggagcaacaaattcttctccaagaaaaagcgagagtaccttctgaagcgggcttatctgcctagagaatctgagctgatcaaagaacgccacctgaacgacaccagatacgcctctaccttcctgaagaacttcatcgagcagaacctgcagttcaaggaagccgaggacaaccccagaaaaagacgggtgcaaaccgtgaacggcgttatcaccgcccacttcagaaagcggtggggcctggagaaggaccggcaggagacatacctccatcacgctatggacgccatcatcgtggcttgtacagaccaccacatggtcaccagagtgaccgagtactatcagatcaaggaaagcaacaagagcgtgaagaagccctattttcctatgccttgggaaggcttccgggacgagctgctgagccacttggcttctcagcctatcgccaagaaaatcagcgaggaactgaaggccggctaccagagcctggactacatcttcgtgtccagaatgcctaagagaagcattacaggcgctgctcataagcagaccatcatgcggaagggaggaattgacaagaagggcaaaacaatcatcatcgaacggctgcacctgaaggatatcaagttcgacgagaacggagatttcaagatggtgggcaaggaacaggacatggccacatacgaagctattaaacagagatacctggagcacggcaagaatagcaagaaggccttcgagacccctctgtacaagcccagcaaaaagggcacaggtaacctgatcaagcgggtgaaggtggaaggacaggccaagagctttgtgagggaagtgaacggcggagtggcccaaaatggcgatctggttagagttgatttgtttgagaaggatgataagtactacatggtccccatctacgtgccagacaccgtgtgtagcgagctgcccaaaaaggtggtcgccagctctaagggctatgagcagtggctgacactggataacagcttcacctttaagttcagcctgtacccttatgatctggtgcggctggtcaagggagatgaggatcggttcctgtactttggcaccctggacatcgacagcgacagacttaacttcaaggacgtgaacaagccaagcaagaagaacgagtaccggtacagcttgaaaaccatcgaggacttggagaagtacgaggtgggcgtgctgggcgatctaagactggtccggaaggaaactcgaagaaacttccac

SEQ ID NO: 129 - DNA, 3213 bp, Artificial Sequence
  source: /note="Description of Artificial Sequence: Synthetic polynucleotide"
  source: /note="APG07513.1 mammalian codon optimized sequence"
atgcgggaactggattacagaattggactggacatcgggaccaactcaattggctggggagtgatcgagctgagctggaacaaggacagagagcagtacgagaagaccagaatcgtggacaagggcgttaggatgttcgacaaggccgagatccccaagaccggagccagcctggccgagcctagacgtatcgccagatcctccagacgtagactgaacagaaagtcccagaggaagaaggacattcggaacctgctggtgcaacacgagatcattagccaaaaagaactgaccagcctgtaccctctgtctaaatccagcatggacatctgggacatccggctggacggcctggacagactgcttgatagattcgagtgggcccggctcctgatccacctggctcagcggcggggctttaaaagcaaccggaagtctgagcttaaagacgtggaaacaggaaaagttctgtccagcatccaggtgaatgaaaagcggctgagcctgtacagaaccgtgggcgagatgtggatgaagaacgccgattgcagcaagtacggcaaacgtagaaatagccccaacgagtacgtgttcagcgtgtctagagccgacttggagaaagaaattgtgacacttttcgaggcccagcgaaaattccacagcagctacgccagtgtggacctgcagaagacatacatccaaatctgggctcatcaactgccatttgcctctggcaatgccattgtgaacaaggtgggatactgctctctgctgaagggcaaagaaaagagagtgcctaaggccacatacacctttcagtattttaacaccctggaccagatcaaccggacaagactgggccctaacttccaacctttcaccaaggagcagagagatatcatcctagacaaaatgttccagagaaccgactactacaagaaaaaaacaatccctgaggtgacatactacgatatcagaaagtggctggccctggacgaaaccatccagttcaagggcctgacctacgatcctaatgaagaactgaagaagatcgagatgaagccattcatcaacctgaaacctttctacgagatcaagaaggtggtgaccaactacgccaagaagacaaacgaggtgttctctgccctggactatgacaccgtggcttatgccctcaccgtgtacaaaacagacaaggatatcagaagctaccttaagcggtccaacaacctgagcaagagatgttacgacgaccaactgatcgaggaactgctgacactgagctacaccaagttcggccacctgtccttcaaggccatcaatcacgtgctgcccatcatgcaggagggcagaacctaccaagaggctattcaccaactgggctatgacacgaccaacctgaagaaggaaaatagaagcatgttcctgcccatcatccctgacgagatcaccaaccctatcgtgaagcgggccctgacgcaggcccggaaagtggtgaatgccatcatccgcagatacggctctcctaattctgtccacatcgagctggccagagagctgagcaaaagccacgacgagcggaagaagatcatgaccgcccacgacgagaactacaagaaaaacaagggcgccgtgtccatcctgatcgataacggcatcctgaatcctacaggatacgatatcgtgcggtacaagctgtggaaggaacagggcgaaagatgcgcctatagcctgaaaaaaatccccgccaacaccttcttcaacgagctaaaaaaggaacggagcggcccacctgtgctggaagtggaccacatcctgccctacagccagagcttcatcgacagctaccacaacaaggtgctggtgtacggcgacgagaaccagaagaagggcaatagaatcccttacacatttttcagcgaagaagataaggaatgggagagcttcgagagctacgttcggagcaacagcttcttcagcaagaaaaagcgcggctacctgctgaagaaggcctacctgcccagagaaagcaacctgatcaaggaacggcacctcaacgacacacggtacgccagcagttacctgaagaatttcatcgagaagaacctgaagttcaaggaagccgtggggatcacccggaagaagtacgtgcaaaccgtgaacggcgtgatcaccgcccacctgcggaagcggtggggccttgagaaggaccggcaggagacctacctgcaccacgctatggacgccatcatcgtggcctgcaccgatcaccacatggtgacgaaggtgaccgagtactaccagatcaaagaaggcaataagagcatcaagaagccttattttcctctgccctggatgggcttcagagaagaaatcctgtctcacctggagtctcaacctatcgccagaaaaatttctgaagagctgaaaattggataccagtcccccgattacatcctggtcagccggatgcctaagagaagcgtgaccggcagcgcccacgatcagaccgtgatgaagaagggcgatatcgataagaagggcaagacaatcatcatcaagcgggtgcacctgaaggatatcaagttcgacgaaaatggcgacttcaaaatggtgggcaaggagcaggacctggctacatacgaagctatcaaacagagatacctggagtaccggaaggaaagcaagaaggccttcgagacccctctgtacaagccatctaaaaaaggaaaaggtaacctgatcaaaaagatcaaggtggaagtgcaaaccaaatctttcgtgagagagattaacggcggagtggcccagaacggcgacctggttagagtggatctgttcgagaaggacaacagatattacatggtccccatctacgtggtggacaccgtgcggtctgaactccccaacaaagcagtgacaagctccaaaggctatgaacagtggctgagcatcgacaatagtttcaccttcaagtttagtctgtacccctacgacctcgtgcggctggtcaagggcgacgaggatcgcttcctgtacttctccaccctggatatcaacagcgacagactgaacttcaaggacgtgaacaagcctagcaagcaggctgaataccggtacagcctgaagacgatcgagaacctggaaaaatacgagatcggtgttctgggagatctgagactcgttagacaggagacaagaaaaattttcaag

SEQ ID NO: 130 - DNA, 3216 bp, Artificial Sequence
  source: /note="Description of Artificial Sequence: Synthetic polynucleotide"
  source: /note="APG08290.1 mammalian codon optimized sequence"
atgagcgagctggattatagaatcggcctggatatcggcaccaattctatcggatggggagtgatcgagctgttctggaacaaggatcgggaacggtacgagaaggtccgcatcgtggacaaaggggtcagaatgtttgacaaggccgagatccccaacaagggcgccagcctggccgagcctcggagaatcgcccggagcagcagaagacgcctgaacaggaagtcccaaaggaagaaggagatccggaacctgctggtgcaacacggcatgatcacccaagaggaactggacctcctgtaccctctgagcaaaaagtccatcgatatctgggacatcagactagacggcctggacagactgctgaaccacttagagtgggctagactgctgattcacctggcccagcggcggggcttcaagagcaaccgcaaaagcgagctgaaggacgctgaaacaggcaaggtgttgtctagcatccaggtgaacgagaagcggctgttcctgtacagaaccgtgggggaaatgtggatcaaggacgcagagttcagcaagtacgacaggcgtagaaactccccaaacgaatacgtgttcagcgtgtcaagagccgacctggaaaaggaaatcgtgacactgtttgaggctcagagaaagttccagagcagctatgcctctaaaaatctgcaggagacctacctgcagatctgggcccaccaactgcctttcgccagcggcaatgccatcctgaacaaagtgggctactgcagcctgctgaaagggaaggaaaggcggattcccaaggccacatacaccttccagtacttctccgccctggatcaggttaaccggacccggctcggccctgacttccaacctttcacccaggaacaaaaggagatcatcctggataagatgttccagagaacagactactacaagaagaagaccatccccgaggtttcttattatgatatcagaaagtggctggaactcgacgagacaatccagtttaagggactgaattacgaccccaacgaagagctgaagaagatcgaaaaaaaacctttcatcaacctgaaggccttctacgagatcaagaaggtggttgctaactacgccgaaagaacaaatgaagccttttctaccctggactacgacgctatcgcctatgccctgacagtctacaagaccgacaaggacatccggtcctacctgaagaaatccaacaacctgtccaagcggtgctacgatgatcaactgatcgaggaactgtttaccctgagctacaccaaattcggccacctgtctttcaaggccattaaccacgtgctgcctatcatgcaggagggcagaacctaccaggaggccatacaccaactgggctacgacaccaccaacctgaagaaagagaatagaagcatgttcctgcctctgatccctgacgagatcacaaaccccattgtgaagcgggccatcacccaggccagaaaggtggtgaacgccatcatcagaagatacggctctcctaacagtgtgcacatcgaactggccagagagctgagcaagagccacgatgagcggaaaaagatcatgaccgcccacgacgagaactacaagaaaaataagggcgctatttctatcctgatcgagaacggcattctgaaccctaccggctacgacatcgtgagatacaagctgtggaaggaacaaggcgagagatgcgcctacagcctgaaagaaattccacctgatacttttttcaacgagctgaagaaagaaagaaacggcagccccattctggaagtggaccacatcctgccttacagccagtccttcatcgacagctaccacaacaaagtgctggtgtactctgacgagaacagaaacaagggcaacagaatcccttacacctacttcctggaaacaaacaaggactgggaggcctttgaaagatacgtgcggagtaacaaactgttttctaagaaaaagagagaatatctgctgaagaagacttacctgcctagagagtctgaactaatcaaggaacggcacctgaacgacactcggtatgcttctacattcctgaagaatttcatcgagcagaatctgcagttcaaagaggtcgaggtcaatctgagaaaaaagagagtgcaaaccgtgaatggcgtgatcaccgcccacctcagaaagcgttggggcctggagaagaaccggcaggagacgtacctgcaccacgctatggacgccatcatcgtggcttgtacagaccaccacatggtgacccggataacagagtactaccagatcaaggaatccaacaagagcgtgaagaaaccttacttccccatgccttgggagggctttagagatgagctgttgtctcacctcgctagccagcctatcgcaaagaagatcagcgaggaactgaaggccggctaccagagcagcgactacatcttcgtgtccagaatgcccaagagaagcgtgaccggcgccgcccatgatcagaccatcagaagaaagggcggcatcgacaagaagggcaagacaatcatcattaagcgggtgcggctgaaagatatcaagttcgacgaaaacggcgatttcaagatggtgggcaaagagcaggacctggcaacctacgaggccatcaagcagagatacctggagcacagaaagaacagtaagaaggccttcgagacccctctgtacaaacctagcaagaagggaacaggaaacctgattaagcgggtgaaaatcgagggacagactaaggccttcgtgcgggaagtgaacggaggcgtggcccaaaatagcgacctggtcagagtggacctgttcgagaaggacgacaagtactatatggtgcctatctacgtgccagacaccgtgtgtagcgagctgcctaagaaggtggttaagagcggaaaaggctatgagcagtggctgaccctggacaacagcttcaccttcaagtctagcctgtacccctacgatctggtgcggctcgtgaagggcaacgaggacagattcctgtacttcggcacactggacattgactccgatagactgaatttcaaggatgtgaacaagcccagcaagcagaacgagtaccggtacagcctgaaaacaatcgagaacctggaaaaatacgaggttggagtgctgggagatctgcggctggtgaaacaggagaccaggaggatctttaacaga

SEQ ID NO: 131 - DNA, 4011 bp, Artificial Sequence
  source: /note="Description of Artificial Sequence: Synthetic polynucleotide"
  source: /note="APG05459.1 mammalian codon optimized sequence"
atgaaaaaagattacgtgatcggcctggacattggcaccaacagcgtcggctgggccgtgatgacagaggactaccaactggtgaagaagaagatgccaatctatggcaatactgagaagaaaaagataaaaaagaatttctggggcgtgcggctgtttgaggagggccacaccgccgaggatcggcggctgaaacggaccgctagaagacggatctctcgccgcagaaatagactgagatatctgcaggccttcttcgaggaagccatgaccgccctggacgagaacttcttcgccagactgcaggagagcttcctggtgcctgaggacaagaaatggcaccggcaccctatcttcgccaagctggaggatgaggtggcctatcacgaaacctaccctacaatctaccacctgagaaagaaactggctgattcctctgaacaggctgacctgagactgatctatctggccctggcccatatcgtgaagtacagaggccacttcctgatcgaaggaaagctgagtaccgagaacatcagcgtcaaggagcagttccagcagttcatgattatctataaccagacatttgtgaacggcgaaagccggctggtgtctgcccctctgcctgagagcgtgctgatcgaagaagagctgaccgaaaaggccagccggacaaagaaatctgagaaggtgctgcaacagtttcctcaggagaaagccaatggactgttcggccagttcctgaaacttatggtaggcaacaaagccgatttcaagaaagtctttggcctggaagaagaggccaaaataacatacgccagcgagtcctacgaggaggatctggaaggcattctggccaaggtgggcgacgagtacagcgatgttttcctggccgctaagaacgtctacgacgccgtggaactgtctaccatcctggccgactccgacaagaagagccacgccaagttgtctagtagcatgatcgttagattcaccgagcaccaggaggacctgaagaagttcaagcggtttatcagagagaattgccccgacgagtacgataacctgttcaagaacgagcaaaaagacggctacgccggctacatcgcccacgccggcaaggtgtcccaactgaagttctaccagtacgtgaagaagataatccaggacatcgccggcgccgaatacttcctggagaaaatcgcccaggagaacttcctgcgaaaacagaggaccttcgacaacggcgtgatcccccaccagatccacctggccgagctgcaggccatcatccacagacaggctgcttactaccctttcctgaaggaaaatcaggaaaagattgagcaactggtgacattcagaatcccctactacgtcggccctctgagcaaaggagatgccagcaccttcgcctggctgaaaagacaaagcgaggaacctatccggccttggaacctgcaagagacagtggacctggaccagtctgctaccgcattcatcgagagaatgaccaacttcgatacctacctgccttctgagaaggtgctgcccaagcacagcctgctctacgaaaaatttatggtgttcaacgagctgaccaagatttcttacactgatgacagaggcatcaaggccaacttcagcggcaaggagaaggagaagatattcgactacctgtttaagacccgccggaaggtgaagaaaaaggatatcatccagttctaccggaacgagtacaacaccgagatcgtcaccctgtctggcctggaagaggaccagttcaatgccagcttcagcacctaccaagatctgctgaagtgcggcctaactagagccgaactggaccaccctgataatgccgagaaactggaggacatcattaagatcctaaccatcttcgaggatagacagcggatcagaacacagctcagcaccttcaagggacagttcagcgccgaggtgctgaagaagctggaacggaagcactacaccggctggggcagactgtccaagaaactcatcaacggcatctacgacaaggaatccggaaagacaatcctggactacctgatcaaagatgacggcgtttctaagcactacaacagaaacttcatgcagctaatcaacgacagccaactgagcttcaagaacgccatccagaaggcccagagcagcgagcatgaggaaaccctgtctgagaccgtgaacgagctggccggcagccctgccatcaagaaaggcatctaccagagcttaaaaatcgttgatgagctggttgccatcatgggctacgcccctaagagaatcgtggtggagatggctagagagaaccagacaacaagcaccggaaagagaagaagcatccagaggctgaagatcgtggaaaaagctatggccgagattggaagcaacctgctcaaggaacagcctaccacaaacgagcaactgagagatacaagactcttcctgtattatatgcagaacggtaaggacatgtacaccggcgacgagctgagcctgcacagactgtctcactacgacatcgaccacatcattcctcagtccttcatgaaggacgattccctggataacctggtgctggtgggcagcaccgagaaccggggcaagtctgacgacgtgcccagcaaggaagtggtgaaggacatgaaagcctactgggagaagctctacgctgctggcttgatcagccagcggaaattccagagactgacgaagggcgagcagggcggcctgaccctggaggacaaagctcatttcatccagagacaactggtggagacaagacagatcaccaagaacgtggctggaattctggatcagagatacaacgccaacagcaaagaaaaaaaggtgcaaatcataacactgaaagcctctctgaccagccagttccggagcatcttcggcctgtataaggtcagagaagtgaacgactatcaccacggccaggatgcgtacctgaactgcgtggtggccactacactcctgaaagtgtaccccaacctggctcctgagttcgtgtacggcgagtaccccaagtttcaggcctttaaggaaaacaaggctacagccaagaccatcatctacaccaatctgatgcggtttttcaccgaggatgaacccagattcatgaaggacggcgagatcctgtggagcaacagctacctgaagaacattaagaaagaactcaactaccatcagatgaacatagtgaaaaaggtggaagtgcaaaagggtggcttctccaaggaaagcatcaagcctaagggccccagcaacaagctgatccctgtgaagaacgggttggacccccagaaatacggcggatttgactctccagtggtcgcttacacagtgctgtttacccacgagaagggcaaaaaaccactgatcaagcaggagatcctgggaatcaccatcatggaaaagaccagattcgagcagaatcctatcctgttcctggaagaaaaaggcttcctgaggcctagagtgctgatgaagctgcctaaatacaccctgtacgagttccctgagggaagacggcggctgctggccagcgccaaagaagcccagaaagggaatcagatggtgctccccgaacacctgctgaccctgctgtaccacgccaaacagtgtctgctgcctaaccagagcgaatctctcgcttacgtggaacaacaccaaccggagttccaagagatcctggagagagtggtggacttcgctgaggtgcacacactggccaagagcaaggtgcaacagatcgtgaaactgtttgaggcaaaccagaccgcagatgtgaaggaaatcgccgcctccttcatccaactgatgcagttcaacgcaatgggagccccatctacctttaaattcttccagaaggacatcgagcgggcccggtacactagcatcaaggaaatcttcgacgccaccatcatctaccagagcacaaccggcctctacgagacacggagaaaggtggtggac

SEQ ID NO: 132 - DNA, 4308 bp, Artificial Sequence
  source: /note="Description of Artificial Sequence: Synthetic polynucleotide"
  source: /note="APG04583.1 mammalian codon optimized sequence"
atggccaagaatatcctgggcctggatctgggtacaaacagcatcggctgggctctggtccagcaggacttcgagaacaaggagggaaacatcctgggcatgggatctagaatcatccctatgagccaggacatcctgggcgaattcggtaagggcaacagcatcagccagaccgccgagagaacaggataccggggcgtgcgtagactgagagagagacacctcctgagaagagagagactgcatagagtgctgcacctgctcggctttctgcctaagcactacgatgaaaaaatcgactttacacaaagattcggcaagttcatcaaccaggctgagcctaagctggcttttgatagcgagttcctgttcaaggacagcttccacgagatgctggccgacttcaagcagaatcaacctgaattcctgaaagacaagaacggagaggactgcctggttccttacgactggaccatctactacctgagaaagaaggctctgacccagaagatcgagaaatacgaactagcttggctgatcctgaacttcaaccaaaagcggggctactaccagcttagaggcgaagaagagaaggaaaaccctaacaaactggtgggcttccactctctgaagattgttgatgtgatccctgatgccgagaccaacaaaaagggcgagacatggtacagcctgcacctggaaaacggctgggtgtacaggcggagcagcaagatcagcctggccgactggaaggacaaggttcgggacttcatcgtcactacagatctgaacgacgatggcagcgagaagctggacaaggacggcatcgtgaagaggtccttcagagccccttctgccgacgattggacactcctgaaaaaaaagactgagaaggacatcgacaactccaacaagactgtgggcacctacatctacgacaacttgctgctgaaccctaaacagaagatcaaggggaaaatggtcagaaccatcgaacgaaagttctacaagcaggagctggagcaaatcctgaaaacccagaaagaatttcactccgagctgcagtctgaaaacctgctgcaggactgcgtgagggagctgtaccggaacaacgagcagcaccagcagatgctggaagccaaggattttgtgcacctgttcctgaacgatatcatcttctaccagagacccctgcgcagccagaaaagctctattagcaactgcaccctggaattccggaagagcaagaacgagaatggagaagaagtgatccaccggctgaaggtgatcgccaagtccaacccctactatcaagagtttcggctgctgcagtgggtgcaaaacctggctatctacactaaggacgacgacaaaaacgtcacaaacgaattcctgaagagcacccaggactgggaggatctgctgagatggctgcacagcaagaaagaaatcaagcaggatgccctgatcaaattcctgatcgaaaagaaaggcctgaagggtaaggccctgaccattgaagtggctaagtacagatggaattacgtgcaagacaaggattatcctggcaacgagacaagatacctgattcagagccggctggacaaggtggaatacgcccctaaggacttcctcacgtacgaaaatgagatggccctgtggcacatcatctactctatcaacgataagatcgaatacgaaaaggccctaaagagcttcgccaacaagaaaggtctcgacgaggtgaccttcgtggaagcctttaagaaattcccacctttcaagagcgattacggcagcttcagcgagaaggccatcaagaagctgctgcctctcatgcggttcggcacacaatggaactgggacaacatcgaccagaactcgaaggaaaggattggaaaaatcctgaccggcgagtacgacgagaatatcaagggtagagtgcgggaaaaagctagacacctgaacagcgagacggactttcaggcgctccctctgtggctggcccagtacgtggtgtacggcagacatagcgaagctgacatcgccggcaagtggaatagtgtggacgacctgaagcagttcttggacgacttcaagcaacacagcctgagaaatcccattgtagaacaggtgattactgagacactgcgggccgtgaaggatatctggaacttctacggcaagggcgccaaggactttttctctgagatccacatcgagctgggaagagagatgaaaaacaccgccgacgagagaaaaaggattaccacaatggtgacagataatgagaataccaatctgagaatcaaagctctgctggctgagatggccctggatcagaacgtggacaatgtgcggccttacagccccatgcagcaagaaatcctgaaaatctatgaggaaggcgtgctgaacgccgaagagaacatcgacgatgacatcctgaagatctctaaaactgctcagcctagcgctaccgatctgaagagatacaagctgtggctggaacagaagtacagaagcccctataccggacagatgatccctctgaacaagctgttcacccctgagtatgaaatcgagcacattatcccccagagcagatacttcgacgattctatgagcaacaaggtgatctgcgaggccgccgtgaacaagctgaaggataaccagatcggcctggtgttcatcaagaaccaccacggcgaagtggtggactttggcatgggcaagcaggtgaaaatcctggaggtgtctgattacgaagatttcgtgaagcagaactacaacaaaaacagaggcaaacggaacaagctgctcctcgaagatatccccgagaaaatgattgaacggcaactgaacgataccagatatatcagcaagtacatcactcaggtgctgtctaatatcgtcagagacgacaaggaaggctctaaggatgacggagtgaacagcaagaacattgtgcccggcaacggcaagattacaaccagactcaagcaggattggggcctgaacgatgtgtggaacgacctggtgctgcctagattcgagagaatgaacaccctcacaaactccaatgattttacaagcaagaacacacacggcaagaccattcctaccgtgcctatcgagctgagcaaggggttcagcaaaaagcggatcgatcacagacaccacgctatggacgccctggtgatcgcctgcgccacccgggaccacgtgaacctgctgaataacgaatccagcaagtctgacacaaagcggtacgacctgaatagaaaactgagaaaatacgagaaggtggcctacaacgaccccaaaaccggcgagaggattgaaaaagaagtgccaaaagacttcatcaagccttgggaaacttttaccgaagataccagaacactgctggagaatatcgtgatctcattcaaacagaacctgagagtgatcaacaaggccaccaactactacgagaagatcgagaacggcaaaaaggtgaaggtggaacaaaagggaatcaactgggccgtgagaaaggctctccataaggagaccgtgtccggccaggtccaccttgacagaatcaaggtggccaagggcaagatcctgaccgccacaagaaagaccctggacgcttcttttaacgagaaaaccatagagagcatcaccgataccggcatccagaagatcctgctgaactacctgaagtcaaaggacaacaaccctgaggtggccttctccccagaaggaattgaggaactaaacaagaatatcagactgtacaatgacggcaaggcccaccagccaatcctaaaagtgcgggtgttcgagcagggcagcaagttcacactgggcgagacaggcaacaagacaaccaagttcgtggaagctgccaagggcaccaatcttttcttcggaatctacgaggacaagagcggaaaacgtagctacgagaccatccccctgaatatcgttattgaaagacagaaacagggcctccaggccgtgcccgagaccaacgagaagggcaagcaactgctgttcaccctgagccccaacgacctggtctacgtgccagaggaaggcgtattcgacgagaacaacatcaaggtggatagaatctacaaggtcgtgtctttcagcacataccaatgttttttcgtgcggaacgacgtatctaccagcgtggtcaacaaggtggagtacagcgccctgaacaagatggaaaaatccatcgacaatatcatgatcaaggaaaactgtgtgaagctgaatgtggaccggctgggtaagatcagcaaggcc

SEQ ID NO: 133 - DNA, 4368 bp, Artificial Sequence
  source: /note="Description of Artificial Sequence: Synthetic polynucleotide"
  source: /note="APG01688.1 mammalian codon optimized sequence"
atgatgatcaagaacattctgggactggatttgggcacaaacagcattggatgggctctgatcaagcaggacttcgagaacaaacacggcgagatcctgggcatgggcagcagaatcatccctatgagccaggatatcctgggcgatttcggcaaagggaactcgataagccagactgctgacagaaccaagtacagaagcgtgcggagactgagagaaagattcttgctgcggcgggaacgcctgcaccgggtgctccacctgctgaacttcctccctcaacactacgcctctcagatcgacttcgagaagaagttcggcaagtttaagtctgagaccgaacctaagctggcctgggaaaactggggaggtaaattctctttcctcttccagaacagcttcaacgagatgctggaagacttcaaggccgccggccagggactcaagattccctatgactggaccatctactacctacggaagaaagctctgtcccagaagatcgagaaagaggagcttgcctggattctgctgaacttcaaccagaagcgaggctactaccagctcagaggcgaggaagaagaagagaacccgaacaagctggtggagttctactccctgaagatcgtggatgtggtcgccgacgagcctcagaaggggaagagcgacatctggtattctctgatcctggaaaacggctgggtctaccgcagagccagtaagatcccactgtttgattggaaggataagaccagagatttcatcgtcaccacagaccttaatgacgacagaagcgtgaagaccgacaaagagggcaacgagaagcggtcctttcgggcccctagcgaaaatgattggaccctggtcaagaagaagacagagcaggagattgaccagagccacaagaccgtgggcacctacatctacgagacactgctgctcaatccaaagcagaaaatcaagggcaagctggtgcgaacaatcgagagaaaattttataaggacgagctgaagcaaatcctggaaaagcagaaggaatttcaccaggagctgaaaaacgacgatctgtacaacgactgcatcagagagctgtaccggaacaacgaggcccaccaactgaccctgagcaagaaagatttcgtgcacctgctgatggacgatctgatcttctaccaaagacccctgcgaagccagaagtccagcatctctaactgcaccctggaattcagaaaatacaaggacgaaaacggcatcgaacacacccagtacctgaaggccatcccaaagagtaatccgtactaccaagagtttagactgtggcagtggatgtacaacctgaacatctacagaaaggacgacgaggctaatgtgaccaaggaattcctgaacaccaataaggacttcgagagcctgtttgagttcctgaataatagaaaggaaatcgaacagaagcctctgatcaagttcctcctggaacagaaagatattaacaagaagctgctgaacgccgaggccgaaaagtatcggtggaattacgtggaagataagaagtatccttgcaacgaaacgaagaccatgatctccagcagactggacaaagtggagaatatctctgacgacttcctgaccagagacattgagcagaagatctggcacatcatctacagcgtcaacgacaagatagaatacgagaaggccctgaagtccttcgccaccagaaacgatctcgacgagaacagctttatcgaagcctttaagaagttcagcccattcaagagcgagtacggatctttttctgagaaagccatcaagaaactgctgcccctgatgagactgggaaagtactggtacgaggacgagattgtgaagcactctgatatttactttaagaacatcgaaaatcttctgggcgacttctccaacagagataaaaaaatatctgaggaagacaaagagaaatggaacaagtctatcaacctgaaactgcaggaggaactgaaggactttcagaccgccgagatcgacctgttccagggccttagactccatatcgcccagtacctggtgtacggccggcacagcgaagccagcatgatcggaaagtggaacagcgccgaggatctggaagaattcctgaaggacttcaagcagcacagcctgagaaaccccatcgtcgagcaagtgatcaccgagaccctgagggtggttaaggatatatggctgaaatacggcaacggcgccaaggacttcttcaacgagattcacatcgagctgggcagagaaatgaagctgcctgccgacgaccggaaaaagctgaccaaccagatcagcgagaacgaaaacacaaatttcagaatcaaggccctgctggctgaaatgatgaacgacagcagtgtggaaaatgtgcggcctttcagccctatgcagcaggagatcctgaagatctatgaagatgacgtcctgaagtctgacattgaaatcgaggatgacatccttaagatctctaaaaccgcccagccttctcctagcgatctcaagcgatacaagctctggctggagcagaagtacaagtctccatacaccggccagatcatacctctgaacaagctgtttacccctgaatacgagatcgagcacattatccctcagtctagatatttcgacgacagcttcagcaacaaagtgatctgcgagagcgccgtgaacaagctgaaagacaactacattggcctggaattcatcaagcaatttggaggcaccatcatcgaactgggctttggcaagtccatcaaagtgttcgagaccaaagagtacgaggacttcgtgaagaaacactacgccaacaatcagggcaagagaaacaagctgctcatggaagacatccccgagaaaatgatcgagagacagatgaacgacaccagatacatctctaagtacatcagcggagtgctgagcaacatcgtcagagtggaagatggatctgatgagggcgtgaacagcaagaacatcgtgcccggcaacggcaagattacaacacaactgaagcaggactggggcctgaatgacgtgtggaacgaccttatcctgccgcggttcgagagaatgaatcaactgaccaacagcaaggtgttcacagcctggaacgaaaactaccagaagttcctgcctacagtgccaatcgaatacagcaaaggcttcagcaagaagcgtatcgatcacagacaccacgccctggatgctctggttatcgcctgcgccaccaaggaccacgtgaacctgctgaacaaccagtctgccaagagcgacaccaagagatacgacttaaagaaaaaaagtatgaaattcgagaaagtggtgtacaatgatgccaagaccggcgaaaagatcgagcgggaagtgcccaagcagttcctgaagccttgggagaacttcaccctggatgtgaagcacaacctggaaacgatcatcgtctcttttaaacaaaatctgcgggtgatcaataaagccacgaactactacgagaagtacgtcgagaaggacggcaccaaaaacaaagagcgcgtggagcagacagggacaaactgggccattagaaagcccatgcacaaggatacagtgtccggcaaagtggaccttccttgggtgaaggtgcctaagggaaagatcctgaccgccacacggaagagcttggatagcagcttcgacctcaagagcatcggctctataacagatacaggcattcagaagatcctaaagaattacctggcattcaaggacggcaaccctgagctggctttcagccctgagggcatcgacgatctgaacaagaacatagagaagtacaacgatggcaaacctcaccagcctatcaacaaggtgcgagtgtttgagctgggcagcaagttccaggtgggacaatctggtaacaagaaggacaagtatgtggaagctgctaagggcaccaatctcttcttcgccgtgtacgaggatgaaaaaggaaagcggaactacgagaccatccctctcaacgaggtgatcgagagacagaagcagggcctgagcgtggtggacctgaagggtacaaacgacttctacctgtgccctaacgactttgtgtacatcccaagcggcgacgagctggaaaacatcaacaacgtggacttcaaggacatcaagaaggagattaacgagcgcatctacaaagtggtgtcttttacaggcaatagactttcttgtatcccttacatggtggccacaacgatcgtcaacaaactcgaattcactcaactgaacaaaatcgagtttaccaaggaaaaagaaatttgtatcaagctcaacgtggacagactgggcaatatctccaaggcc

SEQ ID NO: 134 - DNA, 21 bp, Artificial Sequence
  source: /note="Description of Artificial Sequence: Synthetic oligonucleotide"
  source: /note="SV40 large T-antigen nuclear localization sequence"
cctaagaagaaaagaaaggtg

SEQ ID NO: 135 - DNA, 66 bp, Artificial Sequence
  source: /note="Description of Artificial Sequence: Synthetic oligonucleotide"
  source: /note="Triple FLAG epitope tag"
gactacaaggaccacgacggcgactacaaagatcacgatatcgactacaaggacgacgatgataag

SEQ ID NO: 136 - DNA, 48 bp, Artificial Sequence
  source: /note="Description of Artificial Sequence: Synthetic oligonucleotide"
  source: /note="Nucleoplasmin nuclear localization sequence"
aaaagacctgccgctacaaagaaggccggccaggccaagaaaaagaag

SEQ ID NO: 137 - DNA, 203 bp, Artificial Sequence
  source: /note="Description of Artificial Sequence: Synthetic polynucleotide"
  source: /note="Cytomegalovirus mammalian transcription promoter"
tgatgcggttttggcagtacatcaatgggcgtggatagcggtttgactcacggggatttccaagtctccaccccattgacgtcaatgggagtttgttttggcaccaaaatcaacgggactttccaaaatgtcgtaacaactccgccccattgacgcaaatgggcggtaggcgtgtacggtgggaggtctatataagcagagct

SEQ ID NO: 138 - DNA, 304 bp, Artificial Sequence
  source: /note="Description of Artificial Sequence: Synthetic polynucleotide"
  source: /note="Cytomegalovirus transcription enhancer"
cgttacataacttacggtaaatggcccgcctggctgaccgcccaacgacccccgcccattgacgtcaataatgacgtatgttcccatagtaacgccaatagggactttccattgacgtcaatgggtggagtatttacggtaaactgcccacttggcagtacatcaagtgtatcatatgccaagtacgccccctattgacgtcaatgacggtaaatggcccgcctggcattatgcccagtacatgaccttatgggactttcctacttggcagtacatctacgtattagtcatcgctattaccatg

SEQ ID NO: 139 - DNA, 318 bp, Artificial Sequence
  source: /note="Description of Artificial Sequence: Synthetic polynucleotide"
  source: /note="Human U6 RNA promoter"
tgtacaaaaaagcaggctttaaaggaaccaattcagtcgactggatccggtaccaaggtcgggcaggaagagggcctatttcccatgattccttcatatttgcatatacgatacaaggctgttagagagataattagaattaatttgactgtaaacacaaagatattagtacaaaatacgtgacgtagaaagtaataatttcttgggtagtttgcagttttaaaattatgttttaaaatggactatcatatgcttaccgtaacttgaaagtatttcgatttcttggctttatatatcttgtggaaaggacgaaacacc

SEQ ID NO: 140 - DNA, 20 bp, Artificial Sequence
  source: /note="Description of Artificial Sequence: Synthetic oligonucleotide"
  source: /note="target for Guide 189"
cctgaatgctgtgcggctct

SEQ ID NO: 141 - DNA, 20 bp, Artificial Sequence
  source: /note="Description of Artificial Sequence: Synthetic oligonucleotide"
  source: /note="target for Guide 185"
ggacagtgcgcatctccctg

SEQ ID NO: 142 - DNA, 20 bp, Artificial Sequence
  source: /note="Description of Artificial Sequence: Synthetic oligonucleotide"
  source: /note="target for Guide 168"
cacatctcgagcaagacgtt

SEQ ID NO: 143 - DNA, 20 bp, Artificial Sequence
  source: /note="Description of Artificial Sequence: Synthetic oligonucleotide"
  source: /note="target for Guide 135"
gggccattaaaacctctcca

SEQ ID NO: 144 - DNA, 20 bp, Artificial Sequence
  source: /note="Description of Artificial Sequence: Synthetic oligonucleotide"
  source: /note="target for Guide 139"
aggttttaatggcccagcct

SEQ ID NO: 145 - DNA, 20 bp, Artificial Sequence
  source: /note="Description of Artificial Sequence: Synthetic oligonucleotide"
  source: /note="target for Guide 143"
catggcagtacattagagca

SEQ ID NO: 146 - DNA, 20 bp, Artificial Sequence
  source: /note="Description of Artificial Sequence: Synthetic oligonucleotide"
  source: /note="target for Guide 190"
cctgaatgctgtgcggctct

SEQ ID NO: 147 - DNA, 20 bp, Artificial Sequence
  source: /note="Description of Artificial Sequence: Synthetic oligonucleotide"
  source: /note="target for Guide 194"
gccgcacagcattcaggtcg

SEQ ID NO: 148 - DNA, 20 bp, Artificial Sequence
  source: /note="Description of Artificial Sequence: Synthetic oligonucleotide"
  source: /note="target for Guide 165"
atggggaatgtagcaagacc

SEQ ID NO: 149 - DNA, 20 bp, Artificial Sequence
  source: /note="Description of Artificial Sequence: Synthetic oligonucleotide"
  source: /note="target for Guide 169"
cacatctcgagcaagacgtt

SEQ ID NO: 150 - DNA, 20 bp, Artificial Sequence
  source: /note="Description of Artificial Sequence: Synthetic oligonucleotide"
  source: /note="target for Guide 173"
cttctatagcctccttcccc

SEQ ID NO: 151 - DNA, 20 bp, Artificial Sequence
  source: /note="Description of Artificial Sequence: Synthetic oligonucleotide"
  source: /note="target for Guide 144"
catggcagtacattagagca

SEQ ID NO: 152 - DNA, 20 bp, Artificial Sequence
  source: /note="Description of Artificial Sequence: Synthetic oligonucleotide"
  source: /note="target for Guide 136"
gggccattaaaacctctcca

SEQ ID NO: 153 - DNA, 20 bp, Artificial Sequence
  source: /note="Description of Artificial Sequence: Synthetic oligonucleotide"
  source: /note="target for Guide 145"
catggcagtacattagagca

SEQ ID NO: 154 - DNA, 20 bp, Artificial Sequence
  source: /note="Description of Artificial Sequence: Synthetic oligonucleotide"
  source: /note="target for Guide 188"
ggacagtgcgcatctccctg

SEQ ID NO: 155 - DNA, 20 bp, Artificial Sequence
  source: /note="Description of Artificial Sequence: Synthetic oligonucleotide"
  source: /note="target for Guide 192"
cctgaatgctgtgcggctct

SEQ ID NO: 156 - DNA, 20 bp, Artificial Sequence
  source: /note="Description of Artificial Sequence: Synthetic oligonucleotide"
  source: /note="target for Guide 196"
gccgcacagcattcaggtcg

SEQ ID NO: 157 - DNA, 20 bp, Artificial Sequence
  source: /note="Description of Artificial Sequence: Synthetic oligonucleotide"
  source: /note="target for Guide 167"
atggggaatgtagcaagacc

SEQ ID NO: 158 - DNA, 20 bp, Artificial Sequence
  source: /note="Description of Artificial Sequence: Synthetic oligonucleotide"
  source: /note="target for Guide 171"
cacatctcgagcaagacgtt

SEQ ID NO: 159 - DNA, 20 bp, Artificial Sequence
  source: /note="Description of Artificial Sequence: Synthetic oligonucleotide"
  source: /note="target for Guide 175"
cttctatagcctccttcccc

SEQ ID NO: 160 - DNA, 25 bp, Artificial Sequence
  source: /note="Description of Artificial Sequence: Synthetic oligonucleotide"
  source: /note="target for Guide 197"
cctcacccccacgagcttgtaggaa

SEQ ID NO: 161 - DNA, 25 bp, Artificial Sequence
  source: /note="Description of Artificial Sequence: Synthetic oligonucleotide"
  source: /note="target for Guide 199"
acagtgcgcatctccctggtcacca

SEQ ID NO: 162 - DNA, 25 bp, Artificial Sequence
  source: /note="Description of Artificial Sequence: Synthetic oligonucleotide"
  source: /note="target for Guide 146"
ggctgggccattaaaacctctccag

SEQ ID NO: 163 - DNA, 25 bp, Artificial Sequence
  source: /note="Description of Artificial Sequence: Synthetic oligonucleotide"
  source: /note="target for Guide 148"
gaggctgggccattaaaacctctcc

SEQ ID NO: 164 - DNA, 25 bp, Artificial Sequence
  source: /note="Description of Artificial Sequence: Synthetic oligonucleotide"
  source: /note="target for Guide 176"
gaggctgagacaggagagttgcttg

SEQ ID NO: 165 - DNA, 25 bp, Artificial Sequence
  source: /note="Description of Artificial Sequence: Synthetic oligonucleotide"
  source: /note="target for Guide 177"
cccacaaaccgatgtagctcaagag

SEQ ID NO: 166 - DNA, 25 bp, Artificial Sequence
  source: /note="Description of Artificial Sequence: Synthetic oligonucleotide"
  source: /note="target for Guide 209"
tagggtcttactctgttgtccacgc

SEQ ID NO: 167 - DNA, 25 bp, Artificial Sequence
  source: /note="Description of Artificial Sequence: Synthetic oligonucleotide"
  source: /note="target for Guide 151"
ttctcccgagccaagtacacgtttc

SEQ ID NO: 168 - DNA, 25 bp, Artificial Sequence
  source: /note="Description of Artificial Sequence: Synthetic oligonucleotide"
  source: /note="target for Guide 152"
gaaaatctgctcttagggctcaagg

SEQ ID NO: 169 - DNA, 3210 bp, Artificial Sequence
  source: /note="Description of Artificial Sequence: Synthetic polynucleotide"
  source: /note="APG05083.1 Soy optimized"
atgagagagctagattacaggatcggactcgatatcggaactaattcaatcgggtggggaataattgagctgtcctggaataaagatcgcgagcaatatgaaaaggctaggattgtggataagggagtgaggatgttcgataaggctgaaattcctaagactggagcttctcttgctgaaccaagaagaattgctagatctagcaggaggagattaaacaggaagtctcagcgcaagaaggatataaggaaccttctcgttcagcatgaaatcatttctcagaaggagcttgcttctctctaccctctaaccaaatcaagcatggacatctgggatataaggcttgatggactcgataggcttcttgatagatttgagtggaccaggcttctaatacaccttgctcaaagaaggggcttcaaatcaaaccgcaagtccgaattaaaggatgttgagactggaaaggtgctttcaagcatccaagctaatgaaaagaggctttctttgtacaggactgttggggagatgtggatgaaaaacgaggacttctcaaaatacgataaaaggaggaactcctccaacgagtacgtgttctctgtttctagggctgatcttgagaaggagattgtgactctttttgaggctcaacgcaagttccaatcaagctacgcttctgctgatcttcaaaagacctaccttcaaatttgggctcatcagcttccttttgcttctggaaacgccattgtgaataaagtgggatactgctccctattaaagggaaaggagaagagagtgcctaaggctacctatacattccagtacttctctaccctcgatcaaatcaatagaactaggcttggacctaacttccagccttttactaaggagcagagggatgtgatcctcgatgaaatgttcaacaggaccgactactataaaaagaagaccattcccgaggtgacctactacgatataagaaagtggcttgctctcgatgaaaccattcagttcaagggactaacttatgaccccaacgaggagctgaagaaaatagaactcaagtccttcataaacctcaagcccttctacgaaatcaagaaggtggtaaccaactacgccaagaagaccaacgaagcattctctaccctcgattacgatacattcgcttacgctcttaccgtgtataaaaccgacaaggatataaggtcctacctcaagaaatcaaacaacctctccaagtgctgctacgacgatcaattaattgaggagcttctcaccctctcctatactaagttcggacacctctctttcaaggcaatcaaccatgtgcttccaataatgcaagagggaagaacttaccaagaggcaatacaccaacttggatacgatgctaccaaccttaagaaggagaacaggtctatgttccttcctctcttccctgatgagattactaaccctattgtgaagagagctttgactcaagctaggaaggtggtgaatgctattattaggaggtacggatcacctaactctgtgcatattgagcttgctagggagctttctaagtctcatgatgagaggaccaagattatgaaggctcacgatgagaactacaagaagaacaagggggctatttccattctcattgagaacggaattcttaaccctaccggatacgatattgtgaggtacaagttgtggaaggagcaaggagagagatgcgcttactctcttaagcaaattcctgctaacaccttcttcaacgagatgaagaaggaaagatcaggatctcctgtgcttgagattgatcacattctcccttactcccagtccttcattgattcttaccacaacaaggtgcttgtttacggagatgagaaccaaaagaaggggaacaggattccttacacttacttccttgagggaaacaaggattgggagtctttcgagtcttacgtgaggcttaactccttcttctctaagaagaagaggggataccttcttaagaaggcttatcttcctagggagtccaatatgattaaggagaggcacctaaacgataccaggtacgcttcttcttacctcaagaacttcatcgagaagaaccttaagttcaaggaggttgagggatctactaggaagaagcatgttcagaccgtgaacggaattattactgctcatcttagaaagaggtggggacttgagaaggataggcaagagacttaccttcatcacgctatggatgctattattgtggcttgcactgatcaccatatggtgactaaggttaccgagtactaccagattaaggagtcaaacaagtccatcaggaagccttattttcctcttccttgggttggattcagggaggagattctttctcatcttgctagacaacctatcgctagaaagatttccgaggagcttaagattggataccagtccttcgattacattcttgtgtctaggatgcctaagaggtctgttactggagctgctcatgagcagactattatgaagaagggaggaattgataagaaggggaagaccatcatcattaagagggtgtacctaaaggacatcaagttcgatgagaacggggatttcaagatggttggaaaggagcaggatcttgctacttacgaggctattaagcagaggtacattgagtatggaaaggagtctaagaaggctttcgagactcctctttacaagccttctaagaagggaaaggggaacctcatcaagaagattaaggttgaggttcagactaagtctttcgttagggaggttaatggaggagttgctcagaatggagatcttgtgagggttgatctattcgagaaggacaacaggtactacatgatccctatctacgtgatggatactgttcattccgagcttcctaacaaggctgttacttcttctaagggatacgagcagtggcttaccattgataactctttcaccttcaagttctctctctacccttacgatcttgttaggcttgttaagggaaacgaggataggttcctctacttctccaccctcgatattaactctgataggctcaacttcaaggatgtgaacaagccttcaaagcaagctgagaacaggtactctcttaagaccattgagaaccttgagaagtacgaagtgggagttcttggagatcttaggttcgttaggcaagagattaggaagaacttc

SEQ ID NO: 170 - DNA, 3210 bp, Artificial Sequence
  source: /note="Description of Artificial Sequence: Synthetic polynucleotide"
  source: /note="APG05083.1 Corn optimized"
atgcgcgagctagattacaggatcggcctggatatcggcactaactcaataggctggggcatcatcgagctgagctggaataaagaccgcgagcagtatgaaaaggccaggatcgtggacaagggcgtgaggatgttcgataaggccgagatcccaaagacaggcgcctctctggccgaaccaaggaggatcgccaggtcttctaggaggagattaaacaggaagtctcagcgcaagaaggatataaggaacctgctggtccagcatgaaatcatctctcagaaggagctggccagcctgtacccgctgaccaagtcaagcatggacatctgggatataaggctggatggcctggataggctgctggataggttcgagtggacaaggctgctgatacatctggcccagaggaggggcttcaaatcaaataggaagagcgaattaaaggacgtggagacaggcaaggtgctgtcaagcattcaggccaatgaaaagcgcctgagcctgtacaggacagtgggcgagatgtggatgaaaaacgaggacttctcaaaatacgacaagcgccgcaacagcagcaacgagtacgtgttcagcgtgagcagggccgacctggagaaggagatcgtgacactgttcgaggcccagaggaagttccaatcaagctacgcctctgccgatctgcagaagacatacctgcagatctgggcccaccagctgccattcgctagcggcaatgccatcgtgaataaagtgggctactgctctctattaaagggcaaggagaagagggtgccaaaggccacctatacattccagtacttcagcaccctggaccaaatcaataggacacgcctgggcccaaacttccagccattcacaaaggagcagcgcgacgtgatcctggatgaaatgttcaaccgcaccgactactataaaaagaagaccatcccggaggtgacatactacgatataaggaagtggctggccctggatgaaaccatccagttcaagggcctaacctacgacccgaacgaggagctgaagaaaatagaactgaagagcttcataaacctgaagccgttctacgaaatcaagaaggtggtaaccaactacgccaagaaaaccaacgaagcattcagcaccctggactacgatacattcgcctacgccctgaccgtgtataaaaccgacaaggatataaggagctacctgaagaaatcaaacaacctgagcaagtgctgctacgacgaccaattaatcgaggagctgctgaccctgagctatactaagttcggccacctgagcttcaaggcaatcaaccacgtgctgccaataatgcaggagggccgcacctaccaggaggcaatacaccagctgggctacgacgcaaccaacctgaagaaggagaaccgaagcatgttcctgccgctgttcccggacgagatcaccaacccgatcgtgaagcgcgccctgacccaggcccgcaaggtggtgaacgccatcatccgccgctacggctcaccgaacagcgtgcacattgagctggcccgcgagctgagcaagagccacgacgagcgcacaaagatcatgaaggcccacgacgagaactacaagaagaacaagggcgccatcagcatcctgatcgagaacggcatcctgaacccaacaggctacgacatcgtgaggtacaagctgtggaaggagcagggcgagaggtgcgcctactctctgaagcagatcccagccaatacattcttcaacgagatgaagaaggagaggtcaggctctccagtgctggagattgatcacatcctgccatacagccagagcttcatcgacagctaccacaacaaggtgctggtgtacggcgatgagaaccagaagaagggcaatcgcatcccatacacatacttcctggagggcaacaaggattgggagagcttcgagagctacgtgaggctgaacagcttcttcagcaagaagaagaggggctacctgctgaagaaggcctacctgccaagggagagcaacatgatcaaggagaggcacctaaacgatacaaggtacgccagcagctacctgaagaacttcatcgagaagaacctgaagttcaaggaggtggagggcagcacccgtaagaagcacgtccagaccgtgaacggcatcatcacagcccacctgaggaagaggtggggcctggagaaggataggcaggagacatacctgcatcacgccatggatgccatcatcgtggcttgcacagatcaccacatggtgacaaaggtgacagagtactaccagatcaaggagagcaacaagtcaatccgcaagccatacttcccactgccatgggtgggcttcagggaggagatcctgtctcacctggccaggcagccaatcgccaggaagatctctgaggagctgaagatcggctaccagtctttcgattacatcctggtgtctaggatgccaaagaggtctgtgacaggcgccgcccacgagcagacaatcatgaagaagggcggcatcgataagaagggcaagacaatcatcatcaagagggtgtacctgaaggatatcaagttcgatgagaacggcgatttcaagatggtgggcaaggagcaggatctagccacatacgaggccatcaagcagaggtacatcgagtacggcaaggagtctaagaaggccttcgagacaccactgtacaagccatctaagaagggcaagggcaacctgatcaagaagatcaaggtggaggttcagaccaagagcttcgtgagggaggtgaatggcggcgtggcccagaatggcgatctggtgagggtggatctgttcgagaaggataacaggtactacatgatcccgatctacgtgatggatacagtgcacagcgagctgccaaacaaggccgtgacatcttctaagggctacgagcagtggctaaccatcgacaacagcttcaccttcaagttcagcctgtacccatacgacctggtgaggctggtgaagggcaatgaggacaggttcctgtacttcagcaccctggacatcaacagcgacaggctgaacttcaaggacgtgaacaagccatctaagcaggccgagaacaggtacagcctgaagaccatcgagaacctggagaagtacgaggtgggcgtgctgggcgatctgaggttcgtgaggcaggagatcaggaagaatttc

SEQ ID NO: 171 - DNA, 3213 bp, Artificial Sequence
  source: /note="Description of Artificial Sequence: Synthetic polynucleotide"
  source: /note="APG07433.1 Soy optimized"
atgagagagctagattacaggatcggactcgatatcggaactaattcaattggatggggcgtgattgagctttcctggaataaagatagggagcgttatgaaaaggttaggattgtggatcagggagttaggatgtttgatagagctgagatgcctaagactggagcttcattagctgaaccaagaaggattgctagatctagcaggaggagattaaacaggaagtctcagcgcaagaagaatataaggaaccttcttgttcagcacggagttattactcaggaggagcttgattctctctaccctctctccaagaaatcaatggatatctggggaattaggcttgatggactcgatcgcctattaaaccattttgagtgggctaggcttctaatacaccttgctcaaagaaggggcttcaaatcaaaccgcaagtccgaattaaaggatactgagactggaaaggtgctttcaagcatccagctcaatgaaaagaggctttctttgtataggactgttggggagatgtggatgaaagatcccgacttctcaaaatacgataggaagaggaactctcctaacgagtacgtgttttctgtttctagagctgagcttgagaaggagattgtgactttgtttgctgctcaaaggaggttccaatctccttacgcttctaaggatcttcaagagacctaccttcagatttggactcatcagcttccttttgcttccgggaacgctattctcaataaagtgggatactgctccttattaaagggaaaggagagaaggattcctaaggccacctatacattccagtacttctctgctcttgatcaagtgaatagaactaggcttggacctgatttccagccttttactaaggagcagcgcgagatcatcctcaataatatgttccagaggaccgactactataaaaagaagaccattcccgaggtgacctactacgatataagaaagtggcttgagcttgatgaaaccattcagttcaagggattaaactacgaccccaacgaggagctgaagaaaatagagaagaagcccttcataaacctcaaggccttctacgaaatcaacaaggtggtggctaactactctgagcgaaccaatgaaaccttctctaccctcgattacgatggaattggatacgctcttaccgtgtataaaaccgacaaggatataaggtcctacctcaaatcaagccataatctccctaagaggtgctacgacgatcaattaattgaggagcttctctccctctcctatactaagttcgggcacctctctcttaaggcaatcaaccatgttctaagcattatgcagaaggggaacacatataaggaggctgttgatcagcttggatacgatacttctggacttaagaaggagaagaggtctaagttcctccctcctatttctgatgagattaccaaccctattgtgaagagagctttgactcaagctaggaaggtggtgaatgctattattaggaggcatggatctcctcattctgtgcatattgagcttgctagggagctttcaaagaatcacgatgagaggactaagattgtttctgctcaggacgagaactacaagaagaacaagggggctatttctattctctctgagcacggaattcttaaccctaccggatacgatattgtgaggtataagttgtggaaggagcaaggagagagatgcgcttactctcttaaggaaattcctgctgataccttcttcaacgagcttaagaaggaaaggaacggtgctcctattctagaggtggatcacattcttccttactcccagtccttcattgattcttaccataacaaggtgcttgtgtattccgatgagaacaggaagaagggaaacaggattccttacacctacttccttgagactaataaggattgggaggcttttgagaggtacgtgaggtctaacaagttcttctctaagaagaagagggagtaccttcttaagagggcttatcttcctagggagtcagagcttattaaggagaggcatcttaacgataccaggtacgcttctaccttcctcaagaacttcattgagcagaaccttcaattcaaggaagctgaggataatcctagaaagaggagggttcagactgtgaacggagttattactgctcattttagaaagaggtggggacttgagaaggataggcaagagacttaccttcatcacgctatggatgctattattgtggcttgcactgatcatcatatggtgactagggttaccgagtactaccagatcaaggagtcaaacaagtctgtgaagaagccttattttcctatgccttgggaaggattcagggatgagcttctttctcatcttgcttctcagcctatcgctaagaagatttctgaagagcttaaggctggataccagtcccttgattacattttcgtgtctagaatgcctaagaggtctattactggagctgctcacaagcagactattatgaggaagggaggaattgataagaaggggaagaccatcattattgagaggctccacctcaaggatatcaagttcgatgagaacggagatttcaagatggttggaaaggagcaggatatggctacttacgaggctattaagcagagatatctagagcacggaaagaactctaagaaggctttcgagactcctctttacaagccttctaagaagggaaccggaaaccttattaagagagttaaggttgagggacaggctaagtctttcgttagagaggttaatggaggagttgctcagaatggagatcttgtgagggttgatcttttcgagaaggacgataagtactacatggtgcctatctacgttcctgatactgtttgttccgagcttcctaagaaggttgttgcttcttctaagggatacgagcaatggcttacccttgataactctttcaccttcaagttctctctctacccttacgatcttgttaggctagttaagggagatgaggataggttcctttacttcgggaccctcgatattgattctgataggctcaacttcaaggatgtgaacaagccttctaagaagaacgagtacaggtactctctcaagaccattgaggatcttgagaagtacgaagtgggagttcttggagatcttagacttgttagaaaggagactaggaggaacttccac

SEQ ID NO: 172 - DNA, 3213 bp, Artificial Sequence
  source: /note="Description of Artificial Sequence: Synthetic polynucleotide"
  source: /note="APG07433.1 Corn optimized"
atgcgcgagctagattacaggatcggcctggatatcggcactaactcaatcggctggggcgtgatcgagctgagctggaataaagatcgcgagcgctatgaaaaggtgcgcatcgtggatcagggcgttaggatgttcgatagggccgagatgccaaagacaggcgcctcactggccgaaccaaggaggatagccaggtcttctaggaggagattaaacaggaagtctcagcgcaagaaaaatatcaggaacctgctggttcagcacggcgtgatcacacaggaggagctggattctctgtacccactgagcaagaaaagcatggacatctggggcattaggctagatggcctggaccgcctattaaaccacttcgagtgggcccgcctattaattcacctggcccagaggaggggcttcaaatcaaataggaagagcgaattaaaggacaccgagacaggcaaggtgctgtcaagcatccagctgaatgaaaagcgcctgagcctgtacaggacagtgggcgagatgtggatgaaagacccggacttctcaaaatacgaccgcaagcgcaacagcccgaacgagtacgtgttctctgtgtctagggccgagctggagaaggagatcgtgacactgttcgccgctcagaggaggttccagtctccatacgcctctaaggatctgcaagagacatacctgcagatctggacacaccagctgccattcgcctctggcaatgccatcctgaataaagtgggctactgctctctattaaagggcaaggagaggaggattccaaaggccacctatacattccagtacttcagcgccctggaccaggtgaataggacaaggctgggcccagatttccagccattcacaaaggagcagcgcgagatcatcctgaataatatgttccagcgcaccgactactataaaaagaagaccatcccggaggtgacatactacgatataaggaagtggctggagctggatgaaaccatccagttcaagggattaaactacgacccgaacgaggagctgaagaaaatagagaagaagccgttcataaacctgaaggccttctacgaaatcaacaaggtggtggccaactacagcgagcgaaccaacgagaccttcagcaccctggactacgacggcatcggctacgccctgaccgtgtataaaaccgacaaggatataaggagctacctgaaatcaagccacaacctgccgaagcgctgctacgacgaccaattaatcgaggagctgctgagcctgagctatactaagttcggccacctgagcctgaaggcaatcaaccacgtgctaagcatcatgcagaagggcaatacatacaaggaggccgtggaccagctgggctacgacaccagcggcctgaagaaggagaagcgcagcaagttcctgccgccgatcagcgacgagatcaccaacccgatcgtgaagcgcgccctgacccaggccaggaaggtggtgaacgccatcatcaggaggcacggctctccacatagcgtgcacatcgagctggccagggagctgtctaagaatcacgatgagaggacaaagatcgtgtcagcccaggacgagaactacaagaagaataagggcgccatctctatcctgtctgagcacggcatcctgaacccaacaggctacgacatcgtgaggtacaagctgtggaaggagcagggcgagaggtgcgcctactctctgaaggagatcccagccgatacattcttcaatgagctgaagaaggagaggaatggcgccccaatcctggaggtggatcacatcctgccatactctcagagcttcatcgattcataccacaacaaggtgctggtgtacagcgacgagaacaggaagaagggcaatcgcatcccatacacatacttcctggagaccaacaaggattgggaggccttcgagaggtacgtgcgcagcaacaagttcttcagcaagaagaagcgcgagtacctgctgaagagggcctacctgcctagggagtctgagctgatcaaggagaggcacctgaatgatacaaggtacgccagcaccttcctgaagaacttcatcgagcagaacctacagttcaaggaggccgaggataacccaaggaagaggagggttcagacagtgaatggcgtgatcacagcccacttcaggaagaggtggggcctggagaaggataggcaggagacatacctgcatcacgccatggatgccatcatcgtggcttgcacagatcaccacatggtgacaagggtgacagagtactaccagatcaaggagagcaacaagagcgtgaagaagccatacttcccaatgccatgggagggcttcagggatgagctactgtctcacctggcctctcagccaatcgccaagaagatctctgaggagctgaaggccggctaccagtctctggattacatcttcgtgtctaggatgccaaagaggtctatcacaggcgccgcccacaagcagacaatcatgaggaagggcggcatcgataagaagggcaagacaatcatcatcgagaggctgcatctgaaggacatcaagttcgatgagaacggcgatttcaagatggtgggcaaggagcaggatatggccacatacgaggccatcaagcagcgctacctagagcacggcaagaactctaagaaggccttcgagacaccactgtacaagccatctaagaagggcaccggcaatctgatcaagagggtgaaggtggagggccaggccaagtctttcgtgagggaggtgaatggcggcgtggcccagaatggcgatctggtgagggtggatctgttcgagaaggatgataagtactacatggtgccaatctacgtgccagatacagtgtgctctgagctgccaaagaaggtggtggcctcttctaagggctacgagcagtggctaacactggataacagcttcacattcaagttcagcctgtacccatacgatctggtgaggctggtgaagggcgatgaggataggttcctgtacttcggcacactggatatcgatagcgacaggctgaacttcaaggacgtgaacaagccgagcaagaagaacgagtaccgctacagcctgaagacaatcgaggacctggagaagtacgaggtgggcgtgctgggcgatctgaggctggtgaggaaggagacaaggaggaatttccac

SEQ ID NO: 173 - DNA, 3213 bp, Artificial Sequence
  source: /note="Description of Artificial Sequence: Synthetic polynucleotide"
  source: /note="APG07513.1 Soy optimized"
atgagagagctagattacaggatcggactcgatatcggaactaattcaattggatggggcgtgattgagctttcctggaataaagatcgcgagcaatatgaaaagaccaggattgtggataagggagtgaggatgttcgataaggctgaaattcctaagactggagcttctcttgctgaaccaagaagaattgctagatctagcaggaggagattaaacaggaagtctcagcgcaagaaggatataaggaaccttctcgttcagcatgaaatcatttcccagaaggaattaacctctctctaccctctctccaaatcaagcatggacatctgggatataaggcttgatggactcgataggcttcttgatagatttgagtgggctaggcttctaatacaccttgctcaaagaaggggcttcaaatcaaaccgcaagtccgaattaaaggatgttgagactggaaaggtgctttcaagcatccaggtgaatgaaaagaggctttctttgtataggactgttggggagatgtggatgaaaaacgccgattgctcaaaatatggaaagaggaggaactctcctaacgagtacgtgttttctgtttctagggctgatcttgagaaggagattgtgactctttttgaggctcagaggaagttccactcttcttacgcttctgtggatctccaaaagacatacattcagatttgggctcatcagcttccttttgcttctggaaacgccattgtgaataaagtgggatactgctccctattaaagggaaaggagaagagagtgcctaaggctacctatacattccagtacttcaataccctcgatcaaatcaacagaactaggcttggacctaacttccagccttttactaaggagcagagggatataatcctcgataaaatgttccagcgcaccgactactataaaaagaagaccatccccgaggtgacctactacgatataagaaagtggcttgctctcgatgaaaccattcagttcaagggactaacttatgaccccaacgaggagctgaagaaaatagagatgaaacccttcataaacctcaagcccttctacgaaatcaagaaggtggtaaccaactacgccaagaaaaccaacgaggtgttctctgctcttgattacgatactgtggcttacgctcttaccgtgtataaaaccgacaaggatataaggtcttacctcaagcgctccaataatctctctaagaggtgctacgacgatcaattaattgaggagcttctcaccctctcctatactaagttcggacacctctctttcaaggcaatcaaccatgtgcttccaataatgcaagagggaagaacttaccaagaggcaatacaccagcttggatacgatacaaccaacctcaagaaggagaatagaagcatgttcctcccaatcatccctgatgaaataaccaaccctattgtgaagagagctttgactcaagctaggaaggtggtgaatgcaataattaggaggtacggatcacctaactctgtgcatattgagcttgccagggaattaagcaagtctcatgatgagaggaagaagattatgactgctcacgacgagaactacaagaagaacaagggagctgtgtccattctcattgataacggaattcttaaccctaccggatacgatattgtgaggtacaagttgtggaaggagcaaggagagagatgcgcttactctcttaagaagattcctgctaacaccttcttcaacgagcttaagaaggaaagatctggacctcctgttcttgaggtggatcacattctaccttactcccagtccttcattgattcttaccataacaaggtgcttgtttacggagatgagaaccaaaagaaggggaacaggattccttacactttcttctctgaagaagataaggagtgggagtctttcgagtcttacgtgaggtccaactccttcttctctaagaagaagaggggataccttcttaagaaggcttatcttcctagggagtctaaccttattaaggagaggcaccttaacgataccaggtacgcttcatcttacctcaagaacttcatcgagaagaaccttaagttcaaggaggctgtgggaattactaggaagaagtacgttcagactgtgaacggagtgattactgctcatcttagaaagagatggggacttgagaaggataggcaagagacttaccttcatcacgctatggatgctattattgtggcttgcactgatcaccatatggtgactaaggttaccgagtactaccaaattaaggaggggaacaagtccatcaagaagccttattttcctctaccttggatgggattcagggaggagattctttctcatcttgagtctcaacctatcgctagaaagatttccgaggagcttaagattggataccagtcccctgattacattcttgtgtctagaatgcctaagaggtctgttactggatctgctcatgatcagactgtgatgaagaagggggatattgataagaaggggaagaccatcattattaagagggtgcacctcaaggacatcaagttcgatgagaacggagatttcaagatggttggaaaggagcaggatctagctacttacgaggctattaagcagaggtatcttgagtataggaaggagtctaagaaggctttcgagactcctctttacaagccttctaagaagggaaaggggaacctcatcaagaagattaaggttgaggttcagactaagtctttcgtgagggagattaatggaggagttgctcagaatggagatcttgtgagggttgatcttttcgagaaggacaacaggtactacatggtgcctatctacgttgttgatactgttaggtctgagctacctaacaaggctgttacttcttctaagggatacgagcagtggctctctattgataactctttcaccttcaagttctctctctacccttacgatcttgttaggcttgttaagggagatgaggataggttcctctacttctccaccctcgatattaactctgataggctcaacttcaaggatgtgaacaagccttctaagcaagctgagtacaggtactctcttaagaccattgagaaccttgagaagtacgagattggagttcttggagatctaaggcttgttaggcaggagaccaggaagattttcaag

SEQ ID NO: 174 - DNA, 3213 bp, Artificial Sequence
  source: /note="Description of Artificial Sequence: Synthetic polynucleotide"
  source: /note="APG07513.1 Corn optimized"
atgcgcgagctagattacaggatcggcctggatatcggcactaactcaatcggctggggcgtgatcgagctgagctggaataaagatcgcgagcagtatgaaaagaccaggatcgtggacaagggcgtgaggatgttcgataaggccgagatcccaaagacaggcgcctctctggccgaaccaaggaggatcgccaggtcttctaggaggagattaaacaggaagtctcagcgcaagaaggatataaggaacctgctggtccagcatgaaatcatcagccagaaggagctgacaagcctgtacccgctgagcaagtcaagcatggacatctgggatataaggctggatggcctggataggctgctggataggttcgagtgggccaggctgctgatacatctggcccagaggaggggcttcaaatcaaatcgcaagagcgaattaaaggacgtggagacaggcaaggtgctgtcaagcattcaggtgaatgaaaagaggctgagcctgtacaggacagtgggcgagatgtggatgaaaaacgccgactgctcaaaatacggcaagcgccgcaacagcccaaacgagtacgtgttctctgtgtctagggccgatctggagaaggagatcgtgacactgttcgaggcccagaggaagttccactcttcttacgcctctgtggacctgcagaagacatacatccagatctgggcccaccagctgccattcgcctctggcaatgccatcgtgaataaagtgggctactgctctctattaaagggcaaggagaagagggtgccaaaggccacctatacattccagtacttcaataccctggaccaaatcaacaggacccgcctgggcccaaacttccagccattcacaaaggagcagcgcgatataatcctggataaaatgttccagcgcaccgactactataaaaagaagaccatcccggaggtgacatactacgatataaggaagtggctggccctggatgaaaccatccagttcaagggcctaacctacgacccgaacgaggagctgaagaagatcgagatgaaaccgttcataaacctgaagccgttctacgaaatcaagaaggtggtaaccaactacgccaagaaaaccaacgaggtgttcagcgccctggactacgacaccgtggcctacgccctgaccgtgtataaaaccgacaaggatataaggagctacctgaagcgcagcaataatctgagcaagcgctgctacgacgaccaattaatcgaggagctgctgaccctgagctatactaagttcggccacctgagcttcaaggcaatcaaccacgtgctgccaataatgcaggagggccgcacctaccaggaggcaatacaccagctgggctacgacacaaccaacctgaagaaggagaaccgaagcatgttcctgccaataatcccggacgagataaccaacccgatcgtgaagcgcgccctgacccaggcccgcaaggtggtgaacgcaataatccgccgctacggctcaccgaacagcgtgcacattgagctggcccgcgaattaagcaagagccacgacgagcgcaagaagatcatgaccgcccacgatgaaaactacaagaaaaataagggcgccgtgagcatcctgatcgacaacggcatcctgaacccgaccggctacgacatcgtgcgctacaagctgtggaaggagcagggcgagaggtgcgcctactctctgaagaagatcccagccaacaccttcttcaacgagctgaagaaggagaggtctggcccaccagtgctggaggtggatcacatcctgccatactcacagagcttcatcgatagctaccacaacaaggtgctggtgtacggcgatgagaaccagaagaagggcaatcgcatcccatacacattcttcagcgaggaggataaggagtgggagagcttcgagagctacgtgaggagcaacagcttcttcagcaagaagaagaggggctacctgctgaagaaggcctacctgccaagggagtctaacctgatcaaggagaggcacctgaacgatacaaggtacgccagcagctacctaaagaacttcatcgagaagaacctgaagttcaaggaggccgtgggcatcacccgcaagaagtacgtccagacagtgaacggcgtgatcacagcccacctgaggaagaggtggggcctggagaaggataggcaggagacatacctgcatcacgccatggatgccatcatcgtggcttgcacagatcaccacatggtgacaaaggtgacagagtactaccagatcaaggagggcaacaagagcatcaagaagccatacttcccactaccatggatgggcttcagggaggagatcctgtctcacctggagtctcagccaatcgccaggaagatctctgaggagctgaagatcggctaccagtctccagattacatcctggtgtctaggatgccaaagaggtctgtgacaggctctgcccacgatcagacagtgatgaagaagggcgatatcgacaagaagggcaagaccatcatcatcaagagggtgcacctgaaggacatcaagttcgacgagaacggcgacttcaagatggtgggcaaggagcaggatctagccacatacgaggccatcaagcagcgctacctggagtacaggaaggagtctaagaaggccttcgagacaccactgtacaagccatctaagaagggcaagggcaacctgatcaagaagatcaaggtggaggtccagaccaagagcttcgtgagggagatcaatggcggcgtggcccagaatggcgatctggtgagggtggatctgttcgagaaggataacaggtactacatggtgccaatctacgtggtggatacagtgaggagcgagctaccaaacaaggccgtgacatcttctaagggctacgagcagtggctgagcatcgacaacagcttcaccttcaagttcagcctgtacccatacgatctggtgaggctggtgaagggcgatgaggacaggttcctgtacttcagcacactggacatcaacagcgacaggctgaacttcaaggacgtgaacaagccatctaagcaggccgagtacaggtacagcctgaagaccatcgagaacctggagaagtacgagatcggcgtgctgggcgatctaaggctggtgaggcaggagacaaggaagatcttcaag

SEQ ID NO: 175 - DNA, 3216 bp, Artificial Sequence
  source: /note="Description of Artificial Sequence: Synthetic polynucleotide"
  source: /note="APG08290.1 Soy optimized"
atgtctgagctagattacaggatcggactcgatatcggaactaattcaattggatggggagtgattgagcttttctggaataaagatcgcgagcgctatgaaaaggttaggattgtggataagggagtgaggatgttcgataaggccgagattcctaataaaggagcttcacttgctgaaccaagaaggattgctagatctagcaggaggagattaaacaggaagtctcagaggaagaaggagattaggaaccttcttgttcagcacggaatgattactcaggaggagcttgatcttctctaccctctctccaagaaatcaatcgatatctgggatataaggcttgatggactcgataggctattaaaccatcttgagtgggctaggcttctaatacaccttgctcaaagaaggggcttcaaatcaaaccgcaagtccgaattaaaggatgctgagactggaaaggttctttcaagcatccaggtgaatgaaaagaggcttttcttgtataggactgtgggcgagatgtggataaaagatgccgagttctcaaaatatgataggaggaggaactctcctaacgagtacgtgttttctgtttctagggctgatcttgagaaggagattgtgactttgtttgaggctcaacgcaagttccaatcaagctacgcttctaagaaccttcaagagacctaccttcaaatttgggctcatcagcttccttttgcttccgggaacgctattctcaataaagtgggatactgctccttattaaagggaaaggagagaaggattcctaaggccacctatacattccagtacttctctgctcttgatcaagtgaatagaactaggcttggacctgatttccaacctttcactcaggagcagaaggaaataatcctcgataaaatgttccagcgcaccgactactataaaaagaagaccatccccgaggtgtcctactacgatataagaaagtggcttgagcttgatgaaaccattcagttcaagggattaaactacgaccccaacgaggagctgaagaaaatagagaagaagcccttcataaacctcaaggccttctacgaaatcaagaaggtggttgctaactacgctgaacgaaccaacgaagcattctctaccctcgattacgatgctattgcttacgctcttaccgtgtataaaaccgacaaggatataaggtcctacctcaagaaatcaaacaacctctccaagaggtgctacgacgatcaattaatcgaggagcttttcaccctctcctatactaagttcggacacctctctttcaaggcaatcaaccatgtgcttcctattatgcaagagggaagaacttaccaagaggctattcatcagcttggatacgataccaccaaccttaagaaggagaacaggtctatgttcctccctctcattcctgatgagattactaaccctattgtgaagagggctattactcaagctaggaaggtggtgaatgctattattaggaggtacggatcacctaactctgtgcatattgagcttgctagggagctttctaagtctcatgatgagaggaagaagattatgactgctcacgacgagaactacaagaagaacaagggggctatttccattctcattgagaacggaattcttaaccctaccggatacgatattgtgaggtacaagttgtggaaggagcaaggagagagatgcgcttactctcttaaggaaattcctcctgataccttcttcaacgagcttaagaaggagaggaacggatcacctattcttgaggtggatcacattcttccttactcccagtccttcattgattcttaccataacaaggtgcttgtgtattccgatgagaacaggaacaagggaaacaggattccttacacctacttccttgagactaataaggattgggaggcttttgagaggtatgtgaggtctaacaagctcttctctaagaagaagagggagtacctccttaagaagacttaccttcctagggagtctgagcttattaaggagaggcatctaaacgataccaggtacgcttctaccttcctcaagaacttcattgagcagaaccttcaattcaaggaggttgaggttaaccttaggaagaagagggttcagactgtgaacggagttattactgctcatcttagaaagagatggggacttgagaagaacaggcaagagacttaccttcatcacgctatggatgctattattgtggcttgcactgatcatcacatggtgactaggattaccgagtactaccagattaaggagtcaaacaagtctgtgaagaagccttattttcctatgccttgggagggattcagggatgagcttctttctcatcttgcttctcagcctatcgctaagaagatttctgaagagcttaaggctggataccagtcctctgattacattttcgtgtctagaatgcctaagaggtctgttactggagctgctcatgatcaaactattaggaggaagggaggaattgataagaaggggaagaccatcattattaagagggtgaggctaaaggacatcaagttcgatgagaacggggatttcaagatggttggaaaggagcaggatcttgctacttacgaggctattaagcagagatatcttgagcacaggaagaactctaagaaggctttcgagactcctctttacaagccttctaagaagggaaccggaaaccttatcaagagagttaagattgagggacagactaaggctttcgttagagaggttaatggaggagttgctcagaactctgatcttgtgagggttgatctattcgagaaggacgataagtactacatggtgcctatctacgttcctgatactgtttgttccgagcttcctaagaaggttgttaagtctggaaagggatacgagcaatggcttacccttgataactctttcaccttcaagtcttctctctacccttacgatcttgttaggcttgttaagggaaacgaggataggttcctttacttcgggaccctcgatattgattctgataggctcaacttcaaggatgtgaacaagccttcaaagcaaaacgagtacaggtactctctcaagaccattgagaaccttgagaagtacgaagtgggagttcttggagatcttaggcttgttaagcaagagaccaggaggattttcaatagg

SEQ ID NO: 176 - DNA, 3216 bp, Artificial Sequence
  source: /note="Description of Artificial Sequence: Synthetic polynucleotide"
  source: /note="APG08290.1 Corn optimized"
atgtcagagctggactacaggatcggcctggacataggcactaattcaatcggctggggcgtgatcgagctgttctggaataaagaccgcgagcgctatgaaaaggtgcgcatcgtggacaagggcgttaggatgttcgataaggccgagatcccgaataaaggcgcctcactagccgaaccaaggaggatcgccaggtcttctaggaggagattaaacaggaagtctcagaggaagaaggagatcaggaacctgctggtccagcacggcatgatcacacaggaggagctggatctgctgtacccactgagcaagaaaagcattgacatctgggacatcaggctagatggcctggacaggctgctgaatcacctggagtgggccaggctgctgatacatctggcccagaggaggggcttcaaatcaaatcgcaagtctgaattaaaggatgccgagacaggcaaggtgctgtcaagcatccaggtgaatgaaaagaggctgttcctctaccgcacagtgggcgagatgtggataaaagacgccgagttcagcaagtacgacaggaggaggaacagcccaaacgagtacgtgttctctgtgtcaagggccgatctggagaaggagatcgtgacactgtttgaggctcagcgcaagttccaatcaagctacgccagcaagaacctgcaagagacctacctgcagatctgggcccaccagctgccattcgctagcggcaatgccatcctgaataaagtgggctactgctctctattaaagggcaaggagaggaggattccaaaggccacctatacattccagtacttcagcgccctggaccaggtgaataggacaaggctgggcccagatttccagccattcacacaggagcagaaggaaataatcctggataaaatgttccagcgcaccgactactataaaaagaagaccatcccggaggtgtcatactacgatataaggaagtggctggagctggatgaaaccatccagttcaagggattaaactacgacccgaacgaggagctgaagaaaatagagaagaagccgttcataaacctgaaggccttctacgaaatcaagaaggtggtggccaactacgccgagcgaaccaacgaagcattcagcaccctggactacgacgccatcgcctacgccctgaccgtgtataaaaccgacaaggatataaggtcatacctgaagaaatcaaacaacctgagcaagcgctgctacgacgaccaattaatcgaggagctgttcaccctgagctatactaagttcggccacctgagcttcaaggcaatcaaccacgtgctgccaataatgcaggagggccgcacctaccaggaggcaatacaccagctgggctacgacaccaccaacctgaagaaggagaaccgcagcatgttcctgccgctaatcccggacgagatcaccaacccgatcgtgaagcgcgccatcacccaggctaggaaggtggtgaacgccatcatccgccgctacggcagcccgaacagcgtgcacatcgagctggcccgcgagctgagcaagagccacgacgagcgcaagaagatcatgacagcccacgacgagaactacaagaagaacaagggcgccatctcaatcctgatcgagaacggcatcctgaacccaaccggctatgacatcgtgcgctacaagctgtggaaggagcagggcgagaggtgcgcctactctctgaaggagatcccaccagatacattcttcaacgagctgaagaaggagaggaatggctctccaatcctggaggtggatcacatcctgccatacagccagtcattcatcgacagctaccacaacaaggtgctggtgtacagcgatgagaacaggaacaagggcaaccgcatcccgtacacatacttcctggagaccaacaaggattgggaggccttcgagaggtacgtgaggagcaacaagctgttcagcaagaagaagcgcgagtacctgctgaagaagacctacctgccaagggagtcagagctgatcaaggagaggcacctgaacgatacaaggtacgctagcaccttcctgaagaacttcatcgagcagaacctgcagttcaaggaggtggaggtgaacctgaggaagaagcgcgttcagacagtgaacggcgtgatcacagcccacctgaggaagaggtggggcctggagaagaataggcaggagacatacctacaccacgccatggatgccatcatcgtggcttgcacagatcaccacatggtgacaaggatcacagagtactaccagatcaaggagagcaacaagagcgtgaagaagccatacttcccaatgccatgggagggcttcagggatgagctgctgtctcacctggcctctcagccaatcgccaagaagatctcagaggagctgaaggccggctaccagtcttctgattacatcttcgtgtctaggatgccaaagaggtctgtgacaggcgccgcccacgatcagacaatcaggaggaagggcggcatcgataagaagggcaagacaatcatcatcaagagggtgaggctgaaggatatcaagttcgatgagaacggcgatttcaagatggtgggcaaggagcaggatctagccacatacgaggccatcaagcagcgctacctggagcacaggaagaactctaagaaggccttcgagacaccactgtacaagccatctaagaagggcaccggcaatctgatcaagagggtgaagatcgagggccagacaaaggccttcgtgagggaggtgaatggcggcgtggcccagaattctgatctggtgagggtggatctattcgagaaggacgataagtactacatggtgccaatctacgtgccagatacagtgtgctccgagctgccaaagaaggtggtgaagtctggcaagggctacgagcagtggctcacactggataacagcttcacattcaagagcagcctgtacccatacgatctggtgaggctggtgaagggcaatgaggacaggttcctgtacttcggcacactagacatcgatagcgacaggctgaacttcaaggacgtgaacaagccaagcaagcagaacgagtaccgctacagcctgaagaccatcgagaacctggagaagtacgaggtgggcgtgctgggcgatctgaggctggtgaagcaggagacaaggaggatcttcaatagg

SEQ ID NO: 177 - DNA, 4011 bp, Artificial Sequence
  source: /note="Description of Artificial Sequence: Synthetic polynucleotide"
  source: /note="APG05459.1 Soy optimized"
atgaagaaggactacgtgatcggactagatattggaactaactctgtgggatgggctgttatgactgaggattaccagctagttaagaagaagatgcccatctacgggaatacagagaagaagaagatcaagaagaacttctggggagtgagactatttgaagagggtcatactgctgaggataggagattaaagagaactgctaggagaaggatttctaggaggaggaacaggcttcgttaccttcaagcattctttgaagaggctatgaccgctctagatgaaaatttcttcgctaggcttcaggagtcttttcttgtgcctgaggataaaaagtggcacaggcatcctatttttgctaagttagaggatgaggtggcttaccatgaaacctaccctactatctaccaccttaggaagaagttggctgattcttcagagcaagccgacttgagattaatctaccttgctcttgcccacattgtaaaatataggggacacttccttatcgagggaaaactctccaccgaaaatatttcagtgaaggagcagtttcagcagttcatgatcatctataaccaaaccttcgtgaacggagaatcaaggcttgtgtctgctcctcttcctgagtccgtattaattgaggaggaacttactgagaaagcatccagaaccaagaagtctgagaaggttcttcaacagtttcctcaagagaaggctaacggacttttcggacagttcctcaaattaatggtggggaataaagccgacttcaagaaggtttttggacttgaggaggaggccaaaataacttacgcttctgagtcttatgaggaggatcttgagggaatactagctaaggtgggagatgaatacagcgatgttttccttgctgctaagaacgtttacgacgctgtggaattaagcaccatactagctgactccgataaaaagtctcacgccaaactctcttcaagcatgattgttaggttcactgagcatcaggaggatcttaagaagttcaagaggttcattagggagaactgccctgatgagtacgataaccttttcaagaacgagcaaaaggatgggtacgctggatacattgctcatgctggaaaggtgtcacaattaaagttctaccagtacgtgaagaaaataatccaggatatcgctggagccgagtacttccttgagaaaatagctcaggagaacttccttaggaagcagaggactttcgataacggagtgattcctcaccaaatacaccttgctgagctacaggcaataattcataggcaagctgcatactatcctttcctcaaggagaatcaagagaaaatagagcagctcgtgaccttcagaattccatactacgtgggacctctttctaagggagatgcttctacttttgcttggcttaagagacagtcagaggaaccaattaggccttggaatcttcaagagactgtggatcttgatcaatctgctactgctttcatagagaggatgaccaacttcgatacataccttccttctgagaaggtgctccctaagcattctctcctctatgaaaagttcatggtgttcaacgagctaaccaaaatatcctacaccgacgataggggaatcaaggctaatttctctggaaaggagaaggagaaaatattcgactacctcttcaagaccaggaggaaggtgaagaagaaggacataatacagttctaccgcaacgaatacaacaccgagattgtgaccttgtcaggacttgaggaggatcaattcaacgcttctttctctacctaccaggatctattaaagtgcggacttactagggctgagcttgatcatcctgataatgctgagaagctggaggacataatcaagatactaaccatcttcgaggataggcaaaggattaggacccagctttctactttcaagggacaattctctgctgaggttcttaagaagttggagaggaagcattatactggatggggaaggctctctaagaagctcattaacggaatctacgataaggagtcagggaagaccatcctagattacctcattaaggatgatggagtgtctaagcactacaacaggaacttcatgcagctcattaacgattcccagctctccttcaagaacgctattcaaaaggctcaatcttctgagcatgaagagactctttctgagactgttaacgaattagctgggtcccctgctattaagaagggaatctaccagtctctcaagattgtggatgagcttgtggctattatgggatatgctcctaagaggattgttgttgagatggctagggagaaccaaactacttctactggaaagaggaggtctattcagaggctaaagattgttgaaaaggctatggctgagattggatctaaccttcttaaggagcagcctactactaacgagcaacttagggataccaggctcttcctttactacatgcagaacggaaaggatatgtacactggagatgagctttctcttcataggctctcacactacgacatagatcacattatccctcagtccttcatgaaggatgattctctcgataaccttgtgcttgtgggatctactgagaataggggaaagtctgatgatgttccttctaaggaggtggttaaggatatgaaggcttactgggagaaactatacgctgctggacttatttctcaaaggaagttccagagacttactaagggagagcaaggaggacttactcttgaggataaggctcatttcattcaaaggcagcttgttgagaccaggcagattactaagaacgtggctggaattctagatcaaaggtacaacgctaactctaaggagaagaaggttcagatcattaccctcaaggcttctcttacctcccagttcaggtctattttcggactttacaaggttagggaggtgaacgattaccatcatggacaagatgcttaccttaactgcgtggttgctactactctacttaaggtttatcctaaccttgctcctgagttcgtttacggagagtatcctaagttccaggctttcaaggagaataaggctaccgctaagaccattatctacaccaaccttatgaggttctttactgaggatgagcctaggtttatgaaggatggagagattctctggtcaaactcctacctcaagaacatcaagaaggagcttaactaccaccagatgaacattgtgaagaaggtggaggttcaaaagggaggattctccaaggagtctattaagcctaagggaccttctaacaagctcattcctgtgaagaacggacttgatcctcaaaagtacggaggattcgattcacctgttgttgcttacactgttcttttcactcacgaaaaggggaagaagcctctcattaagcaggagattctcggaattaccattatggagaagactaggttcgagcagaaccctattctttttctagaggagaagggatttcttaggcctagggttcttatgaagctccctaagtacactctttatgagtttcctgagggaagaaggagacttcttgcttctgctaaggaggctcaaaagggaaaccaaatggttcttcctgagcaccttcttactcttctttaccatgctaagcaatgcctacttcctaaccaatctgagtctcttgcttacgtagaacaacatcaacctgagttccaagagattcttgagagggttgtggatttcgctgaggttcatacccttgctaagtctaaggttcagcagattgttaagttgttcgaggctaaccagactgctgatgttaaggagatcgctgcttcattcattcagcttatgcaattcaatgctatgggtgctccttctaccttcaagttcttccagaaggatatagagagggctaggtacacctccatcaaggagattttcgatgctaccattatctaccagtctactactggactttatgagactaggaggaaggtggttgat

SEQ ID NO: 178 - DNA, 4011 bp, Artificial Sequence
  source: /note="Description of Artificial Sequence: Synthetic polynucleotide"
  source: /note="APG05459.1 Corn optimized"
atgaaaaaggactacgtgatcggcctggacatcggcactaattcagtgggctgggccgtgatgacagaggactaccagctggtgaagaagaagatgcctatctacggcaacactgagaagaagaagatcaagaagaacttctggggcgtgcgcctattcgaggagggccacacagccgaggaccgcagattaaagaggacagccaggaggaggatctctaggaggaggaataggctgcgctacctgcaagcattcttcgaggaggccatgacagccctggatgaaaatttcttcgccaggctgcaggagtctttcctagtgccggaggataaaaagtggcacaggcaccctatcttcgccaagctggaggatgaggtggcctaccatgaaacatacccaacaatctaccacctgaggaagaagctggccgattcttctgagcaggccgacctgagattaatctacctggccctggcccacatcgtcaaatacaggggccacttcctgatcgagggcaaactgagcacagaaaatatcagcgtgaaggagcagttccagcagttcatgatcatctataaccaaaccttcgtgaacggcgaatcaaggctggtgagcgccccactgccggagagcgtattaatcgaggaggaactgaccgagaaagcatcccgaaccaagaagagcgagaaggtgctgcagcagttcccgcaagagaaggctaatggcctgttcggtcagttcctgaaactgatggtgggcaataaagccgacttcaagaaggtgttcggcctagaggaggaggccaaaataacctacgccagcgagagctacgaggaggacctggagggcatactagccaaggtgggcgatgaatacagcgatgtgttcctggccgccaagaatgtgtacgatgccgtggagctgtctacaatactagccgacagcgataaaaagagccacgccaagctctcttcaagcatgatcgtgaggttcacagagcatcaggaggacctgaagaagttcaagcgcttcatcagggagaactgcccggacgagtacgacaacctgttcaagaacgagcagaaggatggctacgccggatacatcgcccacgccggtaaggtgtcccaattaaagttctaccagtacgtgaagaaaataatccaggacatcgccggcgccgagtacttcctggagaaaatagcccaggagaacttcctgcgcaagcagaggacattcgacaacggcgtcatcccgcaccagatacatctggccgagctgcaggccatcatacataggcaggccgcatactacccattcctaaaggagaaccaagagaaaatagagcagctggtgaccttccgcatcccatactacgtgggcccactgtctaagggcgatgcctctacattcgcctggctgaagaggcagtctgaggaaccaatcaggccatggaatctgcaagagacagtggatctggatcagtctgccacagccttcatcgagaggatgaccaacttcgatacatacctaccaagcgagaaggtgctgccaaagcatagcctgctgtatgaaaagttcatggtgttcaacgagctaaccaagatcagctacaccgacgaccgcggaatcaaggccaacttcagcggcaaggagaaggagaaaatattcgactacctgttcaagacccgccgcaaggtgaagaagaaggacataatacagttctaccgcaacgaatacaacaccgagatcgtgaccctgagcggccttgaggaggaccagttcaacgccagcttctcaacctaccaggacctattaaagtgcggcctgacccgcgccgagctggaccacccggataacgccgagaagctggaggacataatcaagatactaaccatcttcgaggaccgccagcgcatccgcacccaattaagcaccttcaagggccagttcagcgccgaggtattaaagaagctggagcgcaagcattacacaggctggggcaggctgagcaagaagctaatcaacggcatctacgacaaggagagcggcaagaccatccttgactacctgatcaaggacgatggcgtgagcaagcactacaaccgcaacttcatgcagctgatcaacgacagccagctgagcttcaagaacgccatccagaaggcccagtcttctgagcacgaggagacactgtctgagacagtgaatgagctggccggctcaccagccatcaagaagggcatctaccagtctctgaagatcgtggatgagctggtggccatcatgggctacgccccaaagaggatcgtggtggagatggccagggagaatcagacaacatcaacaggcaagaggaggtctatccagaggctgaagatcgtggagaaggccatggccgagatcggctctaatctgctgaaggagcagccaacaacaaatgagcagctgagggatacaaggctgttcctgtactacatgcagaatggcaaggatatgtacacaggcgatgagctgtctctgcataggctgagccactacgacatcgatcacatcatcccgcagtcattcatgaaggacgactctctggataatctggtgctggtgggctctacagagaacaggggcaagagcgatgatgtgccatctaaggaggtggtgaaggatatgaaggcctactgggagaagctgtacgccgccggcctgatctctcagaggaagttccagaggctgacaaagggcgagcagggcggcctgacactggaggataaggcccacttcatccagaggcagctagtggagacaaggcagatcacaaagaatgtggccggcatcctggatcagaggtacaatgccaattctaaggagaagaaggttcagatcatcacactgaaggcctctctgacatctcagttcaggtctatcttcggcctgtacaaggtgcgcgaggtgaatgattaccaccacggccaggatgcctacctgaattgcgtggtggccacaacactactgaaggtgtacccaaatctggccccagagttcgtgtacggcgagtacccaaagttccaggccttcaaggagaataaggccacagccaagacaatcatctacacaaacctgatgaggttcttcacagaggacgagccaaggttcatgaaggatggcgagatcctgtggagcaacagctacctgaagaacatcaagaaggagctgaactaccaccagatgaacatcgtgaagaaggtggaggtccagaagggcggcttctcaaaggagagcatcaagccgaagggcccgagcaacaagctgatcccagtgaagaatggcctggacccacagaagtacggcggctttgattctccagtggtggcctacacagtgctgttcacacacgagaagggcaagaagccactgatcaagcaggagatcctgggcatcacaatcatggagaagacaaggttcgagcagaacccaatcctgttcctggaggagaagggcttcctgaggccaagggtgctgatgaagctaccaaagtacacactgtacgagttcccagagggcaggaggaggctgctggcctctgccaaggaggcccagaagggcaatcagatggtgctgcctgagcacctgctgacactgctgtaccacgccaagcagtgcctgctgccaaatcagtctgagtctctggcctacgtggagcagcaccagccagagttccaggagatcctggagagggtggtggatttcgccgaggtgcacacactggctaagtctaaggttcagcagatcgtgaagctgttcgaggccaatcagacagccgatgtgaaggagatcgccgcctcattcatccagctgatgcagttcaatgccatgggcgccccatctacattcaagttcttccagaaggatatcgagagggccaggtacacatctatcaaggagatcttcgatgccacaatcatctaccagtctacaacaggcctgtacgagacaaggaggaaggtggtggat

SEQ ID NO: 179 - DNA, 4308 bp, Artificial Sequence
  source: /note="Description of Artificial Sequence: Synthetic polynucleotide"
  source: /note="APG04583.1 Soy optimized"
atggccaaaaatattctaggactcgatctcggaaccaactctattggatgggctcttgttcagcaggactttgaaaataaggaggggaacatactaggaatggggtccagaataattcctatgtctcaggatatactaggagagttcgggaagggtaactctatttctcaaactgctgagagaactggatataggggagttagaaggttaagggagagacatcttcttagaagggagaggcttcatagggtgcttcatcttcttggattcctacctaagcattacgacgagaaaatagacttcactcagaggttcgggaagttcatcaatcaagctgaaccaaagttggctttcgattcagagttcctcttcaaggactccttccatgaaatgctagctgacttcaagcagaatcaacctgagttcctcaaggataaaaacggagaggattgccttgttccttacgactggactatatactacctaaggaagaaagcattgacccagaagatcgaaaaatatgagctggcctggctcatcctcaacttcaatcaaaagaggggatactatcaattaaggggagaggaggagaaggagaaccctaataaactcgtggggttccactctctcaaaatagtggatgttattcctgacgctgaaaccaataaaaagggagagacctggtactcacttcatcttgagaacggatgggtttataggaggtcctccaaaatatctctcgctgattggaaggacaaagtgagggatttcattgtgaccaccgatcttaatgatgatggatcagagaagctcgataaggatggaattgtgaagaggtcttttagggctccttctgctgatgactggaccctattaaagaagaagaccgagaaggatatcgacaactctaataaaaccgtggggacctacatctacgacaacctcctattaaaccccaagcagaaaatcaagggaaagatggttaggaccattgagaggaagttctacaagcaagagctggagcagatattaaagactcagaaggagttccattctgagcttcagtctgagaacttgcttcaagattgcgttagggagctgtacaggaataatgagcaacatcaacagatgcttgaggctaaggatttcgtgcacctcttcctcaacgatataattttctaccagaggcctcttaggtcccagaaatcaagcatttctaattgcacccttgagttccgcaagtccaagaatgaaaacggagaggaggtaatacacagattaaaggtgatcgccaaatcaaacccatactaccaggagttcaggcttcttcaatgggttcagaacctcgctatctatactaaggacgacgataagaacgtaaccaacgagttcctcaaatcaactcaggattgggaggatcttcttaggtggcttcactctaagaaggaaatcaagcaggatgctctaatcaagttcctcattgagaagaagggactcaaggggaaagcattgactattgaggtggcaaaatataggtggaactacgttcaggataaggattaccctggaaatgaaacccgctacctcattcaatcaaggcttgataaggttgagtacgctcctaaggatttcctcacctatgaaaatgaaatggccctctggcatatcatctactcaatcaacgacaagatcgagtatgaaaaggcattaaagtccttcgccaataaaaaggggctcgatgaggtgaccttcgtggaagcattcaagaagttccctcctttcaagtccgattacggatctttctctgagaaggcaatcaagaagctccttccattaatgaggttcggaactcaatggaactgggataacatcgaccaaaatagcaaggagaggattggaaaaatactaaccggggagtacgatgaaaatattaaagggagggttagggagaaggctaggcaccttaactctgagaccgattttcaagcattacctctttggcttgctcagtacgttgtttatggaaggcactctgaagctgatattgctggaaagtggaactctgtggatgatctcaagcagttccttgatgatttcaagcagcattccttgaggaaccctattgtggagcaggttattactgagactcttagggctgttaaggatatttggaacttctacggaaagggggctaaggatttcttctcagaaatacacattgagcttgggagggagatgaaaaataccgctgatgaaaggaagaggattaccaccatggtgaccgacaatgaaaataccaacctcagaatcaaagcattgcttgctgagatggctcttgatcagaacgttgataacgttaggccttactctcctatgcagcaggagattcttaagatctatgaggagggagttctaaacgctgaggagaacatcgatgatgatatcctcaagatttctaagactgctcagccttctgctaccgatcttaagaggtataagttgtggcttgagcaaaagtacaggtctccttacactggacagatgattcctcttaacaagttgttcacccctgagtacgagatcgagcacattattcctcagtctaggtacttcgacgattcaatgtccaacaaggttatttgcgaggctgctgtgaacaagttgaaggataaccagattggactcgtgttcattaagaaccatcatggagaggtggttgatttcggaatgggaaagcaggtgaagattcttgaggtttctgattacgaggatttcgtgaagcagaactataacaagaacaggggaaagaggaacaagctcctcttagaggatatccctgagaagatgattgagaggcagcttaacgataccaggtacatctctaagtacattacccaggtgctttccaacattgttagggatgataaggagggatctaaggatgatggagtgaactccaagaacattgttcctggaaacggaaagattaccaccaggcttaaacaggattggggacttaacgatgtgtggaacgatcttgttcttcctaggttcgagaggatgaacactcttaccaactctaacgatttcacctctaagaacactcacggaaagactattcctactgtgcctattgagctttcaaagggattctccaagaagaggattgatcacaggcatcatgctatggatgctcttgttattgcttgcgctactagggatcatgtgaaccttctcaacaacgagtcttctaagtctgataccaagaggtacgatcttaacaggaagttgaggaagtacgagaaggttgcttacaacgatcctaagactggagagagaattgagaaggaggtgcctaaggattttattaagccttgggagacctttactgaggatactaggacccttcttgagaacatcgtgatttctttcaagcagaacctcagggtgattaacaaggctaccaactactacgagaagattgagaacggaaagaaggtgaaggttgagcagaagggaattaattgggctgttaggaaggctctacataaggagactgtttctggacaggtgcaccttgataggattaaagtggctaagggaaagattcttaccgctactaggaagactcttgatgcttctttcaacgagaagaccattgagtctattaccgataccgggattcagaagattctcctcaactacctcaagtccaaggataacaatcctgaggttgctttctctcctgaaggaattgaggagcttaacaagaacatcaggctctataacgatggaaaggctcaccagcctattcttaaggttagggttttcgagcagggatctaagtttactcttggagagactggaaacaagactactaagtttgttgaggctgctaagggaaccaaccttttcttcggaatctacgaggataagtctggaaagaggtcttacgagaccatccctttgaacattgttattgagaggcaaaagcaaggactacaagctgttcctgagactaacgagaagggaaagcagcttcttttcaccctttctcctaacgatcttgtttatgttcctgaggagggagttttcgatgagaacaacatcaaggtggataggatctacaaggtggtgtctttctctacttaccaatgcttcttcgtgaggaacgatgtgtctacttctgtggttaacaaggttgagtactctgctctcaacaagatggagaagtccatcgacaacatcatgattaaggagaactgcgtgaagttgaacgttgataggctcggaaagatttccaaggct

SEQ ID NO: 180 - DNA, 4308 bp, Artificial Sequence
  source: /note="Description of Artificial Sequence: Synthetic polynucleotide"
  source: /note="APG04583.1 Corn optimized"
atggccaagaacatactaggcctggacctcggaaccaattctatcggctgggccctggttcagcaggactttgagaacaaggagggcaacatactaggcatgggcagccgaataatccctatgtctcaggacatactgggcgagttcggtaagggcaacagcatctcacagacagccgagaggacaggctaccgcggcgtgaggaggctcagggagaggcacctgcttaggagggagaggctacacagggtgctgcatctgctgggcttcctgccaaagcattacgatgaaaagatagatttcacacagaggttcggcaagttcatcaatcaagccgaaccaaagctagccttcgattctgagttcctgttcaaggacagcttccatgaaatgctggccgacttcaagcagaatcaaccggagttcctgaaggataaaaacggcgaggactgcctagtgccgtacgactggaccatatactacctgcgcaagaaggccctcacccagaagatcgaaaaatacgagctggcctggctgatccttaacttcaaccaaaagcgcggatactaccagctacgcggcgaggaggagaaggagaacccgaataaactggtgggcttccacagcctgaaaatagtggacgtgatcccggacgccgagactaataaaaagggcgagacctggtactcacttcacctggagaacggctgggtgtaccgcaggagcagcaaaatatctctggccgactggaaggataaagtgagggacttcatcgtgaccacagacctgaacgacgatggctcagagaagctggacaaggatggcatcgtgaagaggtcattcagggccccatctgccgatgactggaccctattaaagaagaagaccgagaaggacatcgacaacagcaataaaaccgtgggcacctacatctacgacaacctgctattaaacccgaagcagaaaatcaagggcaagatggtgcgcaccatcgagcgcaagttctacaagcaggagctggagcagatactaaagacccagaaggagttccacagcgagctgcagagcgagaacctgctgcaggactgcgtgcgcgagctgtaccgcaataatgagcagcaccagcagatgctggaggccaaggacttcgtgcacctgttcctgaacgatataatcttctaccagaggccgctcaggagccagaagtcaagcatcagcaattgcaccctggagttccgcaagagcaagaatgaaaacggcgaggaggtgatacatcgattaaaggtgatcgccaagagcaacccatactaccaggagttccgcctgctgcagtgggtccagaacctggccatctatactaaggacgacgacaagaacgtaaccaacgagttcctgaaatcaacccaggactgggaggacctgctgcgctggctccacagcaagaaggaaatcaagcaggacgccctaatcaagttcctgatcgagaagaagggattaaagggcaaagcattgaccatcgaggtggcaaaatacaggtggaactacgtccaggacaaggactacccgggcaatgaaacccgctacctaatacagagccgcctggacaaggtggagtacgccccgaaggacttcctgacctacgagaatgaaatggccctgtggcatatcatctactcaatcaacgacaagatcgagtatgaaaaggcattaaagagcttcgccaataaaaagggcctggacgaggtgaccttcgtggaagcattcaagaagttcccgccgttcaagagcgactacggcagcttcagcgagaaggcaatcaagaagctgctgccattaatgcgcttcggcacccagtggaactgggacaacatcgaccaaaatagcaaggagcgcatcggcaaaatactaaccggcgagtacgacgagaacataaagggccgcgtgcgcgagaaggcccgccacctgaacagcgagaccgacttccaagcattgccgctgtggctggcccagtacgtggtctacggcaggcacagcgaggccgatatcgccggcaagtggaacagcgtggatgatctcaagcagttcctggacgatttcaagcagcacagcctgaggaatccaatcgtggagcaggtgatcacagagacactaagggccgtgaaggacatctggaatttctacggcaagggcgccaaggacttcttcagcgagatacatatcgagctgggccgcgagatgaaaaacaccgccgatgaaaggaagaggatcacaaccatggtgaccgacaatgaaaacaccaacctgcgaatcaaggccctgctggccgagatggccctggatcagaacgtggataacgtgaggccatactctccaatgcagcaggagatcctgaaaatatacgaggagggcgtattaaacgccgaggaaaatatcgacgacgacatcctgaaaataagcaagaccgcccaaccaagcgccaccgacctgaagcgatataagctgtggctggagcaaaaatacaggagcccgtacaccggccagatgatcccgctgaataaactgttcaccccggagtatgaaatcgagcatataatccctcagagccgctacttcgacgacagcatgagcaacaaggtgatctgcgaggccgccgtgaacaagctaaaggacaaccagatcggcctggtgttcatcaagaaccaccacggcgaggtggtggacttcggcatgggcaagcaggtgaagatcctggaggtgagcgactacgaggacttcgtgaagcagaactacaacaagaaccgcggcaagaggaacaagctgctgctggaggacatccctgagaagatgatcgagaggcagctgaacgacacccgctacatcagcaagtacatcacacaggtgctgagcaacatcgtgagggacgataaggagggctcaaaggatgatggcgtgaacagcaagaacatcgtgccaggcaacggcaagatcacaacaaggctgaagcaggattggggcctgaacgatgtgtggaatgatctggtgctgccaaggttcgagaggatgaacaccctgaccaacagcaacgacttcacctctaagaacacccacggcaagacaatcccaacagtgccgatcgagctgagcaagggcttcagcaagaagaggatcgatcacaggcaccacgccatggatgccctggtgatcgcctgcgccacaagggatcacgtgaatctactgaataacgagtctagcaagagcgatacaaagaggtacgatctgaacaggaagctgcgcaagtacgagaaggtggcctacaacgatccaaagacaggcgagaggatcgagaaggaggtgccgaaggatttcatcaagccatgggagacattcacagaggacacaaggaccctgctggagaacatcgtgatcagcttcaagcagaacctgcgcgtgatcaacaaggccaccaactactacgagaagatcgagaacggcaagaaggtgaaggtggagcagaagggcatcaattgggccgtgaggaaggccctacataaggagacagtgtctggccaggtgcacctggataggatcaaggtggccaagggcaagatcctgacagccacaaggaagacactggatgcctctttcaacgagaagacaatcgagagcatcacagacaccggcatccagaagatcctgctgaactacctgaagagcaaggacaacaacccagaggtggccttctctccagagggcatcgaggagctgaacaagaacatcaggctgtacaatgatggcaaggcccaccagccaatcctgaaggtgcgcgtgttcgagcagggctcaaagttcacactgggcgagacaggcaataagacaacaaagttcgtggaggccgccaagggcacaaatctgttcttcggcatctacgaggataagtctggcaagaggtcttacgagacaatcccgctgaatatcgtgatcgagaggcagaagcagggactgcaggccgtgccagagacaaatgagaagggcaagcagctgctgttcacactgtctccaaatgatctggtgtacgtgccagaggagggcgtgttcgatgagaacaatatcaaggtggacaggatctacaaggtggtgagcttctcaacctaccagtgcttcttcgtgaggaacgacgtgagcacaagcgtggtgaacaaggtggagtacagcgccctgaacaagatggagaagagcatcgacaacatcatgatcaaggagaactgcgtgaagctgaacgtggaccgcctgggcaagatctctaaggcc

SEQ ID NO: 181 - DNA, 4368 bp, Artificial Sequence
  source: /note="Description of Artificial Sequence: Synthetic polynucleotide"
  source: /note="APG01688.1 Soy optimized"
atgatgatcaagaacatactaggactcgatctcggaaccaactctatcggatgggctctaatcaagcaggatttcgagaacaagcatggagaaatactagggatgggctccagaataattcctatgtcccaggatatactaggagatttcggaaagggtaactctatttctcagaccgctgatagaaccaagtataggtctgttagaaggcttagggagagatttcttcttaggagagagaggcttcatagggtgctccacctattaaacttccttcctcaacactacgcttctcagatcgatttcgagaagaagttcggaaagtttaagtctgagaccgaaccaaagttagcttgggaaaattggggaggaaagttctctttcctcttccaaaatagcttcaatgaaatgctggaggatttcaaggctgctggacaggggctcaaaataccttacgactggaccatatactatctcaggaagaaagcattgtcccagaaaatagagaaggaggagctagcttggatactcctcaacttcaatcaaaagaggggatactatcaattaagaggtgaggaggaggaggagaaccctaataaactcgtggagttctactccctcaaaatagtggatgttgttgctgatgagcctcagaagggaaagtccgatatctggtactcattaattcttgagaacggatgggtttatcgcagggcttccaaaatacctctcttcgactggaaggataaaaccagggatttcattgtgaccaccgatcttaacgatgataggtctgtgaagactgataaggagggaaatgaaaagaggtcttttagggctccttcagagaacgattggactcttgtgaagaagaagactgagcaggagattgatcagtctcataaaaccgtgggaacctacatctatgaaaccctcctattaaaccccaagcagaaaatcaagggaaagttggtgaggaccattgagaggaagttctacaaggacgagcttaagcagatactagagaagcaaaaggagttccaccaggaattaaagaacgacgacctatataacgactgcattagggagctgtacaggaataatgaggctcaccaattaaccctctccaagaaggatttcgtgcacctattaatggacgatctcattttctaccagaggcctcttaggtcccagaaatcaagcatttctaattgcaccctggagttcagaaaatacaaggatgaaaacgggattgagcacacccagtacctcaaggctatcccaaaatcaaacccatactaccaagagtttaggctttggcagtggatgtacaacttgaacatctacagaaaggatgatgaggctaacgtaaccaaggagttcctcaacaccaataaagacttcgagtctctcttcgagttcctcaataatcgcaaggagattgagcagaagcccctaatcaagttccttcttgagcagaaggacataaacaagaagctattaaacgccgaggctgagaaatacaggtggaactacgtggaggataaaaagtacccctgcaatgaaaccaagaccatgatttcctctaggcttgacaaggtggaaaatatctccgatgatttcctcaccagggacatcgagcagaaaatatggcatataatctactccgtgaacgacaagatcgagtatgaaaaggcattaaagtccttcgctaccaggaacgacctcgatgaaaatagcttcatcgaagcattcaagaagttctcccctttcaagtccgagtacggatctttctctgagaaggcaatcaagaagctccttccattaatgaggctcggaaaatactggtacgaggatgaaatcgtgaagcattccgacatctacttcaaaaatattgagaacctcctcggggatttctccaaccgcgacaagaaaatatctgaggaagacaaggagaagtggaacaagtcaatcaaccttaagctccaggaggaattaaaggatttccagaccgctgagattgatttgttccagggacttaggcttcacattgctcagtaccttgtttatggaaggcactccgaagcatctatgattggaaagtggaattctgctgaggatcttgaggagttccttaaggatttcaagcagcattcccttaggaaccctattgtggagcaggttattactgagactcttagggtggttaaggatatttggctaaagtacggaaacggggctaaggatttcttcaacgagattcatattgagcttggaagggaaatgaagttgcctgctgatgataggaagaagctcaccaaccaaatttctgagaacgagaacaccaacttcaggattaaggctctccttgctgagatgatgaacgattcttctgttgagaacgttaggcctttctctcctatgcagcaggagattctaaagatctacgaggatgatgtgctcaagtccgatatcgagatcgaggatgatatcctcaagatttctaagactgctcaaccttctccttctgatcttaagaggtacaagttgtggcttgagcagaagtacaagtctccttacaccggacagattattcctcttaacaagttgttcacccctgagtacgagatcgagcacattattcctcagtcaaggtacttcgatgattccttctccaataaggtgatttgcgagtctgctgtgaacaagctcaaggataactacatcgggcttgagttcattaagcagttcggaggaactattattgagcttggattcgggaagtctattaaggtgttcgagactaaggagtacgaggatttcgtgaagaagcattacgctaacaaccagggaaagaggaacaagctccttatggaagatatccctgagaagatgattgagaggcagatgaacgataccaggtacatctcaaagtacatttctggggtgctttctaacattgttagggtggaagatggatctgatgagggagtgaactctaagaacattgttcctggaaacggaaagattaccacccaacttaagcaggattggggacttaacgatgtgtggaacgatctcattcttcctaggttcgagaggatgaatcagcttactaactctaaggttttcactgcttggaacgagaactaccagaagttccttcctactgtgcctattgagtactccaagggattctcaaagaagaggattgatcacaggcatcatgctcttgatgctcttgttattgcttgcgctactaaggatcacgtgaaccttcttaacaaccagtctgctaagtctgataccaagaggtacgatctcaagaagaagtccatgaagttcgagaaggtggtttacaacgatgctaagactggagaaaagattgagagggaggttcctaagcaatttcttaagccttgggagaacttcactcttgatgtgaagcacaaccttgagaccatcattgtgtcattcaagcagaacctcagggtgattaacaaggctaccaactactacgagaagtacgttgagaaggatggaactaagaataaggagagggttgagcaaactggaactaactgggctattaggaagcctatgcacaaggatactgtgtctggaaaagttgatcttccttgggttaaggtgcctaagggaaagattcttactgctaccaggaagtctctcgattcttctttcgatctcaagtccattggatctattaccgataccgggattcagaagatcctaaagaactacctcgctttcaaggatggaaatcctgagcttgctttctctcctgagggaattgatgacctcaacaagaacatcgagaagtataacgatggaaagcctcaccagcctattaacaaggttagggttttcgagcttggatctaagttccaagttggacagtctggaaacaagaaggataagtatgttgaggctgctaagggaaccaaccttttcttcgctgtttatgaggatgagaagggaaagaggaactacgagactattcctctaaacgaggttattgagaggcaaaagcagggactttctgtggttgatcttaaggggaccaacgatttctatctttgccctaacgatttcgtgtacattccttctggagatgagctggagaacatcaacaacgtggacttcaaggatatcaagaaggagattaacgagaggatctacaaggtggtgtctttcactggaaacaggctttcttgcattccttacatggtggctaccactattgtgaacaagttggagttcacccagctaaacaagattgagttcaccaaggagaaggagatctgcattaagttgaacgtggataggctcggaaacatttctaaggct

SEQ ID NO: 182 - DNA, 4368 bp, Artificial Sequence
  source: /note="Description of Artificial Sequence: Synthetic polynucleotide"
  source: /note="APG01688.1 Corn optimized"
atgatgatcaagaacatcctaggcctggacctcggaaccaattctatcggctgggccctgatcaagcaggacttcgagaacaagcatggcgagatactaggcatgggcagccgaataatcccgatgagccaggacatactaggcgatttcggcaagggcaatagcatctctcagaccgccgacagaaccaagtacaggtctgttaggaggctgagggagaggttccttcttaggagggagaggctgcatagggtgctccacctattaaacttcctgccacagcactacgccagccagatcgacttcgagaagaagttcggcaagttcaagagcgagacagaaccaaagctggcttgggaaaactggggcggcaagttcagcttcctgttccaaaatagcttcaatgaaatgctggaggacttcaaggccgccggccagggattaaagatcccctacgactggaccatatactacctgcgcaagaaagcattgagccagaaaatagagaaggaggagctggcctggatactgctgaacttcaaccaaaagcgcggatactaccagctgcgcggtgaggaggaggaggagaacccgaataaactggtggagttctactcactgaaaatagtggacgtggtggccgacgagccgcagaagggcaagagcgacatctggtacagcctgatactagagaacggctgggtgtaccgccgcgctagcaaaataccgctgttcgactggaaggataaaacccgcgacttcatcgtgaccaccgacctgaacgacgacaggagcgtgaagacagataaggagggcaatgaaaagaggagcttcagggccccaagcgagaacgattggaccctggtgaagaagaagacagagcaggagatcgatcagagccataaaaccgtgggcacatacatctatgaaaccctgctattaaacccgaagcagaaaatcaagggcaagctggtgcgcaccatcgagcgcaagttctacaaggacgagctgaagcagatactagagaagcagaaggagttccaccaggaattaaagaacgacgacctatataacgactgcatccgcgagctgtaccgcaataatgaggcccaccaattaaccctgagcaagaaggacttcgtgcacctattaatggacgacctgatcttctaccagcgcccgctgcgcagccagaagtcaagcatcagcaattgcaccctggagttccgcaaatacaaggatgaaaacggcatcgagcacacccagtacctgaaggccatcccgaagagcaacccatactaccaggagttccgcctgtggcagtggatgtacaacctgaacatctaccgcaaggacgacgaggccaacgtaaccaaggagttcctgaatacaaataaagacttcgagagcctgttcgagttcctgaataatcgcaaggagatcgagcagaagccgctaatcaagttcctgctggagcagaaggacataaacaagaagctattaaacgccgaggccgagaaatacaggtggaactacgtggaggataaaaagtacccgtgcaacgaaaccaagaccatgatcagcagccgcctggacaaggtggaaaatatcagcgacgacttcctgacccgcgacatcgagcagaaaatatggcatataatctacagcgtgaacgacaagatcgagtatgaaaaggcattaaagagcttcgccacccgcaacgacctggatgaaaacagcttcatcgaagcattcaagaagttcagcccgttcaagagcgagtacggcagcttcagcgagaaggcaatcaagaagctgctgccattaatgcgcctgggaaaatactggtacgaggacgagatcgtgaagcatagcgacatctacttcaaaaatatcgagaacctgctgggcgacttcagcaaccgcgacaagaaaataagcgaggaggacaaggagaagtggaacaaaagcatcaacctgaagctgcaggaggaattaaaggacttccagaccgccgagatcgacctgttccagggcctgcgcctccacatcgcccagtacctggtgtacggccgccacagcgaggcaagcatgatcggcaagtggaacagcgccgaggacctggaggagttcctgaaggacttcaagcagcatagcctgcgcaacccgatcgtggagcaggtgatcaccgagaccctgcgcgtggtgaaggacatctggctaaaatacggcaacggcgccaaggacttcttcaatgaaattcacatcgagctgggccgcgagatgaaactgccggccgacgaccgcaagaagctgaccaaccaaatcagcgagaatgaaaacaccaacttccgaatcaaggccctgctggccgagatgatgaacgacagcagcgtggagaacgtgcgcccgttcagcccgatgcagcaggagatcctgaaaatatacgaggacgacgtgctgaagagcgacatcgagatcgaggacgacatcctgaagatcagcaagaccgcccagccgagcccgagcgacctgaagcgctacaagctgtggctggagcagaagtacaagagcccgtacaccggccagatcatcccgctaaacaagctgttcaccccggagtacgagatcgagcacatcatcccgcagagccgctacttcgacgacagcttcagcaacaaggtgatctgcgagagcgccgtgaacaagctgaaggataactacatcggcctggagttcatcaagcagttcggcggcaccatcatcgagctgggcttcggcaagagcatcaaggtgttcgagaccaaggagtacgaggacttcgtgaagaagcactacgccaacaaccagggcaagcgcaacaagctgctgatggaggacatcccggagaagatgatcgagcgccagatgaacgacacccgctacatcagcaagtacatcagcggcgtgctgagcaacatcgtgcgcgtggaggatggctcagatgagggcgtgaacagcaagaacattgtgccgggcaacggcaagatcacaacacagcttaagcaggactggggcctgaacgatgtgtggaacgatctgattctgccaaggttcgagaggatgaaccagctgaccaacagcaaggtgttcaccgcctggaacgagaactaccagaagttcctgccaaccgtgccaatcgagtacagcaagggcttcagcaagaagaggatcgatcacaggcatcatgctctggatgctctggtgatcgcctgcgctacaaaggatcacgtgaacctgctgaacaaccagagcgccaagagcgacacaaagaggtacgacctgaagaagaagagcatgaagttcgagaaggtggtgtacaacgacgccaagaccggcgagaagattgagagggaggtgccgaagcagttcctaaagccatgggagaacttcacactggacgtgaagcacaacctggagaccatcatcgtgagcttcaagcagaacctgagggtgatcaacaaggccaccaactactacgagaagtacgtggagaaggacggcaccaagaacaaggagagggtggagcagacaggcacaaattgggccatccgcaagccaatgcacaaggatacagtgtctggcaaggtggatctgccatgggttaaggtgccaaagggcaagatcctgacagccacaaggaagagcctggatagcagcttcgatctgaagagcatcggctctatcacagacaccggcatccagaagatcctgaagaactacctggccttcaaggatggcaatccagagctggctttctctccagagggcatcgacgacctgaacaagaacatcgagaagtacaacgacggcaagccacaccagccaatcaataaggtgcgcgtgttcgagctaggctctaagttccaggttggccagagcggcaacaagaaggataagtacgttgaggccgccaagggcacaaatctgttcttcgctgtgtacgaggatgagaagggcaagcgcaactacgagacaatcccactgaacgaggtgatcgaaaggcagaagcagggcctgtctgttgtggatctgaagggcaccaacgatttctacctgtgcccgaacgacttcgtgtacattccatctggcgacgagctggagaacatcaacaacgtggacttcaaggacatcaagaaggagatcaacgagcgcatctacaaggtggtgagcttcaccggcaacaggctgagctgcatcccatacatggtggccaccaccatcgtgaacaagctggagttcacccagctgaacaagatcgagttcaccaaggagaaggagatctgcatcaagctgaacgtggacaggctgggcaacatcagcaaggcc

SEQ ID NO: 183 - DNA, 3210 bp, Bacillus sp.
  source: /note="APG05083.1 Native Seq"
atgagagagttggattatcgcataggattagatattggaacgaattctattggctgggggatcattgaattatcttggaacaaagatagagaacaatatgagaaagcaagaattgtcgacaagggtgttcgtatgtttgataaggctgaaatacctaagactggtgcttctcttgctgaaccgaggcgtatagcacgctcatcacgtagaagattaaatcgcaaaagccagagaaaaaaagatatacgtaatttactcgttcaacatgaaattattagtcaaaaggaattggcttcgttatatcccctgacaaaaagttcaatggatatttgggatattcgcttggatggattagatcgcttgttagaccgttttgaatggactcgattattaattcatttagcgcaaagacgcggttttaaatcaaatcgaaagtctgaactgaaagatgtggagacaggaaaagtattatcaagtattcaagcaaatgaaaaacgattatcactgtaccgtacagtgggagagatgtggatgaagaatgaagattttagtaaatatgacaaaaggcgtaattcttctaatgagtatgtattttcggttagccgtgcagatttagaaaaagaaattgtgacactatttgaagcgcaaagaaaatttcagtcatcatatgcatcggctgatttacaaaaaacatacttacaaatttgggcacaccaacttccttttgcttctgggaatgcaattgtaaataaagtaggatattgttcattattaaaagggaaagaaaagagagttccgaaagcaacatatacttttcaatatttcagtacactagatcaaataaatcgaacacgattaggtcctaatttccaaccatttacgaaggaacagagagacgttattttagatgaaatgtttaatcgaacagattattataaaaaaaagacaatacccgaagtcacttactatgatattcggaaatggttagcattagatgaaacaattcaatttaaaggacttacctatgacccaaatgaagagctgaaaaaaatagaattgaaatcctttattaatttaaagccattctatgaaattaaaaaggtagttactaattacgccaaaaaaacaaatgaggcattctcaacattagactatgatacatttgcatatgctttaacagtttataaaacggacaaagatattagatcttatttaaagaaatctaataatttatcaaaatgttgctacgatgatcaattaatagaagagctattaactctctcctatacaaagtttggtcatttatcatttaaagcaattaatcatgtactgccaattatgcaagagggaaggacttatcaggaagcaatacaccaattaggatatgatgccactaatctaaaaaaagaaaacagaagtatgttcttgcccctttttcccgatgagataacaaatccaattgttaaaagagcactaactcaagcacgtaaagttgtaaatgctattattagaagatatggttcccccaattctgttcatattgaactagctcgtgagctttctaaaagtcatgatgagagaacgaaaataatgaaagctcatgatgaaaattataagaaaaataaaggagccatatcaattttgattgagaatggaattttaaatccgacaggatatgatattgtacgttataagttatggaaagagcaaggagaacgatgtgcttattcgctaaaacagattcctgctaatacgttttttaatgaaatgaaaaaagagcgaagtggctccccagttctagagatagatcacattttaccgtatagtcagagttttattgatagttatcataataaagtactagtttatggagatgagaatcaaaaaaagggaaatcgaattccatatacttattttttagaaggaaataaggactgggaaagctttgaaagctacgtacgattgaatagttttttttctaaaaagaagcgcggatatttattgaaaaaagcttacttgccaagagagagtaacatgattaaggagcgtcatttaaatgatactcgatatgctagtagctatttgaaaaacttcattgagaaaaatttgaaatttaaagaagttgaaggtagtacacgaaaaaaacatgtacagacggttaacggtataattacagcccatcttcgaaaaagatggggattagaaaaagataggcaggaaacatatttgcatcatgcaatggacgctattattgttgcttgtacagaccatcatatggtcactaaagtaacggagtactatcaaataaaagaaagtaataagtcaataaggaaaccatactttcctttgccatgggtgggctttagagaggaaattttatcacatttagcaaggcagccaattgctagaaaaattagtgaggaacttaaaattggatatcaatcatttgattatatacttgtatcgcgaatgccaaaaagatctgtcactggagcagctcatgaacagacaatcatgaaaaaaggtggtatcgacaaaaaaggaaaaactattatcataaagcgtgtgtacttaaaggatattaagtttgatgagaatggcgattttaaaatggttggaaaagaacaggatttagcaacttatgaagcgataaagcaaagatatatagagtatggaaaagaatcgaaaaaagcatttgaaacacctttatacaagcctagtaaaaaaggaaaaggaaacctcattaaaaagatcaaagtagaagtgcaaaccaaatcttttgttcgagaagttaatgggggcgtagctcaaaatggtgatttagtaagagtagatttgtttgaaaaggataatagatattatatgatacctatttatgtaatggatactgttcattccgaactaccaaataaagctgtaacaagcagtaaaggctatgagcaatggttaacaatagataacagctttacgttcaaattcagtttatatccttatgatttagtacgacttgtaaaaggtaatgaagatcgtttcctatattttagtacccttgatattaattcggatcgtcttaatttcaaagatgtaaacaagccatcaaagcaggctgaaaatcgttatagccttaaaacaattgagaatttagaaaaatatgaggttggtgttttaggtgatttaaggtttgtgagacaagaaatacgtaaaaatttt

SEQ ID NO: 184 - DNA, 3210 bp, Artificial Sequence
  source: /note="Description of Artificial Sequence: Synthetic polynucleotide"
  source: /note="APG05083.1 E. coli optimized"
atgcgcgagctagattatcgcatcggcctggatattggcactaactcaataggctggggcatcatcgaactgagctggaataaagaccgcgagcagtatgaaaaggcgcgcatcgtggataaaggcgtgcgcatgttcgacaaagcggaaattccgaaaaccggtgcaagtctggcggaaccaagacgtattgcacgtagtagtcgccgccgattaaaccgcaaaagtcagcgcaagaaggatataaggaacctgctggtccagcatgaaatcatcagccagaaggaactggcgagcctgtacccgctgaccaaatcaagtatggacatctgggatataaggctggacggcctggatcgtctgctggatcgctttgaatggacccgcctattaatccatctggcacagcgccgtggcttcaaatcaaaccgcaagagcgaattaaaggacgtggagaccggtaaagtgctgtcaagcattcaggcgaatgaaaagcgcctgagcctgtatcgtaccgtgggcgagatgtggatgaaaaacgaggacttctcaaaatacgataaaaggcgcaacagcagcaacgagtacgtgttcagcgtgagccgcgcggacctggagaaagaaatcgtgaccctgtttgaggcgcagcgcaaattccaatcaagctatgcgagcgcggatctgcagaaaacctacctgcagatttgggcacatcagctgccgtttgcaagcggtaacgcgatcgtgaataaagtgggctattgcagcctattaaaaggcaaagaaaaacgcgtgccgaaagcgacctatacattccagtacttcagcaccctggaccaaatcaaccgcacccgcctgggcccgaacttccagccgttcaccaaagaacagcgcgacgtgatcctggatgaaatgttcaaccgcaccgactactataaaaagaaaaccatcccggaggtgacatactacgatataaggaaatggctggcgctggatgaaaccatccagttcaaaggcttaacctacgatccgaacgaggaattaaagaagatcgaattaaaatcgttcattaatctgaaaccgttctatgaaattaaaaaggtggtaaccaactacgcgaagaaaaccaacgaagcattcagcaccctggactacgatacattcgcgtacgcgctgaccgtgtataaaaccgacaaggatataaggagctacctgaagaaatcaaacaacctgagcaaatgctgctacgacgaccaattaatcgaagaactgctgaccctgagctacaccaaattcggccacctgagcttcaaagcgatcaaccacgtgctgccgatcatgcaggaaggccgcacctaccaggaagcgatccaccagctgggctacgatgcgaccaacctgaaaaaggaaaaccgcagcatgttcctgccgctgttccctgatgaaatcaccaacccgatcgtgaaacgcgcgctgacccaggcgcgcaaggtggtgaacgcgatcatccgccgctacggctcaccgaacagcgtgcacatcgaactggcgcgcgaactgagcaaaagccacgatgaacgcaccaaaatcatgaaagcgcacgatgaaaactacaaaaagaacaaaggcgcgatcagcatcctgatcgaaaacggcatcctgaacccgaccggctacgatatcgtgcgctacaaactgtggaaagaacagggcgaacgctgcgcgtacagcctgaaacagatcccggcgaacaccttcttcaacgaaatgaaaaaggaacgctcaggcagcccggtgctggaaatcgatcacatcctgccgtacagccagagcttcatcgatagctaccacaacaaagtgctggtgtacggcgatgaaaaccagaaaaagggcaaccgcatcccgtacacctacttcctggaaggcaacaaagattgggagagcttcgaaagctacgtgcgcctgaacagcttcttcagcaaaaagaaacgcggctacctgctgaaaaaggcgtacctgccgcgcgaaagcaacatgatcaaagaacgccacttaaacgatacccgctacgcgagcagctacctgaaaaacttcatcgagaaaaacctgaaattcaaagaagtggaaggcagcacccgtaaaaagcatgtccagaccgtgaacggcatcatcaccgcgcatctgcgcaaacgctggggcctggaaaaagatcgccaggaaacctatctgcatcatgcgatggatgcgatcatcgtggcgtgcaccgatcatcatatggtgaccaaagtgaccgaatattatcagatcaaagaaagcaacaaatcaatccgcaaaccgtattttccgctgccgtgggtgggctttcgcgaagaaatcctgagccatctggcgcgtcagccgatcgcgcgtaaaatcagcgaagaactgaaaatcggctatcagagctttgattatatcctggtgagccgcatgccgaaacgcagcgtgaccggcgcggcgcatgaacagaccatcatgaaaaagggcggcatcgataaaaagggcaaaaccatcatcatcaaacgcgtgtatctgaaagatatcaaatttgatgaaaacggcgattttaaaatggtgggcaaggaacaggacttagcgacctacgaagcgatcaaacagcgctacatcgagtacggcaaagagagcaaaaaggcgtttgaaaccccgctgtacaaaccgagcaaaaagggcaagggcaacctgatcaaaaagatcaaagtggaagtccagaccaaatcgtttgtgcgcgaagtgaacggcggcgtggcgcagaacggcgatctggtgcgcgtggatctgtttgaaaaagataaccgctactatatgatcccgatctacgtgatggataccgtgcatagcgagctgccgaacaaagcggtgaccagcagcaaaggctatgaacagtggttaaccatcgataacagctttaccttcaaattcagcctgtatccgtacgacctggtgcgcctggtgaaaggcaacgaagatcgcttcctgtatttcagcaccctggacatcaacagcgatcgcctgaacttcaaggacgtgaacaaaccgagcaaacaggcggaaaaccgctatagcctgaagaccatcgagaacctggagaaatatgaagtgggcgtgctgggcgatctgcgctttgtgcgccaggaaattcgcaaaaacttc

SEQ ID NO: 185 - DNA, 3213 bp, Bacillus sp.
  source: /note="APG07433.1 Native Seq"
atgagggagttggactatcgcatagggttagatattgggacgaattctattggatggggtgttattgaattatcctggaacaaggacagagaacgatatgaaaaagtaaggattgtcgaccagggtgttcgtatgtttgatagggctgaaatgccaaaaacaggtgcttctcttgctgaaccgaggcgtatagcacgttcatcacgtagaaggttaaatcgtaaaagtcagaggaagaaaaatatacgtaatttacttgttcaacatggggtgattactcaagaagagctggattcgttatatcctctttcaaaaaaatcaatggatatttggggtattcgattggatggattagatcgtctgctaaatcattttgaatgggctcgattattaattcatttagctcaaagacgtggttttaaatcgaatcgtaagtctgaactgaaagatacggagacggggaaggtattatcgagtattcaattaaatgaaaaacgattatcactgtaccgtacagtgggagaaatgtggatgaaagatcctgattttagtaagtatgatagaaaacggaattctcctaatgagtatgtattttcggttagtcgtgcggaactagaaaaggaaatagttactttatttgcagcacaaagaaggtttcagtcaccatacgcatcgaaggatttacaagaaacatatttacaaatttggacacaccaacttccctttgcttctgggaatgcaattttaaataaagtgggatattgttcattattgaaagggaaagaaagaagaattccgaaagcaacatatacttttcagtattttagtgcactagatcaagtgaatcgaacacgattaggacctgattttcagccatttacgaaggaacaaagagaaattattttaaataacatgtttcaacgtacagattattataaaaaaaagactatacctgaagttacatactatgatatccggaaatggctagaactagatgaaactattcaatttaaaggacttaattatgatccaaacgaagaattgaaaaaaatagaaaagaaaccatttattaatttaaaggcattctatgaaattaataaggtagtcgcaaattattctgagagaacaaatgagacattttcaacgttagactatgatgggattggatatgctttaacagtttataaaacggacaaagatattaggtcttatttgaagagctctcataatttacctaaacgttgttacgatgatcaattaatagaggaactattaagtctttcttatacaaagtttggtcacttatcactgaaagcaatcaatcacgtactatcgattatgcaaaaaggcaatacttataaagaagcagtagaccagttagggtatgatacaagcggtttaaagaaagaaaaaagaagtaagttcttgcctcctatttcagatgagataacgaatccaattgttaaaagagcgttaacacaagcgcgtaaagttgtgaatgctataattagaagacatggttctccacattcagttcatattgaactggctcgtgaactttctaaaaatcatgacgagagaacaaaaatagtgtcagctcaagatgaaaattataagaagaataaaggggctatatcaattttaagtgagcatggaattttgaatccaacaggctatgatattgttcgttataagttatggaaagaacaaggagaacgatgtgcttattcgttaaaggagattcctgcggatacgttttttaatgaattaaaaaaagaacgaaatggtgctccaattctagaggtagatcacattttaccgtacagtcaaagttttattgatagttatcataataaagtattagtttacagtgatgaaaatcgaaaaaaggggaatcgaattccatatacctattttttagagacaaataaggattgggaagcttttgaaagatatgtaagatcaaataaatttttttctaaaaagaagcgtgagtatttattgaaaagagcatatttgccaagagaaagtgaactgataaaggagcgacatttaaatgatacgcgatatgctagtacctttttgaaaaacttcattgagcagaatttgcaatttaaagaagctgaagataatccgcgtaaaagacgtgtacaaacagttaacggtgtaattacagcacattttcgaaaaagatggggattagaaaaagatagacaagaaacatacttacatcatgcaatggacgctatcattgttgcttgtacagaccatcatatggttactagagtaacagagtattatcaaataaaagaaagtaataaatcagtaaagaaaccgtattttcctatgccatgggagggctttagagatgaactcttatcacatttagcgagtcagccaatagctaaaaaaattagtgaggagcttaaagctggatatcaatcattagattatatatttgtgtctcgaatgccaaaaagatctatcactggagcagcacataaacaaacgatcatgagaaaaggcggtattgataaaaaaggaaaaactattattatagagcgtttgcatttaaaggatattaagtttgatgagaatggtgattttaaaatggttggcaaagaacaagatatggcaacttacgaggcgataaagcaaagatatttggagcatggaaaaaactcgaaaaaagcatttgaaacacctctatacaaacctagtaaaaaaggaacaggaaatcttattaaaagagttaaagttgaaggacaagctaaatcttttgttcgagaagtaaatgggggcgtagcccaaaatggtgatttagtgagagttgatttatttgaaaaagatgataaatattacatggtgcctatttatgtaccagataccgtttgttcagaattacccaaaaaagttgtggcaagtagtaagggttatgagcaatggttaacactagataacagctttacgtttaaatttagtttatacccttatgatttagtacggcttgtaaaaggggacgaagatcgtttcttatactttggtactctcgatatcgattcagatcgtcttaattttaaagatgtaaataagccatcaaaaaagaatgaatatcgttatagccttaaaacaattgaggatttagaaaaatatgaggtgggtgttttaggagatttaaggttagtaagaaaagaaacacgtagaaattttcac

SEQ ID NO: 186 - DNA, 3213 bp, Artificial Sequence
  source: /note="Description of Artificial Sequence: Synthetic polynucleotide"
  source: /note="APG07433.1 E. coli optimized"
atgcgcgagctagattatcgcatcggcctggatattggcactaactcaataggctggggcgtgatcgaactgagctggaataaagaccgcgagcgctatgaaaaggtgcgcattgtggatcagggcgtcagaatgtttgatcgtgcggaaatgccgaaaaccggtgcatcactggcagaaccaagacgtatagcacgtagtagtcgccgccgattaaaccgtaaaagccagcgcaagaaaaatatccgcaacctgctggttcagcatggcgtcatcacccaggaagaactggatagcctgtacccgctgagcaagaaatcaatggacatctggggcattcgtctggatggtctggaccgcctattaaaccactttgaatgggcccgcctattaattcatctggcgcagcgccgcggcttcaaatcaaaccgcaagagcgaattaaaggacaccgagaccggtaaagtgctgtcatcgatccagctgaatgaaaaacgcctgagcctgtatcgcaccgtgggcgagatgtggatgaaagacccggacttctcaaaatacgaccgcaaacgcaacagcccgaacgaatacgtgtttagcgttagccgtgcggaactggagaaagaaatcgtgaccctgtttgcagctcagcgccgttttcagagcccgtatgcgagcaaagatctgcaagaaacctacctgcagatctggacccatcagctgccgtttgcaagcggtaacgcgatattaaacaaagtgggctattgcagcctattaaaaggcaaagaacgccgcatcccgaaagcgacctatacattccagtacttcagcgcgctggaccaggtgaaccgtacccgtctgggtccggattttcagccgttcaccaaagaacagcgcgagatcatattaaacaacatgttccagcgcaccgactactataaaaagaaaaccatcccggaggtgacatattacgatataaggaaatggctggaactggatgaaaccatccagttcaaaggcctgaactacgatccgaacgaggagctgaaaaaaatcgagaaaaaaccgttcattaatctgaaagcgttctatgaaatcaacaaagtggtggcgaactacagcgaacgcaccaatgaaaccttctcaaccctggattacgatggcatcggctacgcgctgaccgtgtataaaaccgacaaggatataaggagctacctgaaatcaagccacaacctgccgaaacgctgctacgacgaccaattaatcgaagaactgctgagcctgagctatactaagttcggccacctgtcattaaaagcgattaatcacgtgttaagcatcatgcagaaaggcaacacatataaagaagcggtggatcagctgggctacgataccagcggattaaaaaaagaaaaacgcagcaaattcctgccgccgatcagcgatgaaatcaccaacccgatcgtgaaacgcgcgctgacccaggcgcgcaaagtggtgaacgcgatcatccgccgccacggcagcccgcacagcgtgcacatcgaactggcgcgcgaactgagcaaaaaccacgatgaacgcaccaaaatcgtgagcgcgcaggatgaaaactacaaaaagaacaaaggcgcgatcagcatcctgtcagaacacggcatcctgaacccgaccggctacgatatcgtgcgctacaaactgtggaaagagcagggcgaacgctgcgcgtacagcctgaaagaaatcccggcggataccttcttcaacgagctgaaaaaagaacgcaacggcgccccgatcctggaagtggatcacatcctgccgtacagccagagcttcatcgatagctaccacaacaaagtgctggtgtacagcgatgaaaaccgcaaaaaaggcaaccgcatcccgtacacctacttcttagagaccaacaaagattgggaagcgttcgaacgctacgtgcgcagcaacaagttcttcagcaaaaagaagcgcgagtacctgctgaaacgcgcgtacctgccgcgcgaaagcgaactgatcaaagaacgccatctgaacgatacccgctacgcgagcaccttcctgaaaaacttcatcgaacagaacctgcagttcaaagaagcggaagataacccgcgcaaacgccgcgtccagaccgtgaacggcgtgatcaccgcgcattttcgcaaacgctggggcttagaaaaagatcgccaggaaacctatctgcatcatgcgatggatgcgatcatcgtggcgtgcaccgatcatcatatggtgacccgcgtgaccgaatattatcagatcaaagaaagcaacaaaagcgtgaaaaaaccgtattttccgatgccgtgggaaggctttcgcgatgaactgctgagccatctggcgagccagccgatcgcgaaaaaaatcagcgaagaactgaaagcgggctatcagagcctggattatatctttgtgagccgcatgccgaaacgctcaatcaccggcgcggcgcataaacagaccatcatgcgcaaaggcggcatcgataaaaaaggcaaaaccatcatcatcgaacgcctgcatctgaaagatatcaaatttgatgaaaacggcgattttaaaatggtgggcaaagaacaggacatggcgacctacgaagcgatcaaacagcgctatctggagcatggcaagaacagcaaaaaagcgtttgagaccccgctgtacaaaccgagcaaaaaaggcaccggcaacctgatcaaacgcgtgaaagtggaaggccaggcgaaatcatttgtgcgcgaagtgaacggcggcgtggcgcagaacggcgatctggtgcgcgtggatctgtttgaaaaagatgacaaatattatatggtgccgatctatgtgccggataccgtgtgtagcgaactgccgaaaaaagtggtggcgagcagcaaaggctatgaacagtggctgaccctggataacagctttaccttcaaattcagcctgtatccgtatgatctggtgcgcctggtgaaaggcgatgaagatcgctttctgtattttggcaccctggacatcgattcagatcgcctgaacttcaaggacgtgaacaaaccgagcaaaaagaacgaatatcgctatagcctgaaaaccattgaagatctggaaaaatatgaagtgggcgtgctgggcgatctgcgcctggtgcgcaaagagacccgccgcaactttcat

SEQ ID NO: 187 - DNA, 3213 bp, Bacillus sp.
  source: /note="APG07513.1 Native Seq"
atgagagagttggattatcgcataggattagatattggaacgaattctattggctggggtgttattgaattatcttggaacaaagatagagaacaatatgagaaaacgagaattgtcgacaagggtgttcgtatgtttgataaggctgaaatacctaagactggtgcttctcttgctgaaccgagacgtatagcgcgctcatcacgtagaaggttaaatcgtaaaagccagagaaaaaaagatatacgtaatttacttgttcaacatgaaattattagccaaaaggaattgacttcgttatatcccctgtcaaaaagttcaatggatatttgggatattcgcttagatggattagatcgcttgttagaccgttttgaatgggctcgattattaattcatttagcacaaagacgcggttttaaatcaaatcgaaagtctgaactgaaagatgtggagacaggaaaagtattatcaagtattcaagtaaatgaaaaacgattatctctgtaccgtacagtgggagagatgtggatgaagaatgcggattgtagtaaatatggcaaaaggcgtaattctcctaatgagtatgtattttcggttagccgtgcagatttagaaaaggaaattgtgactctatttgaggcgcaaagaaaattccattcatcatatgcatcggttgatttacaaaaaacatatatacaaatttgggcacaccaacttccttttgcttctgggaatgcaattgtaaataaagtaggatattgttcattattaaaaggtaaagaaaagagagttccaaaagcaacatatacttttcaatatttcaatacactagatcaaataaaccgaacacgattagggcccaatttccaaccatttacgaaggaacagagagacataattttagataaaatgtttcaacggacagattattataaaaaaaagacaatacccgaagttacttactatgatattcggaaatggttagcactagatgaaacaattcaatttaaaggacttacctatgacccaaacgaagagctgaaaaaaatagaaatgaaaccctttattaatttaaagccattctatgaaattaaaaaggtagttactaattacgcaaaaaaaacaaatgaggtattctcagcattagattatgatacagttgcatacgctttaacagtttataaaacggacaaagatattagatcttatttgaagagatctaataatttatcaaaacgttgctacgatgatcaattaatagaagagctattaactctctcctatacaaagtttggtcatttatcatttaaagcaattaatcatgtactgccaattatgcaagagggaaggacttatcaggaagcaatacaccaattagggtatgataccactaatcttaaaaaagaaaacagaagtatgttcttgcctattattccagatgagataacaaatccaattgttaaaagagcgttaactcaagcacgtaaagttgtaaatgctattattagaagatatggttctccaaattctgttcatattgaactagctcgtgagctttcgaaaagtcatgacgagagaaaaaaaataatgacagctcatgatgaaaattataagaaaaataaaggagctgtatcaattttgatcgataatggaattttaaatccgacaggatatgatattgtacgttataagttatggaaagagcaaggagaacgatgtgcttattcgttaaaaaagattcctgctaatacgttttttaatgaattgaaaaaagagcgaagtggccctccggttctagaggtagatcacattttaccgtatagtcagagttttattgatagttaccataataaagtattagtttatggggatgaaaatcaaaaaaagggaaatcgaattccatatacttttttttcagaagaagataaggagtgggaaagctttgaaagctacgtaagatcgaatagttttttttctaaaaagaagcgcggatatttattgaaaaaagcttacttgccaagagagagtaacttgattaaggagcgtcatttaaatgatacccgatatgctagtagctatttgaaaaacttcattgagaaaaatttaaaatttaaagaagctgtaggtattacacgaaaaaaatatgtacagacggttaacggtgtaattacagcccatctgcgaaaaaggtggggtttagaaaaagataggcaggaaacatatttgcatcatgcaatggacgctattattgttgcttgtacagatcatcatatggtcactaaagtaacggagtactatcaaataaaagaaggtaataagtcaataaagaaaccgtattttcctttgccatggatgggatttagagaggaaattttatcacatttagaaagtcagccaattgctagaaaaattagtgaggaacttaaaattggatatcaatcacctgattatatacttgtatcgcgaatgccaaaaagatctgtcactggatcagctcatgatcagacagtcatgaaaaaaggcgatatcgataaaaaaggaaagactattatcataaagcgtgtgcacttaaaggatattaagtttgatgagaatggcgattttaaaatggttggcaaagaacaagatttagcaacttacgaagcgataaagcaaagatatttagagtatagaaaagaatcgaaaaaagcatttgaaacacctttatacaagcctagtaaaaaaggaaaaggaaacctcattaaaaaaattaaagtagaagtgcaaaccaaatcttttgttcgagaaattaatgggggcgtagctcaaaatggtgatttagtaagagtagatttgtttgaaaaggataataggtattatatggtgcctatttacgtagtagatactgttcgttccgaactaccaaataaagctgtaacaagcagtaaaggctatgagcaatggttatcaatagataacagctttacgttcaaattcagtttatatccttatgatttagtacgacttgtaaaaggcgatgaagatcgttttctatactttagtactcttgatattaattcggaccgtcttaattttaaagatgtaaataagccatcaaagcaagctgaatatcgttatagtcttaaaacaattgagaatttagaaaaatatgagattggtgttttaggtgatttaaggttagtgagacaagaaacacgtaaaatttttaaa

SEQ ID NO: 188 - DNA, 3213 bp, Artificial Sequence
  source: /note="Description of Artificial Sequence: Synthetic polynucleotide"
  source: /note="APG07513.1 E. coli optimized"
atgcgcgagctagattatcgcatcggcctggatattggcactaactcaataggctggggcgtgatcgaactgagctggaataaagaccgcgagcagtatgaaaagacccgcatcgtggataaaggcgtgcgcatgttcgacaaagcggaaattccgaaaaccggtgcaagtctggcggaaccaagacgtattgcacgtagtagtcgccgccgattaaaccgcaaaagtcagcgcaagaaggatatcaggaacctgctggtccagcatgaaatcatcagccagaaggaattaaccagcctgtacccgctgagcaaatcaagtatggacatctgggatataaggctggacggcctggaccgcctgctggatcgttttgaatgggcccgcctattaatccatctggcacagcgccgtggcttcaaatcaaaccgcaagagcgaattaaaggacgtggagaccggtaaagtgctgtcaagcattcaggtgaatgaaaagcgcctgagcctgtatcgcaccgtgggcgagatgtggatgaaaaacgcggactgctcaaaatatggcaaacgccgcaacagcccgaacgaatacgtgtttagcgttagccgtgcggacctggaaaaagaaatcgtgaccctgtttgaggcgcagcgcaaattccatagcagctatgcgagcgtggatctgcagaaaacatacatccagatctgggcacatcagctgccgtttgcgagcggtaacgcgatcgtgaataaagtgggctattgcagcctattaaaaggcaaagaaaaacgcgtgccgaaagcgacctatacattccagtacttcaatacactggaccaaatcaaccgcacccgcctgggcccgaacttccagccgttcaccaaagaacagcgcgatataatcctggataaaatgttccagcgcaccgactactataaaaagaaaaccatcccggaggtgacatactacgatataaggaaatggctggcgctggatgaaaccatccagttcaagggcttaacctacgatccgaacgaggagctgaaaaagatcgagatgaaaccgttcattaatctgaaaccgttctatgaaattaaaaaggtggtaaccaactacgcgaagaaaaccaacgaagtgttcagcgcgctggattacgataccgtggcgtacgcgctgaccgtgtataaaaccgacaaggatataaggagctacctgaaacgcagcaataatctgagcaaacgctgctacgacgaccaattaatcgaagaactgctgaccctgagctatactaagttcggccacctgagcttcaaagcgattaatcacgtgctgccaataatgcaggaaggccgcacctaccaggaagcaatacaccagctgggctacgatacaaccaacctgaaaaaggaaaataggagcatgttcctgccaataatcccggatgaaatcaccaacccgatcgtgaaacgcgcgctgacccaggcgcgcaaagtggtgaacgcaataatccgccgctacggctcaccgaacagcgtgcacatcgaactggcgcgcgaactgagcaaaagccacgatgaacgcaaaaagatcatgaccgcgcacgatgaaaactacaaaaagaacaaaggcgcggtgagcatcctgatcgataacggcatcctgaacccgaccggctacgatatcgtgcgctacaaactgtggaaagaacagggcgaacgctgcgcgtacagcctgaaaaagatcccggcgaacaccttcttcaacgaactgaaaaaggaacgctcaggcccgccggtgctggaagtggatcacatcctgccgtacagccagagcttcatcgatagctaccacaacaaagtgctggtgtacggcgacgaaaaccagaaaaagggcaaccgcatcccgtacaccttcttcagcgaagaagacaaagaatgggagagcttcgaaagctacgtgcgcagcaacagcttcttcagcaaaaagaaacgcggctacctgctgaaaaaggcgtacctgccgcgcgaaagcaacttaatcaaagaacgccatctgaacgatacccgctacgcgagcagctacctgaaaaacttcattgagaaaaacctgaaattcaaggaagcggtgggcatcacccgcaagaagtacgtccagaccgtgaacggcgtgatcaccgcgcatctgcgcaaacgctggggcctggaaaaagatcgccaggaaacctatctgcatcatgcgatggatgcgatcatcgtggcgtgcaccgatcatcatatggtgaccaaagtgaccgaatattatcagatcaaagaaggcaacaaatcaatcaaaaagccgtattttccgctgccgtggatgggcttccgcgaagaaatccttagccatctggaaagccagccgatcgcgcgcaaaatcagcgaagaactgaaaatcggctatcagagcccggattatatcctggtgagccgcatgccgaaacgcagcgtgaccggcagcgcgcatgatcagaccgtgatgaaaaagggcgatatcgataaaaagggcaaaaccatcatcatcaaacgcgtgcatctgaaagacatcaaattcgacgaaaacggcgacttcaaaatggtgggcaaggaacaggacttagcgacctacgaagcgatcaaacagcgctacctggaataccgcaaagagagcaaaaaggcgtttgaaaccccgctgtacaaaccgagcaaaaagggcaagggcaacctgatcaaaaagatcaaagtggaagtccagaccaaatcgtttgtgcgcgagatcaacggcggcgtggcgcagaacggcgatctggtgcgcgtggatctgtttgaaaaagataaccgctattatatggtgccgatctacgtggtggataccgtgcgcagcgaactgccgaacaaagcggtgaccagcagcaaaggctatgaacagtggttaagcatcgataacagcttcaccttcaaattcagcctgtacccgtatgatctggtgcgcctggtgaaaggcgatgaagatcgcttcctgtattttagcaccctggacatcaacagcgatcgcctgaacttcaaagacgtgaacaaaccgagcaaacaggcggaatatcgctacagcctgaagaccatcgagaacctggagaaatacgaaattggcgtgctgggcgatctgcgcctggtgcgccaggaaacccgcaaaatcttcaaa

SEQ ID NO: 189 - DNA, 3216 bp, Bacillus sp.
  source: /note="APG08290.1 Native Seq"
atgagtgagttggattaccgcatagggttggatattggtacgaattccattggctggggtgttattgaattattttggaacaaggacagagaacgatatgaaaaagtaaggattgtcgacaagggcgttcgtatgtttgataaggctgaaatacctaataagggtgcttctcttgctgaaccgagacgtatagcgcgttcatcacgtagaaggttaaatcgcaaaagtcagaggaagaaagagatacgtaatttacttgttcaacacggaatgattacccaagaggaattggatttgttatatcctctttcaaaaaaatcaatagatatttgggatattcgtttggatggattagatcgtctgttgaatcatcttgaatgggctcgattattaattcatttagcacaaagacgtggttttaagtcgaatcgaaagtctgaattgaaagatgctgagacggggaaggtattatcgagtattcaagtaaatgaaaaacgactatttctgtaccgtacagtgggggaaatgtggataaaagatgctgagtttagtaagtatgatagaagacgtaattctcctaatgagtatgtattttcggttagtcgtgcggacttagaaaaggaaattgttactctatttgaagcacaaagaaagtttcagtcatcatacgcatcgaagaacttacaagaaacatatttacaaatttgggcacaccaacttccttttgcttctgggaatgcaattttaaacaaagtaggctattgttcattattgaaagggaaagaaaggagaattccgaaagcaacatatacttttcaatatttcagtgcactagatcaggtgaatcgaacacgattaggacctgattttcaaccatttacgcaggaacagaaagagattattttagataaaatgtttcaacgtacagattattataaaaaaaagactatacctgaagttagctactatgatatacggaaatggctagagttagatgaaactattcaatttaaaggacttaattatgatccaaacgaagaactgaaaaaaatagaaaaaaaaccatttattaatttaaaggcattctatgaaattaaaaaggtagttgcaaattatgctgagagaacaaatgaggcattttcaacgttagactatgatgcgattgcatatgctttaacagtttataaaacggacaaagatattagatcttatttgaagaaatctaataatttatcaaaacgttgctacgacgatcaattaatagaagagctatttactctctcctatacaaagtttggtcatttatcatttaaagcaattaatcatgtacttccaattatgcaagagggaaggacttatcaagaagcgatacaccaattaggatatgataccactaatcttaaaaaagaaaacagaagtatgttcttgcctcttattccagatgaaataacaaatccaattgttaaaagagcgataactcaagcacgtaaagttgtaaacgctattattagaagatatggttctccaaattctgttcatattgaactagctcgtgagctttctaaaagtcatgacgagagaaagaaaataatgacggctcatgatgaaaattataagaaaaataaaggagctatatccattttgatcgagaatggaattttaaatccgacaggatatgatattgtacgttataagttatggaaagagcaaggagaacgatgtgcttattcgttaaaggagattcctccggatacgttttttaatgaattaaaaaaagaacgaaatggttctccaattctagaggtagatcacattttaccgtatagccaaagttttattgatagttatcataataaagtattagtttacagtgatgaaaatcgaaacaagggaaatcgaattccatatacctattttttagagacaaataaggattgggaagcttttgaaaggtatgtaagatcaaataagcttttttctaaaaagaagcgtgagtatttattgaaaaaaacatatttgccaagagagagtgaactaataaaggagcgacatttaaatgatacgcgatatgctagtacctttttgaaaaacttcattgagcagaacttgcaatttaaagaagttgaagttaatctgcgtaaaaaacgtgtgcaaacagttaatggtgtaattacagcgcaccttcgaaaaagatggggattagaaaaaaatagacaggaaacatatctgcatcatgcaatggacgctatcattgttgcttgtacagaccatcatatggttactagaataacagagtattatcaaataaaagaaagtaataaatcagtaaagaaaccatattttccgatgccatgggagggttttagagatgaactcttatcacatttagcgagccagccaattgctaaaaaaattagtgaggagcttaaagctggatatcaatcatctgattatatatttgtgtctcgaatgccaaaaagatctgtcactggagcagctcatgatcaaacgattaggagaaaaggtggtattgataaaaaaggaaaaactattattataaagcgtgtgcgcttaaaggatattaagtttgatgagaatggcgattttaaaatggttggaaaagaacaagatttagcaacttatgaggcgataaagcaaagatatttggagcatagaaaaaactcgaaaaaagcatttgaaacacctctatacaagcctagtaaaaaagggacaggaaatctcatcaaaagagttaaaattgaaggacaaactaaagcttttgttcgagaagtaaatgggggagtagcccaaaatagtgatttagtaagagttgatttatttgaaaaagatgataaatattacatggtgcctatttatgtaccagataccgtttgttcagaattacccaaaaaagttgtgaaaagtggtaagggttatgagcaatggctaacactagataacagctttacgtttaaatctagtttatacccttatgatttagtacgtcttgtaaaaggtaatgaagatcgttttttatactttggtactctcgatatcgattctgaccgtcttaattttaaagatgtaaataagccatcaaaacagaatgaatatcgttatagtcttaaaacaattgagaatttagaaaaatatgaggttggtgttttaggtgatttaaggttagtgaaacaagaaacacgtagaatttttaataga

SEQ ID NO: 190 - DNA, 3216 bp, Artificial Sequence
  source: /note="Description of Artificial Sequence: Synthetic polynucleotide"
  source: /note="APG08290.1 E. coli optimized"
atgagcgagctagattatcgcatcggcctggatatcggcactaactcaataggctggggcgtgatcgaactgttctggaataaagaccgcgagcgctatgaaaaggtgcgcatcgtggacaaaggcgtcaggatgttcgacaaagcggagatcccgaataaaggtgcatcactggcggaaccaagacgtatagcacgtagtagtcgccgccgattaaaccgcaaaagtcagcgcaagaaagagatccgtaacctgctggttcagcatggcatgatcacccaggaagaactggatctgctgtacccgctgagcaagaaatcaatcgacatctgggatataaggctggacggcctggaccgcctattaaaccatctggaatgggcccgcctattaatccatctggcgcagcgtagaggcttcaaatcaaaccgcaagagcgaattaaaggacgcggagaccggtaaagtgctgtcaagcattcaggtgaatgaaaagcgcctgttcctgtatcgcaccgtgggcgagatgtggattaaagacgcggagttctcaaaatacgaccgccgtcgcaacagcccgaacgaatacgtgtttagcgttagccgtgcggacctggagaaagaaatcgtgaccctgtttgaagcgcagcgcaaattccaatcaagctacgcgagcaagaacctgcaagagacctacctgcagatttgggcacatcagctgccgtttgcaagcggcaacgcgatattaaacaaagtgggctattgcagcctattaaaaggcaaagaacgccgcatcccgaaagcgacctatacattccagtacttcagcgcgctggaccaggtgaaccgtacccgtctgggccctgattttcagccgtttacccaggaacagaaagaaataatcctggataaaatgttccagcgcaccgactactataaaaagaaaaccatcccggaagtgtcatattacgatataaggaaatggctggagctggatgagaccatccagttcaagggcctgaactacgatccgaacgaggagctgaaaaaaatcgagaaaaaaccgttcattaatctgaaagcgttctatgaaattaaaaaagtggtggcgaactacgcggaacgaaccaacgaagcattcagcaccctggattacgatgcgatcgcgtacgcgttaaccgtgtataaaaccgacaaggatataaggagctacctgaaaaaatcaaacaacctgagcaaacgctgctacgacgaccaattaatcgaagaactgttcaccctgagctatactaagttcggccacctgagcttcaaagcgattaatcacgtgctgccaataatgcaggaaggccgcacctaccaggaagcgatccaccagctgggctacgataccaccaacctgaaaaaagaaaaccgcagcatgttcctgccgctgatcccggatgaaatcaccaacccgatcgtgaaacgcgcgatcacccaggcgcgcaaagtggtgaacgcgatcatccgccgctacggctcaccgaacagcgtgcacatcgagctggcgcgcgagctgagcaaaagccacgacgagcgcaaaaaaatcatgaccgcgcacgacgagaactacaagaaaaacaaaggcgcgatcagcatcctgatcgagaacggcatcctgaacccgaccggctacgatatcgtgcgctacaaactgtggaaagaacagggtgaacgctgcgcgtacagcctgaaagaaatcccgccggataccttcttcaacgaactgaaaaaagaacgcaacggctcaccgatcctggaagtggatcacatcctgccgtacagccagagcttcatcgatagctaccacaacaaagtgctggtgtacagcgatgaaaaccgcaacaaaggcaaccgcatcccgtacacctacttcctggaaaccaacaaagattgggaagcgttcgaacgctacgtgcgcagcaacaaactgttcagcaaaaagaaacgcgaatacctgctgaaaaaaacctacctgccgcgcgaaagcgaactgatcaaagaacgccacttaaacgatacccgctacgcgagcaccttcctgaaaaacttcatcgaacagaacctgcagttcaaagaagtggaggtgaacctgcgtaaaaagcgcgtccagaccgtgaacggcgtgatcaccgcgcatctgcgcaaacgctggggcctggaaaaaaaccgccaggaaacctatctgcatcatgcgatggatgcgatcatcgtggcgtgcaccgatcatcatatggtgacccgcatcaccgaatattatcagatcaaagaaagcaacaaatcagtgaaaaaaccgtattttccgatgccgtgggaaggctttcgcgatgaactgctgagccatctggcgagccagccgatcgcgaaaaaaatcagcgaagaactgaaagcgggctatcagagcagcgattatatctttgtgagccgcatgccgaaacgcagcgtgaccggcgcggcgcatgatcagaccatccgccgcaaaggcggcatcgataaaaaaggcaaaaccatcatcatcaaacgcgtgcgcctgaaagatatcaaatttgatgaaaacggcgattttaaaatggtgggcaaagaacaggacttagcgacctacgaagcgatcaaacagcgctatctggagcatcgcaagaacagcaaaaaagcgtttgagaccccgctgtacaaaccgagcaaaaaaggcaccggcaacctgatcaaacgcgtgaaaatcgagggccagaccaaagcgtttgtgcgcgaagtgaacggcggcgtggcgcagaacagcgatctggtgcgcgtggatctgtttgaaaaagatgacaaatattatatggtgccgatctatgtgccggataccgtgtgtagcgaactgccgaaaaaagtggtgaaaagcggcaaaggctatgaacagtggttaaccctggataacagcttcaccttcaagagcagcctgtacccgtatgatctggtgcgcctggtgaaaggcaacgaagatcgctttctgtattttggcaccctggacatcgatagcgatcgcctgaacttcaaagacgtgaacaaaccgagcaagcagaacgaataccgctacagcctgaagaccatcgagaacctggagaaatatgaagtgggcgtgctgggcgatctgcgcctggtgaaacaggaaacccgccgcatttttaaccgc

SEQ ID NO: 191 - DNA, 4011 bp, Enterococcus sp.
  source: /note="APG05459.1 Native Seq"
atgaagaaagactacgttattggtctggatatagggactaattctgtcggctgggcagttatgacagaagactatcagttggtgaagaaaaaaatgcctatttatggaaacactgaaaaaaagaaaatcaagaaaaatttttggggtgtgcgtttatttgaagaagggcatacagccgaagatcgccgattaaaaagaacagcacgacgaagaattagtcgtcgacggaatcgtttacgctacttacaagctttttttgaagaagcgatgacagctttggatgaaaacttttttgctcgtttacaagagagttttttagtgcctgaagataagaagtggcacagacatccgatttttgctaagttggaagatgaagtagcttaccatgaaacgtatccgacaatctaccatttacgcaaaaaattagcagattcatctgagcaagcagatttacgactaatttatttggcgttggcacatattgtcaaatatcgtggacattttttaattgaaggaaaattaagtacagaaaatatttctgttaaagaacaatttcaacaatttatgatcatttataaccaaacctttgtgaatggagagagtcgcttagttagtgcgccattacctgaatctgtcttgattgaggaagagttgactgaaaaagcttctcgtactaaaaaatctgaaaaagtcttacaacaatttcctcaagaaaaagctaatggcttatttggtcagttcttaaagctaatggtagggaataaagctgactttaaaaaagtttttggtttggaagaagaagccaaaataacctacgctagtgaaagctatgaagaagatttagaaggcattttagcaaaggttggggatgaatatagtgacgtgtttttagctgctaaaaatgtgtacgatgcagttgaattatcaacgattttagcagattcggataaaaaaagtcacgcgaaattatcttctagcatgattgtccgttttacagaacatcaagaagatttaaaaaaattcaaacgatttattcgtgaaaattgtccagacgaatatgataatctctttaaaaatgaacagaaagacggctatgcaggctacattgcacacgcaggtaaggtttcacagcttaaattttaccagtatgttaagaaaatcattcaagatattgctggagcagaatattttttagaaaaaattgctcaagaaaactttttaagaaagcaacggacctttgataatggggtgattcctcatcaaattcatttggctgagttacaagcaatcattcatcgtcaagcggcctattatccatttttaaaagaaaatcaagaaaaaattgaacaactggttacatttcgaattccttattatgtcggaccattatcaaaaggagatgcaagtaccttcgcttggctaaaacgtcaaagtgaggaaccaattcgaccttggaaccttcaagaaaccgttgatttggaccaatcagcgacagcctttattgaacgaatgaccaattttgatacgtatttaccttctgaaaaagttttaccgaaacatagtttgttatatgaaaagtttatggtatttaatgaattgaccaagatttcttatacggatgatcgaggaatcaaagccaatttttcaggtaaagaaaaagaaaaaatctttgattatctgtttaagacgcgtcgaaaagttaagaaaaaggatatcattcaattctatcgaaacgaatataatacggagattgtcacgcttagtggacttgaagaagaccaatttaatgctagttttagcacgtatcaggatttactgaaatgtggtttaacaagagctgaattagaccaccctgataatgccgaaaaattggaagatatcataaaaattttaactatttttgaagatcggcaacgaattcggacgcaactttccacattcaaagggcagttctcagcagaagtactaaaaaaattagaacgcaagcactacactggctggggaagattgtcgaaaaaattaatcaatggtatctacgataaagaatcgggtaaaacaattttggactatttaattaaagatgatggggtctcaaaacactataatcgcaattttatgcaactgattaatgattcacaattatcttttaaaaatgctattcaaaaagcacagtccagtgaacatgaagaaacattaagtgaaactgtcaatgaattagctggtagtccagcaataaaaaaaggaatttatcaaagtttaaaaattgtcgatgaactagtcgcgattatgggttatgcgcccaagcggattgttgtcgaaatggcacgtgaaaatcaaacgactagcactggcaagagaagatccatccaacgcttgaaaatagttgaaaaagcaatggccgaaatcggcagcaatttattaaaagaacaaccaacgactaatgaacagttacgagatacccgtcttttcctttactatatgcaaaatggtaaagatatgtacacgggagatgaattatcgcttcatcgtttatctcactatgatattgatcatattatcccacaaagctttatgaaagacgattcattggataacctagttttagtgggctctactgaaaatcgagggaaatccgatgatgtacctagcaaggaagttgttaaggatatgaaagcttattgggagaaattatatgctgctggcttaattagtcaacggaaattccaacgtctgaccaagggggagcaaggtggcttgactctcgaagacaaagcgcattttatccaacgacaattagtagaaactcgtcaaattaccaaaaatgttgcagggatcttagatcaacgctacaatgctaattcaaaagagaaaaaagtccaaatcatcaccttgaaagctagtttaacgagccaatttcgttcgatttttggcttgtataaagttcgtgaagtgaatgattatcaccatggacaagatgcttatttaaactgtgtggtcgcaaccacgttattaaaagtttatcctaatttagcaccagaatttgtttacggagaatatcctaaattccaggcctttaaagaaaataaagccacggcgaagactataatttatacaaatttgatgcgctttttcacggaagatgaaccacggttcatgaaggatggcgaaattctttggagtaacagttatttaaaaaatatcaaaaaagaattaaattaccatcaaatgaatattgtcaaaaaagtagaagtgcaaaaaggcggtttttcaaaagagtcgattaaacccaaaggaccatcgaataaattgattcctgtcaaaaatggtttggatccccaaaaatatggcggttttgatagtcctgtagttgcttatacagtgttattcacgcatgaaaaaggtaaaaaacctcttattaaacaggagatactgggcattacgattatggaaaaaacaaggtttgaacaaaatcctattctttttttagaggagaaaggcttcctacggcctcgtgtattaatgaaattgcctaagtatacactgtatgaatttccagaggggcgcaggcgcttattagccagcgctaaagaagcgcaaaaagggaaccagatggttttacctgaacatttacttacgttactgtaccatgcgaaacaatgtttgttaccaaatcaatcagaaagtttggcttatgtagaacaacatcaaccagaatttcaagagattttagagagagtggttgactttgctgaagtgcatacattagccaagtcaaaagtccagcaaattgtgaaactttttgaagcaaatcaaacagcagatgtgaaagagattgcggcatcctttatccaacttatgcagtttaatgcgatgggcgcaccaagtacgtttaaatttttccaaaaagacattgagcgagcacgctacacgtcaatcaaagaaatttttgatgccactatcatttaccaatcgactacgggactgtatgaaacacgcagaaaggttgtcgac

SEQ ID NO: 192 - DNA, 4011 bp, Artificial Sequence
  source: /note="Description of Artificial Sequence: Synthetic polynucleotide"
  source: /note="APG05459.1 E. coli optimized"
atgaaaaaggactacgtgatcggcctagacatcggcactaacagcgttggttgggcggtgatgaccgaagattaccagctagtgaagaagaagatgcctatctacggtaatacagagaagaagaagattaaaaagaacttctggggcgtgaggctattcgaggagggtcacaccgcggaggaccgccgcctgaagcgcaccgctagacgccgtatttcacgtcgtcgtaaccgtctgcgttacctgcaagcattcttcgaagaagcaatgaccgcgctggatgaaaacttcttcgctaggctgcaggagtcatttctggtgccggaggataaaaagtggcaccgtcatccgatcttcgcgaaactagaagacgaggtggcgtaccatgaaacctacccgactatctaccacctgcgcaaaaagctggcggatagcagcgaacaagcagacctgcgattaatctatctggcgctggcgcacatcgtaaaatacagaggccacttcctcatcgagggcaaattatcgaccgaaaatattagcgtgaaggagcagttccagcagttcatgatcatctacaaccaaaccttcgtgaacggcgaatcaaggctggtgagcgcgccgctgccggagagcgtattaattgaggaggaattaaccgagaaagcgagccgcactaagaaaagcgagaaagtgcttcagcagttcccgcaagaaaaagcgaacggcctgttcggccagttcctgaaattaatggtgggcaataaagcggacttcaaaaaggtgttcggcctggaagaggaggcgaaaataacctacgcgagcgaaagctacgaggaagacctggagggcatactagcgaaagtgggcgacgaatacagtgacgtgttcctggcggctaaaaacgtgtacgacgcggtggaattaagcaccatactagcggacagcgataaaaagagtcacgcgaaattaagctcaagcatgatcgtgcgcttcaccgaacaccaggaagacctgaaaaagttcaaacgcttcatccgcgaaaactgcccggacgaatacgataacctgttcaaaaacgaacagaaagatggctacgcgggatacatcgcgcacgcgggcaaagtgtcacaattaaagttctaccagtacgtgaagaaaataatccaggatatcgcgggcgcggaatacttcctggagaaaatagcgcaggagaacttccttaggaaacagcgcaccttcgacaacggcgtgatcccgcaccaaatacacctggcggaactacaggcaataattcaccgccaggcggcatactacccgttcctgaaagagaaccaggagaaaatagaacagctggtgaccttccgcatcccatactacgtgggcccgcttagcaaaggcgatgcgagcaccttcgcgtggctgaaacgccagagcgaagaaccaatccgcccgtggaacttacaagaaaccgtggatctggatcagagcgcgaccgcgttcatcgaacgcatgaccaacttcgatacatacctgccgagcgaaaaagtgctgccgaagcatagcctgctgtatgaaaaattcatggtgttcaacgaactgaccaaaataagctacaccgatgatcgcggcattaaagcgaacttcagcggcaaagaaaaagagaaaatattcgattacctattcaaaacccgccgcaaagtgaaaaagaaagacataatacagttctaccgcaacgaatacaacaccgaaatcgtgaccctgagcggcctggaagaagatcagttcaacgcgagcttcagcacctaccaggacttattaaaatgcggcctgacccgcgcggagcttgaccacccggacaacgcggaaaaactggaagatatcattaaaatactgaccatcttcgaagatcgccagcgcatccgcacccagctgagcaccttcaagggccagttcagcgcggaagtgctgaaaaagctggaacgcaaacattacaccggctggggccgcctgagcaaaaagctgatcaacggcatctacgataaagaatcaggcaaaaccatcctggactacctgatcaaagatgacggcgtgagcaaacactacaaccgcaacttcatgcagctgatcaacgatagccagctgagcttcaagaacgcgatccagaaagcgcagagcagcgaacatgaagaaaccctgagcgaaaccgtgaacgaactggcgggcagcccggcgatcaaaaagggcatctatcagagcctgaaaatcgtggatgaattagtggcgatcatgggctatgcgccgaaacgcatcgtggtggaaatggcgcgcgaaaaccagaccaccagcaccggcaaacgccgcagcatccagcgcctgaaaatcgtggaaaaagcgatggcggaaatcggcagcaacctgctgaaagaacagccgaccaccaacgaacagctgcgcgatacccgcctgtttctgtattatatgcagaacggcaaagatatgtataccggcgatgaactgtcactgcatcgcctcagccattatgatatcgatcatatcatcccgcagagctttatgaaagatgatagcctggataacctggtgctggtgggcagcaccgaaaaccgcggcaaaagcgatgatgtgccgagcaaagaagtggtgaaagatatgaaagcgtattgggaaaaactgtatgcggcgggcctgatcagccagcgcaaatttcagcgcctgaccaaaggcgaacagggcggcctgaccttagaagataaagcgcattttatccagcgccagctggtggaaacccgccagatcaccaaaaacgtggcgggcatcctggatcagcgctataacgcgaacagcaaagaaaagaaagtccagatcatcaccctgaaagcgagcctgaccagccagtttcgcagcatctttggcctgtataaagtgcgcgaagtgaacgattatcatcatggccaggatgcgtatctgaactgcgtggtggcgaccaccttactgaaagtgtatccgaacctggcgccggaatttgtgtatggcgaatatccgaaatttcaggcgtttaaagaaaacaaagcgaccgcgaaaaccatcatctataccaacctgatgcgcttctttaccgaagatgaaccgcgctttatgaaagatggcgaaattctgtggagcaacagctatctgaaaaacatcaaaaaggaactgaactaccaccagatgaacatcgtgaaaaaggtggaggtccagaaaggcggcttctcaaaggaaagcatcaaaccgaaaggcccgagcaacaaactgatcccggtgaaaaacggcctggacccgcagaaatatggcggctttgatagcccggtggtggcgtataccgtgctgtttacccatgaaaaaggcaaaaagccgctgatcaaacaggaaattctgggcatcaccatcatggagaaaacccgctttgaacagaacccgatcctgttcctggaagaaaaaggctttctgcgcccgcgcgtgctgatgaaactgccgaaatataccctctatgaatttccggaaggccgccgccgcctgctggcgagcgcgaaagaagcgcagaaaggcaaccagatggtgttaccggaacatctgctgaccctgctgtatcatgcgaaacagtgcctgctgccgaaccagagcgaaagcctggcgtatgtggaacagcatcagccggaatttcaggaaattctggaacgcgtggtggattttgcggaagtgcataccctggcgaaaagcaaagttcagcagattgttaaactgtttgaagcgaaccagaccgcggatgtgaaagaaattgcggcgagctttattcagctgatgcagtttaacgcgatgggcgccccgagcaccttcaaattctttcagaaagatattgaacgcgcgcgctataccagcattaaagaaatttttgatgcgaccattatctatcagtcaaccaccggcctgtatgaaacccgccgcaaagtggtggat

SEQ ID NO: 193 - DNA, 4308 bp, Enterococcus sp.
  source: /note="APG04583.1 Native Seq"
atggctaaaaatatacttggattagatttgggaaccaatagtattggttgggcgttggtacagcaagactttgaaaacaaagaaggaaatattcttggaatgggaagtaggattattccgatgtcgcaagatattttaggagaattcggtaaggggaattctatttctcaaactgctgaacgtactggttatcgtggtgtccgtcggttaagagaacgacatttattacgtcgtgagcgtttgcaccgagttttgcatttgttgggtttcttgccaaaacattatgatgaaaaaatagattttacacaacgttttgggaaattcattaaccaagccgaacctaaattggcttttgatagtgaatttctttttaaagattctttccatgaaatgttagctgattttaaacaaaatcaaccagagtttttgaaagataaaaatggagaagattgtttagttccttatgattggacgatttattatttacgtaaaaaagcattaacgcaaaaaattgagaaatatgaattagcttggttgattcttaattttaatcaaaaacgtggttattatcaattaagaggtgaagaagagaaagaaaatccaaataaattggtgggatttcattctttgaaaatcgttgatgttattcccgatgctgaaacaaataaaaaaggagagacttggtattctttgcatttagaaaatggttgggtatatcgccgttcttctaaaatttcattagcggattggaaagataaagttcgagattttattgttacgactgatttaaacgatgatggttctgaaaaattggataaagatggaattgtgaaacgtagctttcgtgcaccaagtgcggatgattggactttgttgaaaaagaaaacagaaaaagatattgataactctaacaaaactgttggaacttatatttacgacaatcttttattgaacccaaaacaaaaaataaaaggaaaaatggttcgtaccatcgaacgtaagttttacaagcaagaattagaacaaattttaaaaactcaaaaagaatttcattcagaattacaaagtgaaaatttgctacaagattgtgttcgagaattgtatcgaaataatgaacaacatcaacaaatgttagaagctaaagattttgtgcatttgttcctaaatgatattattttctatcaacgtcctttgagaagtcaaaaatccagtatatcgaattgtactttggaatttagaaaatcgaaaaatgaaaatggtgaagaagttattcatcgtttaaaagtaattgcaaaatcgaatccatattatcaggaatttagattgttacaatgggtgcaaaatttagcaatttatacaaaagatgatgataaaaatgtaacaaacgaatttctaaagtctactcaagattgggaggatttattgagatggctacattctaaaaaagaaattaaacaggatgctttaattaagtttttgattgaaaagaaaggtttaaaaggcaaagctttaactattgaagtagcaaaatatcgttggaattatgttcaggacaaagattaccctggtaatgaaacccgatatttaattcaatctcgtttggataaagttgaatatgcacctaaggattttttaacttatgaaaatgaaatggctttgtggcacatcatttattcgataaacgataaaattgagtacgaaaaagccttaaaatcttttgccaacaaaaaaggtttggacgaagtaacttttgttgaagcgtttaagaaattcccgccttttaaaagtgattacggaagtttttctgaaaaagcaatcaagaaattattgcctttgatgcgttttggaactcaatggaattgggataatatcgatcaaaattctaaagaaagaattggaaaaatattgacaggcgaatatgatgaaaacatcaaaggtcgtgttcgcgaaaaagcaagacatctcaattctgaaaccgattttcaagctttacctttgtggttggcgcaatacgtagtttacggaagacattctgaagctgatattgcaggtaaatggaattcggtggatgatttaaagcaatttttagatgactttaaacaacattcgcttcgtaatcctattgtagagcaagtgattactgaaacgttgcgtgcggtaaaagatatttggaatttttatggaaaaggtgctaaagatttcttctctgaaattcatatcgagctggggcgtgaaatgaaaaatacggctgatgaacgcaagcgtattactacaatggttacggataacgaaaacaccaatttgcgtatcaaagctttgttggctgaaatggctttggatcaaaatgtagataatgttcgtccatattctccaatgcaacaagaaattttgaaaatctatgaagaaggtgttttgaatgctgaagaaaatatcgatgatgatattctgaaaattagtaaaacggctcaaccttctgctacagatttaaagcgttacaaattgtggttagaacaaaaatatcgttcgccttatacaggtcaaatgattcctttgaataagctgtttacacctgaatatgagattgaacacataattccgcaaagtcgctattttgatgatagtatgagcaataaagtgatttgcgaagcagcggtgaataaacttaaagacaatcaaattggtttggttttcattaagaatcatcacggagaagttgtggatttcggaatgggaaaacaagtgaagattttggaagtttccgattatgaggattttgtaaaacaaaattacaataaaaacagaggaaaacgtaataagttgttattggaagatattcctgagaaaatgattgaacgtcaactaaatgatacacgttacatcagcaaatatattacgcaagtgttatcgaatattgttcgtgatgataaagaaggtagtaaagatgatggtgtaaattctaaaaatattgttcctggaaacggaaaaattaccacaagacttaaacaagattggggattgaatgacgtttggaatgatttggttttacctcgttttgaacgaatgaatacattgactaattcaaatgattttacatcaaaaaatacacatggaaaaacaattccaacagttccaattgagttatccaaaggtttttctaaaaaacgtatcgatcatcgtcatcacgcaatggatgcgttggtaattgcctgtgcaacgagagatcacgtgaatttgttgaataacgaaagttcaaaatcggatacaaaacgttatgatttgaataggaaattaagaaaatacgagaaagtagcttacaatgatcccaaaacaggcgaacgaattgagaaagaagttccaaaagacttcattaaaccttgggagacctttaccgaagatacgcgaactttgttagaaaatattgtaattagtttcaagcaaaatctacgagttatcaataaagcaaccaattattatgaaaaaattgagaatgggaaaaaagtaaaagttgaacaaaagggaataaattgggctgtaagaaaagctttgcataaagaaaccgtttctggacaagtgcatttggatagaataaaagttgcaaaaggtaaaatattaacggctactcgtaaaactttggatgcctcttttaatgaaaaaacaattgagtcaattacggatacagggattcaaaagattttattgaattatttaaaatcaaaagataacaatccagaggttgcattttcaccagaaggaatagaagaattaaataaaaatattaggctatataatgatggaaaagcacatcaaccaattttgaaagttcgtgtttttgagcaaggaagcaaatttactttaggtgagacgggaaataaaaccactaagtttgtagaagcagcaaagggtactaatctatttttcggaatttatgaagacaaatcaggtaagagaagctacgaaaccattccattaaatattgtcatcgaaagacaaaaacaaggtctgcaagctgttcccgaaaccaatgagaaagggaaacaattgttgtttacgttatctccaaatgatttggtttacgttcctgaagaaggagtttttgatgagaataatatcaaggtagataggatttataaggtagtgagtttttctacctatcaatgtttttttgtaagaaatgatgtttctacttctgtagttaataaggttgaatattccgctttaaataaaatggaaaaatctattgacaacataatgataaaagaaaactgcgtcaaactgaatgtagaccgtttaggaaagatttcaaaagct

SEQ ID NO: 194 - DNA, 4308 bp, Artificial Sequence
  source: /note="Description of Artificial Sequence: Synthetic polynucleotide"
  source: /note="APG04583.1 E. coli optimized"
atggcgaagaacatactaggcctggatctcggaaccaacagcattggttgggcactggtccagcaggacttcgagaataaagagggcaacatactaggcatgggcagccgaataatccctatgagtcaggacatactaggcgagttcggcaagggcaacagcattagccagaccgcagaacgtactggttatcgtggtgtgcgccgtttacgtgaacgtcatctgttacgtcgtgaacgtctgcatcgtgttctgcatctgttaggcttcctgccgaagcattacgatgaaaagatcgacttcacccagcgcttcggcaagttcattaatcaagcggaaccaaagctggcgttcgacagcgagttcctgttcaaggacagcttccatgaaatgctagcggacttcaagcagaatcaaccggagttcctgaaggataaaaacggcgaggactgcctggtgccgtacgactggaccatatactacctgcgcaagaaagcactgacccagaagatcgaaaaatacgagctagcgtggctcatcctgaacttcaatcaaaagcgcggatactaccagcttaggggcgaggaggagaaagagaacccgaataaactggtgggcttccacagcctgaaaatagtggacgtgatcccggacgcggaaaccaataaaaagggcgagacctggtactcactgcatctggaaaacggctgggtgtaccgccgcagcagcaaaataagcctggcggactggaaagacaaagtgcgcgacttcatcgtgaccaccgacctgaacgatgacggcagcgaaaaactggacaaagacggcatcgtgaaacgcagctttcgtgcaccgagcgcagatgattggaccctattaaagaaaaagaccgaaaaagacatcgacaacagcaataaaaccgtgggcacctacatctacgacaacctgttattaaacccgaagcagaaaatcaaaggcaaaatggtgcgcaccatcgaacgcaaattctacaaacaggagctggagcagatcctgaaaacccagaaggaattccacagcgaactgcagagcgaaaacctgctgcaggattgcgtgcgcgaactgtaccgcaataatgaacagcaccagcagatgctggaagcgaaagatttcgtgcacctgttcctgaacgatataatcttctaccagcgcccgctgcgcagccagaaatcaagcatcagcaattgcaccctggaattccgcaaaagcaagaatgaaaacggcgaagaagtgatccaccgcctgaaagtgatcgcgaaaagcaacccatactaccaggaattccgcctgctgcagtgggtccagaacctggcgatctatactaaagacgacgacaagaacgtaaccaacgagttcctgaaatcaacccaggactgggaagatctgctgcgctggctgcatagcaagaaggagattaaacaggacgcgctgatcaagttcctgatcgagaaaaagggcctgaagggcaaagcattgaccatcgaggtggcaaaataccgctggaactacgtccaggacaaagattacccgggcaatgaaacccgctacctgatccaatcaaggctggacaaagtggaatacgcgccgaaagatttcctgacctacgagaatgaaatggcgctgtggcacatcatctacagcattaatgataaaatcgaatatgaaaaagcattaaaatcgttcgcgaataaaaagggcctggatgaagtgaccttcgtggaagcattcaaaaagttcccgccgttcaaaagcgattacggcagcttcagcgaaaaagcgattaaaaagctgctgccattaatgcgcttcggcacccagtggaactgggataacatcgatcaaaatagcaaagaacgcatcggcaaaatactaaccggcgaatacgatgaaaatattaaaggccgcgtgcgcgaaaaagcgcgccatctgaacagcgaaaccgatttccaagcattgccgctgtggctggcgcagtacgtggtgtacggccgccatagcgaagcggatatcgcgggcaaatggaacagcgtggatgatctgaaacagttcctggatgatttcaaacagcatagcctgcgcaacccgatcgtggaacaggtgatcaccgaaaccctgcgcgcggtgaaagatatctggaacttctatggcaaaggcgcgaaagatttcttcagcgaaatacacatcgaactgggccgcgaaatgaaaaataccgcggatgaaagaaaacgcatcaccaccatggtgaccgataatgaaaataccaacttacgcattaaagcattgctggcggaaatggcgctggatcagaacgtggataacgtgcgcccgtatagcccgatgcagcaggaaatcctgaaaatatatgaagaaggcgtattaaacgcggaagaaaatatcgacgatgatatcctgaaaataagcaaaaccgcgcaaccaagcgcgaccgatctgaaacgctataaactgtggctggaacagaaatatcgcagcccgtataccggccagatgatcccgctgaacaaactgtttaccccggaatatgaaatcgaacatatcatcccgcagagccgctattttgatgatagcatgagcaacaaagtgatctgcgaagcggcggtgaacaaactgaaagataaccagatcggcctggtgtttatcaaaaaccatcatggcgaagtggtggattttggcatgggcaaacaggtgaaaatcctggaagtgagcgattatgaagattttgtgaaacagaactataacaaaaaccgcggcaaacgcaacaaattactgctggaagatatcccggagaaaatgatcgaacgccagctgaacgatacccgctatatcagcaaatatatcacccaggtgctgagcaacatcgtgcgcgatgataaagaaggcagcaaagatgatggcgtgaacagcaaaaacatcgtgccgggcaacggcaaaatcaccacccgcctgaaacaggattggggcctgaacgatgtgtggaacgatctggtgctgccgcgctttgaacgcatgaacaccctgaccaacagcaacgattttaccagcaaaaacacccatggcaaaaccattccgaccgtgccgattgaactgagcaaaggctttagcaaaaagcgcattgatcatcgccatcatgcgatggatgcgctggtgattgcgtgcgcgacccgcgatcatgtgaacttactgaacaacgaaagcagcaaaagcgataccaaacgctatgatctgaaccgcaaactgcgcaaatatgaaaaagtggcgtataacgatccgaaaaccggcgaacgcattgaaaaagaagtgccgaaagattttattaaaccgtgggaaacctttaccgaagatacccgcaccctgctggaaaacattgtgattagctttaaacagaacctgcgcgtgattaacaaagcgaccaactattatgagaaaattgaaaacggcaaaaaggtgaaagtggaacagaaaggcattaactgggcggtgcgcaaagcgctgcataaagaaaccgtgagcggccaggtgcatctggatcgcattaaagtggcgaaaggcaaaattctgaccgcgacccgcaaaaccctggatgcgtcattcaacgagaaaaccattgaaagcattaccgataccggcattcagaaaattctgctgaactatctgaaaagcaaagataacaacccggaagtggcgtttagcccggaaggcattgaagaactgaacaaaaacattcgcctgtataacgatggcaaagcgcatcagccgattctgaaagtgcgcgtgtttgaacagggcagcaaattcaccctgggcgaaaccggcaacaaaaccaccaaatttgtggaagcggcgaaaggcaccaacctgttctttggcatctatgaagataaaagcggcaaacgcagctatgaaaccattccgctgaacattgtgattgaacgccagaaacagggcctgcaagcggtgccggaaaccaacgaaaaaggcaaacagctgctgtttaccctgtcaccgaacgatctggtgtatgtgccggaagaaggcgtgtttgatgaaaacaacattaaagtggatcgcatctataaagtggtgagctttagcacctatcagtgcttctttgtgcgcaacgatgtgagcaccagcgtggtgaacaaagtggaatatagcgcgctgaacaaaatggaaaaatcgattgataacattatgattaaagaaaactgcgtgaaactgaacgtggatcgcctgggcaaaattagcaaagcg

SEQ ID NO: 195 - DNA, 4368 bp, Empedobacter sp.
  source: /note="APG01688.1 Native Seq"
atgatgattaaaaatatacttggattagatttggggactaactctattgggtgggcattgataaaacaagattttgaaaataagcatggcgaaattcttggaatgggtagccggattattccgatgtcacaggatattctgggcgattttgggaaaggaaattctatttcgcaaaccgctgatcgtaccaaatacagaagcgtgagaagattacgtgaacgatttttattgaggagagaacgactacacagagttttacatcttttaaattttcttccacagcattatgcttcacaaattgattttgaaaaaaaattcgggaagtttaaatctgaaactgaacccaaattggcatgggaaaattggggtggaaagttttcattccttttccaaaactctttcaatgaaatgcttgaagattttaaagcagctggacagggtttaaaaattccttacgactggacaatttattatctccgtaaaaaagcactttcacaaaaaattgaaaaggaggaactggcctggattcttttaaactttaatcagaaacgaggatattatcaattgcgtggtgaggaagaagaagagaatcctaataagctggttgaattttattctttaaaaattgtagatgttgtagcagatgaacctcaaaaaggaaaatctgatatttggtattctttgattttagagaatggatgggtttacagacgagcaagcaaaatacccctatttgactggaaagataaaacaagagattttattgtaacaactgatttgaatgatgacagaagtgttaaaacagacaaagaaggaaatgaaaaaagaagtttcagagcaccaagcgaaaacgattggacattggtaaaaaagaaaaccgaacaggaaatcgaccaatctcacaaaaccgttggaacctatatctacgaaacacttcttctaaatccgaaacaaaaaattaaaggaaaattggttcggacgattgaaagaaaattctataaagatgagctaaaacaaattttagaaaaacaaaaggaatttcatcaggaacttaaaaatgatgatttgtataatgattgcattcgtgagttgtacagaaacaacgaagcacatcagctgactttgagcaagaaagattttgttcatcttttgatggatgatcttattttctaccaaagacctttgagaagccagaaatcatctatttccaactgtacgttagagtttagaaaatataaagatgaaaatggaatagagcatacacaatatttaaaagccattccaaaatccaatccgtattatcaggaatttcgtctttggcaatggatgtataatctgaatatttacagaaaggacgatgaagcgaatgttaccaaagaatttttaaatacgaacaaagattttgaaagtctgtttgaatttttaaataatagaaaagaaattgagcaaaagccattgattaaatttcttttggaacaaaaagatatcaataaaaaattgcttaacgctgaagcagaaaaatatcgctggaactatgtagaagacaagaaatatccttgcaatgaaaccaaaacgatgatttcttctcgtttggataaagtcgaaaacatttctgatgatttcctgacaagggacattgagcagaaaatttggcacatcatctattccgtcaatgataaaatagaatatgaaaaagctttgaaatcttttgcaactagaaacgatttggatgaaaactcttttatcgaagcgtttaagaaattctcgccttttaaaagtgaatatggttctttttcggaaaaagcaattaaaaagttactgcctttaatgcgattgggtaaatattggtatgaagatgaaattgtaaagcatagtgatatttatttcaaaaatattgagaatcttttgggtgatttttcaaatagagacaaaaaaatttctgaagaagacaaagagaaatggaataaatctataaatctaaagttacaggaagagttaaaagattttcaaacagctgaaatagatttatttcaaggattacgattgcatattgctcaataccttgtttatggaagacattcagaagcttcaatgattggaaaatggaattccgccgaagatttagaagaatttttaaaggattttaaacagcattcgcttcgcaacccgattgtagaacaagtgattacagaaactttgcgtgttgtaaaagatatttggttgaaatacggaaatggagcaaaggatttcttcaatgaaattcatattgagttaggaagagaaatgaaacttcccgcagatgatcgaaaaaaactaacgaaccagatttctgaaaacgaaaataccaatttccgcatcaaagctctattggctgaaatgatgaatgacagttcggtagaaaatgtccgtccgttttcgccgatgcagcaagaaattttaaaaatttatgaagacgatgttttaaaatcagatatagaaattgaagatgatattctgaaaatcagcaaaaccgctcaaccttctccttccgatttgaaacgatataaactttggttggaacagaaatacaaatcgccttacacggggcaaattattcctttgaataaattgtttacaccagaatacgaaattgagcacattattccgcagagccgatattttgatgacagttttagcaataaagtaatttgtgagtctgcggttaataaattgaaagataactacatcggacttgaatttattaagcagttcggaggaacgattattgaacttggttttggtaaaagcataaaagtttttgaaacaaaagaatacgaagatttcgtcaaaaaacattacgccaacaatcaaggtaaaagaaacaaacttttgatggaagatattccagagaaaatgattgaacgtcaaatgaacgatacacgatatatcagcaaatatatttcgggcgttttgtctaatattgttcgggtagaagatggttcagatgaaggggtaaattctaaaaatattgttcccggaaacggaaaaatcaccacacagctgaaacaagattggggattgaatgatgtttggaatgatttgattttaccacgctttgaaagaatgaaccaactcaccaattcaaaagtttttactgcctggaatgagaattatcaaaagtttttaccaactgttcctattgaatattccaaagggttttcaaagaaaagaatagaccaccgccatcacgctttagatgctttggtgattgcctgtgctacaaaagatcacgtgaatttattaaataatcaatcggcaaaatcggataccaaacgatacgatttgaaaaagaaatcgatgaagtttgaaaaagtagtttacaatgatgccaaaacaggagagaaaatcgaaagggaagtgccaaaacaatttttaaaaccttgggaaaattttacgctagatgttaaacataatttggaaactattattgtaagttttaagcaaaatcttcgtgttattaataaagcgactaattattacgaaaagtatgttgagaaagacggtacaaaaaataaggaaagagtagagcagaccggaacaaactgggcgattaggaaaccaatgcataaagacacggtttccggtaaagtagatttaccttgggtaaaagtcccaaaagggaaaattttaacagcaacaaggaaaagccttgatagttcgtttgacttaaagtcaataggctctattacggatacaggaattcagaaaatactcaaaaattatttagcatttaaagacggaaatcctgaactggctttttcaccagaaggaattgacgatttgaataaaaatattgaaaaatacaatgatggaaaaccgcatcaacccatcaataaagtaagggtttttgaattgggaagtaaatttcaggtaggacaaagtggaaataaaaaagataaatatgtagaagctgcaaaaggaactaatctattctttgctgtttatgaagatgaaaaaggaaagagaaattatgaaaccattcctttgaatgaagtgattgaaaggcaaaagcaaggtttatctgtggttgatttaaaaggtacaaatgatttctacttatgtccgaatgattttgtatatattccatcaggcgacgaacttgaaaatataaataatgttgattttaaagacattaaaaaagagataaacgaaagaatttacaaagtagtaagttttacaggtaatagactttcctgtattccatatatggttgcaacaacgattgttaataaattagagtttacgcaacttaataaaattgaattcacaaaagaaaaagaaatttgtataaaactaaatgtcgatcgtttaggtaacatttcaaaagcg

SEQ ID NO: 196 - DNA, 4368 bp, Artificial Sequence
  source: /note="Description of Artificial Sequence: Synthetic polynucleotide"
  source: /note="APG01688.1 E. coli optimized"
atgatgattaaaaatatcctaggcctggacctgggaaccaacagcatcggctgggcgctgattaaacaggacttcgaaaataagcatggcgagatactaggcatgggcagccgaataatcccgatgagtcaggacatactaggcgacttcggcaagggcaacagcatcagccagaccgcggaccgcacaaaatatcgcagcgtgcgtagactgcgcgaacgctttctgttacgtcgtgaacgtctgcatcgtgttcttcacctattaaacttcctgccgcagcattacgctagccagatcgacttcgagaagaagttcggcaagttcaagagcgagaccgaaccaaaactggcgtgggaaaactggggcggcaaattcagcttcctattccaaaatagcttcaacgagatgctagaggacttcaaggcggcgggtcagggattaaaaataccgtacgactggaccatatactacctgcgcaagaaagcgctgagccagaagatcgagaaggaggagctggcgtggatactactgaactttaatcaaaagcgcggatactaccagctgcgcggcgaggaggaggaggagaacccgaataaactggtggagttctacagcctgaaaatagtggacgtggtggcggacgagccgcagaaaggcaaaagcgacatctggtactcactcatactagaaaacggctgggtgtatcgccgcgcgagcaaaataccgctgttcgactggaaagataaaacccgcgacttcatcgtgaccaccgacctgaacgacgaccgcagcgtgaaaaccgacaaagaaggcaatgaaaaacgcagctttcgcgcgccgagcgaaaacgattggaccctggtgaaaaagaaaaccgaacaggaaatcgatcagagccataaaaccgtgggcacatatatctatgaaaccctgttattaaacccgaagcagaagattaaaggcaaactggtgcgcaccatcgaacgcaaattctacaaagacgaattaaaacagatactagaaaaacagaaagaattccaccaggaattaaagaacgacgacttatataacgattgcatccgcgaactgtaccgcaataatgaagcgcaccaattaaccctgagcaaaaaggatttcgtgcacttattaatggatgatctgatcttctaccagcgcccgctgcgcagccagaaatcaagcatcagcaattgcaccctggaattccgcaaatacaaagatgaaaacggcatcgaacacacccagtacctgaaagcgatcccgaaatcaaacccatactaccaggaattccgcctgtggcagtggatgtacaacctgaacatctaccgcaaagatgatgaagcgaacgtaaccaaagaattcctgaacaccaataaagatttcgaaagcctgttcgaattcctgaataatcgcaaagaaatcgaacagaaaccattaatcaaattcctgctggaacagaaagatattaataaaaagttattaaacgcggaagcggaaaaatacagatggaactacgtggaagataaaaagtacccgtgcaatgaaaccaaaaccatgatcagcagccgcctggataaagtggaaaatatcagcgatgatttcctgacccgcgatatcgaacagaaaatatggcatataatctacagcgtgaacgataaaatcgaatatgaaaaagcattaaaatcgttcgcgacccgcaacgatctggatgaaaatagcttcatcgaagcattcaaaaagttcagcccgttcaaaagcgaatacggcagcttcagcgaaaaagcgattaaaaagctgctgccattaatgcgcctgggaaaatactggtacgaagatgaaatcgtgaaacacagcgatatctacttcaaaaacatcgaaaacctgctgggcgatttcagcaaccgcgataaaaagatcagcgaagaagataaagaaaaatggaacaaaagcatcaacctgaaactgcaggaagaactgaaagatttccagaccgcggaaatcgatctgttccagggcctgcgcctgcatatcgcgcagtacctggtgtacggccgccatagcgaagcgagcatgatcggcaaatggaactcagcggaagatctggaagaattcctgaaagatttcaaacagcatagcctgcgcaacccgatcgtggaacaggtgatcaccgaaaccctgcgcgtggtgaaagatatctggctgaaatatggcaacggcgcgaaagatttctttaacgaaattcatatcgaactgggccgcgaaatgaaactgccggcggatgatcgcaaaaagctgaccaaccagatcagcgaaaacgaaaacaccaactttcgcatcaaagcgctgctggcggaaatgatgaacgatagcagcgtggaaaacgtgcgcccgtttagcccgatgcagcaggaaatcctgaaaatctatgaagatgatgtgctgaaaagcgatatcgaaatcgaagatgatatcttaaaaatcagcaaaaccgcgcagccgagcccgagcgatctgaaacgctataaactgtggctggaacagaaatataaaagcccgtataccggccagatcatcccgctgaacaaactgtttaccccggaatatgaaatcgaacatatcatcccgcagagccgctattttgatgatagctttagcaacaaagtgatctgcgaaagcgcggtgaacaaactgaaagataactatatcggcctggaattcatcaaacagtttggcggcaccatcatcgaactgggctttggcaaaagcatcaaagtgtttgaaaccaaagaatatgaagattttgtgaaaaagcattatgcgaacaaccagggcaaacgcaacaaactgttaatggaagatatcccggagaaaatgatcgaacgccagatgaacgatacccgctatatcagcaaatatatcagcggcgtgctgagcaacatcgtgcgcgtggaagatggcagcgatgaaggcgtgaacagcaaaaacatcgtgccgggcaacggcaaaatcaccacccagctgaaacaggattggggcctgaacgatgtgtggaacgatctgatcctgccgcgctttgaacgcatgaaccagctgaccaacagcaaagtgtttaccgcgtggaacgaaaactatcagaaatttctgccgaccgtgccgattgaatatagcaaaggctttagcaaaaagcgcattgatcatcgccatcatgcgctggatgcgttagtgattgcgtgcgcgaccaaagatcatgtgaacctgctgaacaaccagagcgcgaaaagcgataccaaacgctatgatctgaaaaagaaaagcatgaaatttgaaaaagtggtgtataacgatgcgaaaaccggcgagaaaattgaacgcgaagtgccgaaacagtttctgaaaccgtgggaaaactttaccctggatgtgaaacataacctggaaaccattattgtgagctttaaacagaacctgcgcgtgattaacaaagcgaccaactattatgaaaaatatgtggaaaaagatggcaccaaaaacaaagaacgcgtggaacagaccggcaccaactgggcgattcgcaaaccgatgcataaagataccgtgtcaggcaaagtggatctgccgtgggtgaaagtgccgaaaggcaaaattctgaccgcgacccgcaaaagcctggatagcagctttgatctgaaaagcattggcagcattaccgataccggcattcagaaaattctgaaaaactatctggcgtttaaagatggcaacccggaactggcgtttagcccggaaggcattgatgatctgaacaaaaacattgaaaaatataacgatggcaaaccgcatcagccgattaacaaagtgcgcgtgtttgaactgggcagcaaatttcaggtgggccagagcggcaacaaaaaggacaaatatgtggaagcggcgaaaggcaccaacctgttctttgcggtgtatgaagatgaaaaaggcaaacgcaactatgaaaccatcccgttaaacgaagtgattgaacgccagaaacagggcctgagcgtggtggatctgaaaggcaccaacgatttttatctgtgcccgaacgattttgtgtatattccgagcggcgatgaactggaaaacattaacaacgtggattttaaagatattaaaaaggaaattaacgaacgcatctataaagtggtgagctttaccggcaaccgcctgagctgcattccgtatatggtggcgaccaccattgtgaacaaactggaattcacccagctgaacaaaattgaattcaccaaagaaaaagaaatttgcattaaactgaacgtggatcgcctgggcaacattagcaaagcg

SEQ ID NO: 197 - DNA, 25 bp, Homo sapiens
  source: /note="target seq for Ataxia-telangiectasia syndrome"
gaattattccagaaagccaaagtag

SEQ ID NO: 198 - DNA, 20 bp, Homo sapiens
  source: /note="target seq for Very long chain acyl-CoA dehydrogenase deficiency"
ggcttcatgaaggtacagga

SEQ ID NO: 199 - DNA, 25 bp, Homo sapiens
  source: /note="target seq for Abnormality of T cell physiology"
ggtgtgctcaccagaatggagtaca

SEQ ID NO: 200 - DNA, 25 bp, Homo sapiens
  source: /note="target seq for Cardiovascular phenotype"
gcagatcattggggtggatcccgaa

SEQ ID NO: 201 - DNA, 25 bp, Homo sapiens
  source: /note="target seq for 3-Oxo-5 alpha-steroid delta 4-dehydrogenase deficiency"
ggctgcaagcttttcaccaccayag

SEQ ID NO: 202 - DNA, 25 bp, Homo sapiens
  source: /note="target seq for Acute myeloid leukemia"
gggcggcatgaaccggaggcccatc

SEQ ID NO: 203 - DNA, 20 bp, Homo sapiens
  source: /note="target seq for Acute myeloid leukemia"
gcatgggcggcatgaaccgg

SEQ ID NO: 204 - DNA, 20 bp, Homo sapiens
  source: /note="target seq for Cutaneous malignant melanoma 3"
gtggccactgtggggatcac

SEQ ID NO: 205 - DNA, 20 bp, Homo sapiens
  source: /note="target seq for Alpha-1-antitrypsin deficiency"
gtgctgaccatcgacgagaa

SEQ ID NO: 206 - DNA, 20 bp, Homo sapiens
  source: /note="target seq for Charcot-Marie-Tooth disease, type 2"
ggcgagctgcatgatctgcg

SEQ ID NO: 207 - DNA, 25 bp, Homo sapiens
  source: /note="target seq for Hereditary cancer-predisposing syndrome"
gcacatgacggaggttgtgaggcgc

SEQ ID NO: 208 - DNA, 25 bp, Homo sapiens
  source: /note="target seq for Hereditary cancer-predisposing syndrome"
gaggttgtgaggcactgcccccacc

SEQ ID NO: 209 - DNA, 20 bp, Homo sapiens
  source: /note="target seq for Hereditary cancer-predisposing syndrome"
gcagcatccggctgcaggta

SEQ ID NO: 210 - DNA, 25 bp, Homo sapiens
  source: /note="target seq for Brugada syndrome"
ggccaaggggatccgcacgctgctc

SEQ ID NO: 211 - DNA, 20 bp, Homo sapiens
  source: /note="target seq for Brugada syndrome"
gcctgatgacgcaggactgc

SEQ ID NO: 212 - DNA, 20 bp, Homo sapiens
  source: /note="target seq for GRACILE syndrome"
ggtacgaagtctcgacactg

SEQ ID NO: 213 - DNA, 20 bp, Homo sapiens
  source: /note="target seq for Enhanced s-cone syndrome"
ggcattggcggtggacccca

SEQ ID NO: 214 - DNA, 25 bp, Homo sapiens
  source: /note="target seq for Charcot-Marie-Tooth disease, type 2"
gaagaacaggttctggacgtcaaag

SEQ ID NO: 215 - DNA, 20 bp, Homo sapiens
  source: /note="target seq for Charcot-Marie-Tooth disease, type 2"
gaacaggttctggacgtcaa

SEQ ID NO: 216 - DNA, 20 bp, Homo sapiens
  source: /note="target seq for Arylsulfatase a, allele a"
gacaggtcatagagcagcgg

SEQ ID NO: 217 - DNA, 20 bp, Homo sapiens
  source: /note="target seq for Familial hypercholesterolemia"
gaacgtggtcgctctggaca

SEQ ID NO: 218 - DNA, 20 bp, Homo sapiens
  source: /note="target seq for Familial hypercholesterolemia"
gaacgtggtcgctctggaca

SEQ ID NO: 219 - DNA, 25 bp, Homo sapiens
  source: /note="target seq for HEMOGLOBIN ARLINGTON PARK"
ggtgcatctgactcctgaggagaag

SEQ ID NO: 220 - DNA, 20 bp, Homo sapiens
  source: /note="target seq for Familial hypertrophic cardiomyopathy 1"
gaagtccgaggctcgccgca

SEQ ID NO: 221 - DNA, 20 bp, Homo sapiens
  source: /note="target seq for Cardiovascular phenotype"
gtcaaggtcatcggtgaggc

SEQ ID NO: 222 - DNA, 25 bp, Homo sapiens
  source: /note="target seq for Cardiovascular phenotype"
ggtcatcagtgaggccggccggggt

SEQ ID NO: 223 - DNA, 25 bp, Homo sapiens
  source: /note="target seq for Brugada syndrome"
gtctcagccttacgcaccttccgag

SEQ ID NO: 224 - DNA, 25 bp, Homo sapiens
  source: /note="target seq for Brugada syndrome"
gcaccttccaagtcctccgggccct

SEQ ID NO: 225 - DNA, 26 bp, Homo sapiens
  source: /note="target seq for Hereditary cancer-predisposing syndrome"
gaagccagcccctcagggcaactgac

SEQ ID NO: 226 - DNA, 20 bp, Homo sapiens
  source: /note="target seq for Deficiency of butyryl-CoA dehydrogenase"
ggcgactcatgggttctgaa

SEQ ID NO: 227 - DNA, 25 bp, Homo sapiens
  source: /note="target seq for Deficiency of butyryl-CoA dehydrogenase"
gcgactcacgggttctgaatggaac

SEQ ID NO: 228 - DNA, 20 bp, Homo sapiens
  source: /note="target seq for Benign scapuloperoneal muscular dystrophy with cardiomyopathy"
ggaactgcgggcccagcatg

SEQ ID NO: 229 - DNA, 20 bp, Homo sapiens
  source: /note="target seq for Benign scapuloperoneal muscular dystrophy with cardiomyopathy"
ggacgagtaccaggagcttc

SEQ ID NO: 230 - DNA, 20 bp, Homo sapiens
  source: /note="target seq for Cone-rod dystrophy 6"
ggatctgatccgggagcgca

SEQ ID NO: 231 - DNA, 25 bp, Homo sapiens
  source: /note="target seq for Cone-rod dystrophy 6"
gaatgcactatgttctattccatcc

SEQ ID NO: 232 - DNA, 25 bp, Homo sapiens
  source: /note="target seq for Stargardt disease 1"
gagctgctcacaggacgagaacatc

SEQ ID NO: 233 - DNA, 20 bp, Homo sapiens
  source: /note="target seq for Leber congenital amaurosis 2"
gtctatccagtaagtatctc

SEQ ID NO: 234 - DNA, 20 bp, Homo sapiens
  source: /note="target seq for Cone-rod dystrophy 3"
ggtacgtccatgccacaccc

SEQ ID NO: 235 - DNA, 20 bp, Homo sapiens
  source: /note="target seq for Nonsyndromic Oculocutaneous Albinism"
ggacctttacggcgtaatcc

SEQ ID NO: 236 - DNA, 20 bp, Homo sapiens
  source: /note="target seq for Phenylketonuria"
gtcatcctttggtgaattac

SEQ ID NO: 237 - DNA, 25 bp, Homo sapiens
  source: /note="target seq for Phenylketonuria"
gtattacgtggcagagagttttaat

SEQ ID NO: 238 - DNA, 20 bp, Homo sapiens
  source: /note="target seq for Breast-ovarian cancer, familial 1"
ggacgctcttgtattatctg

SEQ ID NO: 239 - DNA, 25 bp, Homo sapiens
  source: /note="target seq for Hyperphenylalaninemia, non-pku"
gcccttctcagttcgctacgaccca

SEQ ID NO: 240 - DNA, 20 bp, Homo sapiens
  source: /note="target seq for Hyperphenylalaninemia, non-pku"
gctacgacccatacacccaa

SEQ ID NO: 241 - DNA, 20 bp, Homo sapiens
  source: /note="target seq for Hereditary cancer-predisposing syndrome"
gcgctatgttctattccatc

SEQ ID NO: 242 - DNA, 25 bp, Homo sapiens
  source: /note="target seq for Hereditary cancer-predisposing syndrome"
ggggctggtattcatgaaaggcaac

SEQ ID NO: 243 - DNA, 20 bp, Homo sapiens
  source: /note="target seq for Hereditary cancer-predisposing syndrome"
gcgctatgttctattccatc

SEQ ID NO: 244 - DNA, 25 bp, Homo sapiens
  source: /note="target seq for Hereditary cancer-predisposing syndrome"
gtgttctcaggttatcggtaagttt

SEQ ID NO: 245 - DNA, 25 bp, Homo sapiens
  source: /note="target seq for Hereditary cancer-predisposing syndrome"
ggaaatgctgttagtcggtatgtcg

SEQ ID NO: 246 - DNA, 25 bp, Homo sapiens
  source: /note="target seq for Hereditary cancer-predisposing syndrome"
ggaaatgctgttagtcagtatgtcg

SEQ ID NO: 247 - DNA, 20 bp, Homo sapiens
  source: /note="target seq for Anterior segment dysgenesis 6"
gtggccactgatcggaaacg

SEQ ID NO: 248 - DNA, 25 bp, Homo sapiens
  source: /note="target seq for Brugada syndrome"
gaacctgatcctggccgtggtcgca

SEQ ID NO: 249 - DNA, 20 bp, Homo sapiens
  source: /note="target seq for Brugada syndrome"
gatcctggccgtggtcgcaa

SEQ ID NO: 250 - DNA, 25 bp, Homo sapiens
  source: /note="target seq for Ornithine carbamoyltransferase deficiency"
gaagggccatgaccttctcactcta

SEQ ID NO: 251 - DNA, 25 bp, Homo sapiens
  source: /note="target seq for Osteogenesis imperfecta type I"
ggtgctcgaggattgcccggaacag

SEQ ID NO: 252 - DNA, 25 bp, Homo sapiens
  source: /note="target seq for Osteogenesis imperfecta type I"
gctcgaggattgcccggaacagctg

SEQ ID NO: 253 - DNA, 25 bp, Homo sapiens
  source: /note="target seq for Constipation"
gattccagttaaatggatggcaatt

SEQ ID NO: 254 - DNA, 25 bp, Homo sapiens
  source: /note="target seq for Dopamine beta hydroxylase deficiency"
ggacactgcctattttgcggtgagt

SEQ ID NO: 255 - DNA, 25 bp, Homo sapiens
  source: /note="target seq for Cystic fibrosis"
gacttcatccaggtatgtaaaaata

SEQ ID NO: 256 - DNA, 25 bp, Homo sapiens
  source: /note="target seq for Phenylketonuria"
gatgtaaacctgacccacactgaat

SEQ ID NO: 257 - DNA, 20 bp, Homo sapiens
  source: /note="target seq for Deficiency of UDPglucose-hexose-1-phosphate uridylyltransferase"
gagcccctgacacccttacc

SEQ ID NO: 258 - DNA, 20 bp, Homo sapiens
  source: /note="target seq for Amyloid Cardiomyopathy, Transthyretin-related"
gtcaccaatcccaaggaatg

SEQ ID NO: 259 - DNA, 25 bp, Homo sapiens
  source: /note="target seq for Carbohydrate-deficient glycoprotein syndrome type I"
ggctactccatgacagcgcctgagg

SEQ ID NO: 260 - DNA, 25 bp, Homo sapiens
  source: /note="target seq for Metachromatic leukodystrophy"
gcatcccgtactcccacgaccagat

SEQ ID NO: 261 - DNA, 25 bp, Homo sapiens
  source: /note="target seq for Smith-Lemli-Opitz syndrome"
gttcttcaatgggcgccccgggatc

SEQ ID NO: 262 - DNA, 20 bp, Homo sapiens
  source: /note="target seq for Deafness, autosomal recessive 1A"
gcaggtgagcccgccggccc

SEQ ID NO: 263 - DNA, 25 bp, Homo sapiens
  source: /note="target seq for Congenital omphalocele"
gccagcgctcctagtggccatgcac

SEQ ID NO: 264 - DNA, 25 bp, Homo sapiens
  source: /note="target seq for Congenital omphalocele"
gcgctcctagtggccatgcacgtgg

SEQ ID NO: 265 - DNA, 20 bp, Homo sapiens
  source: /note="target seq for Congenital omphalocele"
gtccacgccagcgctcctag

SEQ ID NO: 266 - DNA, 20 bp, Homo sapiens
  source: /note="target seq for Congenital omphalocele"
gctcctagtggccatgcacg

SEQ ID NO: 267 - DNA, 25 bp, Homo sapiens
  source: /note="target seq for Congenital myotonia, autosomal dominant form"
gagaggattctttgcagccacgttc

SEQ ID NO: 268 - DNA, 20 bp, Homo sapiens
  source: /note="target seq for Breast-ovarian cancer, familial 1"
ggtgacccgagagtgggtgt

SEQ ID NO: 269 - DNA, 20 bp, Homo sapiens
  source: /note="target seq for Breast and/or ovarian cancer"
gatgcctggacagaggacaa

SEQ ID NO: 270 - DNA, 20 bp, Homo sapiens
  source: /note="target seq for Breast-ovarian cancer, familial 1"
ggacaatggcttccatggta

SEQ ID NO: 271 - DNA, 20 bp, Homo sapiens
  source: /note="target seq for Breast-ovarian cancer, familial 1"
gggctagaaatctgttgcta

SEQ ID NO: 272 - DNA, 20 bp, Homo sapiens
  source: /note="target seq for Breast-ovarian cancer, familial 1"
ggtgacccgagagtgggtgt

SEQ ID NO: 273 - DNA, 20 bp, Homo sapiens
  source: /note="target seq for Breast-ovarian cancer, familial 1"
gattctgcaactttcaattg

SEQ ID NO: 274 - DNA, 20 bp, Homo sapiens
  source: /note="target seq for Breast-ovarian cancer, familial 1"
ggacaatggcttccatggta

SEQ ID NO: 275 - DNA, 25 bp, Homo sapiens
  source: /note="target seq for Inborn genetic diseases"
gaaagcccgacttatagccagtaat

SEQ ID NO: 276 - DNA, 20 bp, Homo sapiens
  source: /note="target seq for Breast-ovarian cancer, familial 2"
gattacatgaacaaatgggc

SEQ ID NO: 277 - DNA, 20 bp, Homo sapiens
  source: /note="target seq for Breast-ovarian cancer, familial 2"
gattacatgaacaaatgggc

SEQ ID NO: 278 - DNA, 20 bp, Homo sapiens
  source: /note="target seq for Breast-ovarian cancer, familial 2"
gactggaaaaggaatacagt

SEQ ID NO: 279 - DNA, 25 bp, Homo sapiens
  source: /note="target seq for Breast and/or ovarian cancer"
gttggctgatggtggatggctcata

SEQ ID NO: 280 - DNA, 25 bp, Homo sapiens
  source: /note="target seq for Breast-ovarian cancer, familial 2"
gttggctgatggtggatggctcata

SEQ ID NO: 281 - DNA, 20 bp, Homo sapiens
  source: /note="target seq for Breast-ovarian cancer, familial 2"
ggtcagaagattattcttca

SEQ ID NO: 282 - DNA, 20 bp, Homo sapiens
  source: /note="target seq for Breast-ovarian cancer, familial 2"
ggcttctagtctcttttgtt

SEQ ID NO: 283 - DNA, 20 bp, Homo sapiens
  source: /note="target seq for Breast-ovarian cancer, familial 2"
ggcttctagtctcttttgtt

SEQ ID NO: 284 - DNA, 20 bp, Homo sapiens
  source: /note="target seq for Smith-Lemli-Opitz syndrome"
gttgcgattttgcagccatt

SEQ ID NO: 285 - DNA, 25 bp, Homo sapiens
  source: /note="target seq for Alport syndrome 1, X-linked recessive"
ggcctatgggtccccctggtttcgg

SEQ ID NO: 286 - DNA, 20 bp, Homo sapiens
  source: /note="target seq for Acute neuronopathic Gaucher's disease"
ggcatcaggtgagtgagtca

SEQ ID NO: 287 - DNA, 20 bp, Homo sapiens
  source: /note="target seq for Gonadotropin deficiency"
gtaactctccagcataccat

SEQ ID NO: 288 - DNA, 20 bp, Homo sapiens
  source: /note="target seq for Distal arthrogryposis type 1A"
gaagctggaggaggccgaga

SEQ ID NO: 289 - DNA, 20 bp, Homo sapiens
  source: /note="target seq for Distal arthrogryposis type 1A"
gctggaggaggccgagaagg

SEQ ID NO: 290 - DNA, 20 bp, Homo sapiens
  source: /note="target seq for Hereditary cancer-predisposing syndrome"
gctgccaccttcagggcctc

SEQ ID NO: 291 - DNA, 20 bp, Homo sapiens
  source: /note="target seq for Inborn genetic diseases"
gataaacttcttgaagagga

SEQ ID NO: 292 - DNA, 25 bp, Homo sapiens
  source: /note="target seq for Death in early adulthood"
gtgttctccatgttcgaacagaccc

SEQ ID NO: 293 - DNA, 20 bp, Homo sapiens
  source: /note="target seq for Death in early adulthood"
gttcgaacagacccaaatcc

SEQ ID NO: 294 - DNA, 20 bp, Homo sapiens
  source: /note="target seq for Severe autosomal recessive muscular dystrophy of childhood - North African type"
gaaatctgtgtgtgtccaga

SEQ ID NO: 295 - DNA, 20 bp, Homo sapiens
  source: /note="target seq for Cardiovascular phenotype"
ggtcatcattgagagcgacc

SEQ ID NO: 296 - DNA, 20 bp, Homo sapiens
  source: /note="target seq for Carbohydrate-deficient glycoprotein syndrome type I"
gaatgctgaagatgatcgac

SEQ ID NO: 297 - DNA, 20 bp, Homo sapiens
  source: /note="target seq for Charcot-Marie-Tooth disease, type I"
gaatgctgaagatgatcgac

SEQ ID NO: 298 - DNA, 25 bp, Homo sapiens
  source: /note="target seq for Inborn genetic diseases"
gctcagtacaccaccgtcggccgca

SEQ ID NO: 299 - DNA, 20 bp, Homo sapiens
  source: /note="target seq for Inborn genetic diseases"
gtacaccaccgtcggccgca

SEQ ID NO: 300 - DNA, 25 bp, Homo sapiens
  source: /note="target seq for Familial Mediterranean fever"
ggacacgtgatggagggaagaacac

SEQ ID NO: 301 - DNA, 25 bp, Homo sapiens
  source: /note="target seq for Deafness, autosomal recessive 2"
ggacctttgtcaatgggacacggac

SEQ ID NO: 302 - DNA, 25 bp, Homo sapiens
  source: /note="target seq for Deafness, autosomal recessive 2"
ggacctttgtcaatgggacacagac

SEQ ID NO: 303 - DNA, 25 bp, Homo sapiens
  source: /note="target seq for Deafness, X-linked 2"
gcgctcctagtggccatgcacgtgg

SEQ ID NO: 304 - DNA, 25 bp, Homo sapiens
  source: /note="target seq for Enlarged vestibular aqueduct"
gccaccactgctctttcccgcacgg

SEQ ID NO: 305 - DNA, 20 bp, Homo sapiens
  source: /note="target seq for Congenital sensorineural hearing impairment"
gtggtcattaacacaaactc

SEQ ID NO: 306 - DNA, 20 bp, Homo sapiens
  source: /note="target seq for Deficiency of UDPglucose-hexose-1-phosphate uridylyltransferase"
gccagatattgcccagcgtg

SEQ ID NO: 307 - DNA, 20 bp, Homo sapiens
  source: /note="target seq for Very long chain acyl-CoA dehydrogenase deficiency"
gccactaatcgtacccagtt

SEQ ID NO: 308 - DNA, 20 bp, Homo sapiens
  source: /note="target seq for Cardiovascular phenotype"
gatattccactggtggtcga

SEQ ID NO: 309 - DNA, 20 bp, Homo sapiens
  source: /note="target seq for Pyruvate kinase deficiency of red cells"
ggaagactcctgggcataag

SEQ ID NO: 310 - DNA, 25 bp, Homo sapiens
  source: /note="target seq for Autosomal dominant progressive external ophthalmoplegia with mitochondrial DNA deletions 1"
gaagtcgttgatggatctggccaat

SEQ ID NO: 311 - DNA, 20 bp, Homo sapiens
  source: /note="target seq for Very long chain acyl-CoA dehydrogenase deficiency"
gaagatcacagcttttgtgg

SEQ ID NO: 312 - DNA, 20 bp, Homo sapiens
  source: /note="target seq for Cystinosis, ocular nonnephropathic"
gtccatctccttctaccctc

SEQ ID NO: 313 - DNA, 20 bp, Homo sapiens
  source: /note="target seq for Pyruvate kinase deficiency of red cells"
gctcagcccagcttctgtct

SEQ ID NO: 314 - DNA, 25 bp, Homo sapiens
  source: /note="target seq for Distal myopathy, Tateyama type"
gattgacctggtgaaccaagacccc

SEQ ID NO: 315 - DNA, 25 bp, Homo sapiens
  source: /note="target seq for Malignant hyperthermia, susceptibility to, 1"
ggccctgcggatccgcgccatcctc

SEQ ID NO: 316 - DNA, 25 bp, Homo sapiens
  source: /note="target seq for Malignant hyperthermia, susceptibility to, 1"
ggatccgcgccatcctccgctccct

SEQ ID NO: 317 - DNA, 25 bp, Homo sapiens
  source: /note="target seq for Myopathy, Central Core"
ggtctgatcatcgacgcttttggtg

SEQ ID NO: 318 - DNA, 20 bp, Homo sapiens
  source: /note="target seq for Myopathy, Central Core"
ggtctgatcatcgacgcttt

SEQ ID NO: 319 - DNA, 25 bp, Homo sapiens
  source: /note="target seq for Myopathy, Central Core"
gatcatcgacacttttggtgagctc

SEQ ID NO: 320 - DNA, 25 bp, Homo sapiens
  source: /note="target seq for Malignant hyperthermia, susceptibility to, 1"
ggcggaggcattggggacgagatcg

SEQ ID NO: 321 - DNA, 20 bp, Homo sapiens
  source: /note="target seq for Ceroid lipofuscinosis neuronal 2"
gtgacagtggggccgggtgt

SEQ ID NO: 322 - DNA, 25 bp, Homo sapiens
  source: /note="target seq for Ceroid lipofuscinosis neuronal 2"
ggggccgggtattggtctgtctctg

SEQ ID NO: 323 - DNA, 25 bp, Homo sapiens
  source: /note="target seq for Niemann-Pick disease type C1"
ggatcgacgattatttcgactgggt

SEQ ID NO: 324 - DNA, 25 bp, Homo sapiens
  source: /note="target seq for Glutaric aciduria, type 1"
gagtatcacgtgatccggcacgcca

SEQ ID NO: 325 - DNA, 25 bp, Homo sapiens
  source: /note="target seq for CAPN3-Related Disorders"
gccctgatgcagaagaaccggcgga

SEQ ID NO: 326 - DNA, 20 bp, Homo sapiens
  source: /note="target seq for CAPN3-Related Disorders"
gatgcagaagaaccggcgga

SEQ ID NO: 327 - DNA, 20 bp, Homo sapiens
  source: /note="target seq for Glycogen storage disease, type II"
gtcccagaacagctcccctc

SEQ ID NO: 328 - DNA, 25 bp, Homo sapiens
  source: /note="target seq for Nonsyndromic Oculocutaneous Albinism"
gtacagggatctgccaacgatccta

SEQ ID NO: 329 - DNA, 20 bp, Homo sapiens
  source: /note="target seq for Familial hypercholesterolemia"
gcgaagatggctcggatgag

SEQ ID NO: 330 - DNA, 20 bp, Homo sapiens
  source: /note="target seq for Familial hypercholesterolemia"
gagtggccgcagcgctgtag

SEQ ID NO: 331 - DNA, 20 bp, Homo sapiens
  source: /note="target seq for Deafness, autosomal recessive 7"
ggtctcaagctctctcttcg

SEQ ID NO: 332 - DNA, 20 bp, Homo sapiens
  source: /note="target seq for Chronic infantile neurological, cutaneous and articular syndrome"
gacggcttcgatgagctgca

SEQ ID NO: 333 - DNA, 20 bp, Homo sapiens
  source: /note="target seq for Eichsfeld type congenital muscular dystrophy"
gactctccgggagactgtcc

SEQ ID NO: 334 - DNA, 20 bp, Homo sapiens
  source: /note="target seq for Inborn genetic diseases"
gctcaaaagtggatgagcgc

SEQ ID NO: 335 - DNA, 20 bp, Homo sapiens
  source: /note="target seq for Hyperkalemic Periodic Paralysis Type 1"
gcagctgcgggtcttcaagc

SEQ ID NO: 336 - DNA, 20 bp, Homo sapiens
  source: /note="target seq for Inclusion body myopathy 2"
ggacgtggatgtggtggttt

SEQ ID NO: 337 - DNA, 25 bp, Homo sapiens
  source: /note="target seq for Severe APG05083.1, APG07433.1, APG07513.1, APG08290.1 immunodeficiency due to ADA Deficiency"
gaagagcggcattcaccgtactgtc

SEQ ID NO: 338 - DNA, 25 bp, Homo sapiens
  source: /note="target seq for Severe APG05083.1, APG07433.1, APG07513.1, APG08290.1 immunodeficiency due to ADA Deficiency"
gcggtacagtccgcacctgctggcc

SEQ ID NO: 339 - DNA, 20 bp, Homo sapiens
  source: /note="target seq for Cardiovascular phenotype"
gtgtccgagcagcgccactg

SEQ ID NO: 340 - DNA, 20 bp, Homo sapiens
  source: /note="target seq for Cystic fibrosis"
ggacacttcgtgccttcgga

SEQ ID NO: 341 - DNA, 20 bp, Homo sapiens
  source: /note="target seq for Cystic fibrosis"
ggacacttcgtgccttcgga

SEQ ID NO: 342 - DNA, 25 bp, Homo sapiens
  source: /note="target seq for Adrenocortical carcinoma, pediatric"
gggcgtgagcacttcgagatgttcc

SEQ ID NO: 343 - DNA, 20 bp, Homo sapiens
  source: /note="target seq for Fumarase deficiency"
gattggacgtactcatactc

SEQ ID NO: 344 - DNA, 20 bp, Homo sapiens
  source: /note="target seq for Adenocarcinoma of prostate"
gaacactgtccattggcatg

SEQ ID NO: 345 - DNA, 20 bp, Homo sapiens
  source: /note="target seq for Familial hypertrophic cardiomyopathy 1"
gcatcctctacggggacttc

SEQ ID NO: 346 - DNA, 25 bp, Homo sapiens
  source: /note="target seq for Adult hypophosphatasia"
gacaacgagatgccccctgaggcct

SEQ ID NO: 347 - DNA, 25 bp, Homo sapiens
  source: /note="target seq for Adult hypophosphatasia"
ggtactcagacaacaagatgccccc

SEQ ID NO: 348 - DNA, 25 bp, Homo sapiens
  source: /note="target seq for Adult hypophosphatasia"
gacaacaagatgccccctgaggcct

SEQ ID NO: 349 - DNA, 25 bp, Homo sapiens
  source: /note="target seq for Inborn genetic diseases"
gccttcttggacaacgtcaccacca

SEQ ID NO: 350 - DNA, 25 bp, Homo sapiens
  source: /note="target seq for Inborn genetic diseases"
ggtttgccatccgaggggtagtgct

SEQ ID NO: 351 - DNA, 20 bp, Homo sapiens
  source: /note="target seq for Crouzon syndrome"
gcaaatgcctccacagtggt

SEQ ID NO: 352 - DNA, 20 bp, Homo sapiens
  source: /note="target seq for Propionyl-CoA carboxylase deficiency"
gacatcataggcacctccat

SEQ ID NO: 353 - DNA, 25 bp, Homo sapiens
  source: /note="target seq for Cardiovascular phenotype"
ggtggaagggatcggctacgacttc

SEQ ID NO: 354 - DNA, 25 bp, Homo sapiens
  source: /note="target seq for Dysostosis multiplex"
ggagcagctctgggccgaagtgtcg

SEQ ID NO: 355 - DNA, 20 bp, Homo sapiens
  source: /note="target seq for Multiple sulfatase deficiency"
ggcgactcctttgtctttga

SEQ ID NO: 356 - DNA, 20 bp, Homo sapiens
  source: /note="target seq for Bifunctional peroxisomal enzyme deficiency"
ggtggtactggtcaccggcg

SEQ ID NO: 357 - DNA, 25 bp, Homo sapiens
  source: /note="target seq for Bifunctional peroxisomal enzyme deficiency"
gtactggtcaccagcgcgggggcag

SEQ ID NO: 358 - DNA, 20 bp, Homo sapiens
  source: /note="target seq for Hereditary cancer-predisposing syndrome"
ggaaacttgtaagggcttcg

SEQ ID NO: 359 - DNA, 25 bp, Homo sapiens
  source: /note="target seq for Cardiovascular phenotype"
gtgcagacattgacgaatgccgcat

SEQ ID NO: 360 - DNA, 25 bp, Homo sapiens
  source: /note="target seq for Cardiovascular phenotype"
gacattgacgaatgccgcatatctc

SEQ ID NO: 361 - DNA, 20 bp, Homo sapiens
  source: /note="target seq for Limb-girdle muscular dystrophy, type 2L"
gcatagtagtaaactagacg

SEQ ID NO: 362 - DNA, 25 bp, Homo sapiens
  source: /note="target seq for Familial hypercholesterolemia"
gcatcgatgtcaacgagggcaaccg

SEQ ID NO: 363 - DNA, 20 bp, Homo sapiens
  source: /note="target seq for Spastic Paraplegia, Recessive"
gcactgctgctcggcccccc

SEQ ID NO: 364 - DNA, 20 bp, Homo sapiens
  source: /note="target seq for Isovaleryl-CoA dehydrogenase deficiency"
ggagcagtggggctcagtta

SEQ ID NO: 365 - DNA, 20 bp, Homo sapiens
  source: /note="target seq for Familial hypercholesterolemia"
gaggagctgcctcacaggtg

SEQ ID NO: 366 - DNA, 20 bp, Homo sapiens
  source: /note="target seq for Biotinidase deficiency"
gctccagcgcctgagttgta

SEQ ID NO: 367 - DNA, 20 bp, Homo sapiens
  source: /note="target seq for Biotinidase deficiency"
gcctgagttgtatggccatc

SEQ ID NO: 368 - DNA, 25 bp, Homo sapiens
  source: /note="target seq for Leber congenital amaurosis"
gcataatttgtacagctctaagagt

SEQ ID NO: 369 - DNA, 25 bp, Homo sapiens
  source: /note="target seq for Familial hyperinsulinism"
ggtggctgagcccagcccggccccc

SEQ ID NO: 370 - DNA, 25 bp, Homo sapiens
  source: /note="target seq for Familial cancer of breast"
ggatgcttggcagtgggaaaaactt

SEQ ID NO: 371 - DNA, 20 bp, Homo sapiens
  source: /note="target seq for Cohen syndrome"
ggaggtctactacaggtctg

SEQ ID NO: 372 - DNA, 25 bp, Homo sapiens
  source: /note="target seq for Cardiovascular phenotype"
gctccctctgtactgtgcaggagtc

SEQ ID NO: 373 - DNA, 20 bp, Homo sapiens
  source: /note="target seq for Wilson disease"
ggcaatgaacacaaagagca

SEQ ID NO: 374 - DNA, 25 bp, Homo sapiens
  source: /note="target seq for Wilson disease"
gccctggatgggctcagcggccatg

SEQ ID NO: 375 - DNA, 20 bp, Homo sapiens
  source: /note="target seq for Wilson disease"
gcagccctggatgggctcag

SEQ ID NO: 376 - DNA, 20 bp, Homo sapiens
  source: /note="target seq for Familial hypercholesterolemia"
gtggcccagcgaagatgcga

SEQ ID NO: 377 - DNA, 20 bp, Homo sapiens
  source: /note="target seq for Familial hypercholesterolemia"
gaagatgcgaaggtgatttc

SEQ ID NO: 378 - DNA, 20 bp, Homo sapiens
  source: /note="target seq for Floating-Harbor syndrome"
gctgaagctggagtgggtcg

SEQ ID NO: 379 - DNA, 25 bp, Homo sapiens
  source: /note="target seq for Congenital long QT syndrome"
gatgctacacgtcgaccgccaggga

SEQ ID NO: 380 - DNA, 20 bp, Homo sapiens
  source: /note="target seq for Congenital long QT syndrome"
gatgctacacgtcgaccgcc

SEQ ID NO: 381 - DNA, 25 bp, Homo sapiens
  source: /note="target seq for Andersen Tawil syndrome"
gaggaagagatcaaggtcctttcca

SEQ ID NO: 382 - DNA, 25 bp, Homo sapiens
  source: /note="target seq for Cardiovascular phenotype"
gagctgataaccaccctgtacatcg

SEQ ID NO: 383 - DNA, 20 bp, Homo sapiens
  source: /note="target seq for Familial hypercholesterolemia"
ggaaaactgcggtatgggcg

SEQ ID NO: 384 - DNA, 25 bp, Homo sapiens
  source: /note="target seq for Cardiovascular phenotype"
gtatttgaaggtctcctccggggtc

SEQ ID NO: 385 - DNA, 20 bp, Homo sapiens
  source: /note="target seq for Gastrointestinal stroma tumor"
gagggctaaagtgggctcgg

SEQ ID NO: 386 - DNA, 20 bp, Homo sapiens
  source: /note="target seq for Dyskeratosis congenita"
gctgccaagcctgctggcaa

SEQ ID NO: 387 - DNA, 25 bp, Homo sapiens
  source: /note="target seq for Dyskeratosis congenita"
gccctgcctgtgacttccagcactg

SEQ ID NO: 388 - DNA, 25 bp, Homo sapiens
  source: /note="target seq for Glycogen storage disease IIIa"
gatgagtagaacagaaaaatacaag

SEQ ID NO: 389 - DNA, 25 bp, Homo sapiens
  source: /note="target seq for Dilated cardiomyopathy 1DD"
gtctcgtagtccggtgagccggtca

SEQ ID NO: 390 - DNA, 20 bp, Homo sapiens
  source: /note="target seq for Renal carnitine transport defect"
gtggccatggaatagcgccg

SEQ ID NO: 391 - DNA, 25 bp, Homo sapiens
  source: /note="target seq for Baraitser-Winter syndrome 1"
gatcctcaccgagcgcggctacagc

SEQ ID NO: 392 - DNA, 25 bp, Homo sapiens
  source: /note="target seq for Very long chain acyl-CoA dehydrogenase deficiency"
gggcatgcatgaccttggcgtgggc

SEQ ID NO: 393 - DNA, 20 bp, Homo sapiens
  source: /note="target seq for Familial hypercholesterolemia"
gtcagatttgtccttgcagt

SEQ ID NO: 394 - DNA, 20 bp, Homo sapiens
  source: /note="target seq for Limb-girdle muscular dystrophy, type 2A"
gtacggggttgctctgccgg

SEQ ID NO: 395 - DNA, 25 bp, Homo sapiens
  source: /note="target seq for Familial hypercholesterolemia"
gacagtagcccctgctcggccttcg

SEQ ID NO: 396 - DNA, 20 bp, Homo sapiens
  source: /note="target seq for Aortic aneurysm, familial thoracic 6"
gccccatgccatcatgcgtc

SEQ ID NO: 397 - DNA, 25 bp, Homo sapiens
  source: /note="target seq for Acromicric dysplasia"
gctttgtcatcgacatttataccgg

SEQ ID NO: 398 - DNA, 25 bp, Homo sapiens
  source: /note="target seq for Charcot-Marie-Tooth disease type 2C"
ggcggacatgcggcaccaggactcg

SEQ ID NO: 399 - DNA, 25 bp, Homo sapiens
  source: /note="target seq for Breast-ovarian cancer, familial 2"
gtgtaactgtatacgtatggcgttt

SEQ ID NO: 400 - DNA, 20 bp, Homo sapiens
  source: /note="target seq for Breast-ovarian cancer, familial 1"
gatgcctggacagaggacaa

SEQ ID NO: 401 - DNA, 25 bp, Homo sapiens
  source: /note="target seq for Charcot-Marie-Tooth disease type 2C"
gcctaactgatgaggagtttcgagg

SEQ ID NO: 402 - DNA, 25 bp, Homo sapiens
  source: /note="target seq for Charcot-Marie-Tooth disease type 2C"
gcctaactgatgaggagtttcaagg

SEQ ID NO: 403 - DNA, 20 bp, Homo sapiens
  source: /note="target seq for Hereditary cancer-predisposing syndrome"
gagcgctgctcagatagcga

SEQ ID NO: 404 - DNA, 25 bp, Homo sapiens
  source: /note="target seq for Early infantile epileptic encephalopathy"
gatgatccgcatggaccggcgggga

SEQ ID NO: 405 - DNA, 20 bp, Homo sapiens
  source: /note="target seq for Early infantile epileptic encephalopathy"
ggatgatccgcatggaccgg

SEQ ID NO: 406 - DNA, 25 bp, Homo sapiens
  source: /note="target seq for Early infantile epileptic encephalopathy"
gcggatgatccgcatggaccagcgg

SEQ ID NO: 407 - DNA, 20 bp, Homo sapiens
  source: /note="target seq for Acromicric dysplasia"
gtacgtgatccatcctaggt

SEQ ID NO: 408 - DNA, 25 bp, Homo sapiens
  source: /note="target seq for Hypertrophic cardiomyopathy"
gacaccacggtctccctcaagtggc

SEQ ID NO: 409 - DNA, 25 bp, Homo sapiens
  source: /note="target seq for Cardiovascular phenotype"
gctgtccggggtagccccaagatag

SEQ ID NO: 410 - DNA, 25 bp, Homo sapiens
  source: /note="target seq for Cardiovascular phenotype"
gtccacggtgagggggccctggtgt

SEQ ID NO: 411 - DNA, 25 bp, Homo sapiens
  source: /note="target seq for Cardiovascular phenotype"
gcctagactgcaggacacagggact

SEQ ID NO: 412 - DNA, 25 bp, Homo sapiens
  source: /note="target seq for Familial hypertrophic cardiomyopathy 1"
gcatctgcagacatagagacctgtg

SEQ ID NO: 413 - DNA, 20 bp, Homo sapiens
  source: /note="target seq for Benign scapuloperoneal muscular dystrophy with cardiomyopathy"
gccctccaagagcttgcggt

SEQ ID NO: 414 - DNA, 25 bp, Homo sapiens
  source: /note="target seq for Glycogen storage disease, type II"
ggccctcaccctgcgctacgcactc

SEQ ID NO: 415 - DNA, 25 bp, Homo sapiens
  source: /note="target seq for Diffuse mesangial sclerosis"
gtttaggcacttgttttacctgtat

SEQ ID NO: 416 - DNA, 20 bp, Homo sapiens
  source: /note="target seq for Colobomatous microphthalmia"
gggtcgaggcggacgccata

SEQ ID NO: 417 - DNA, 20 bp, Homo sapiens
  source: /note="target seq for Ataxia-telangiectasia syndrome"
gtaaatacatatttactact

SEQ ID NO: 418 - DNA, 20 bp, Homo sapiens
  source: /note="target seq for Familial cancer of breast"
ggctacagcacacagctcgt

SEQ ID NO: 419 - DNA, 25 bp, Homo sapiens
  source: /note="target seq for Limb-girdle muscular dystrophy, type 2A"
gctacgagatgcaaaatgcagtcaa

SEQ ID NO: 420 - DNA, 20 bp, Homo sapiens
  source: /note="target seq for Hereditary cancer-predisposing syndrome"
gccgcttaccaaaaggagta

SEQ ID NO: 421 - DNA, 25 bp, Homo sapiens
  source: /note="target seq for Asymmetric septal hypertrophy"
gtgctgcaggttgttggtgcatggc

SEQ ID NO: 422 - DNA, 20 bp, Homo sapiens
  source: /note="target seq for Hereditary cancer-predisposing syndrome"
gtaattctataactccttag

SEQ ID NO: 423 - DNA, 25 bp, Homo sapiens
  source: /note="target seq for Familial hypertrophic cardiomyopathy 2"
gctaaagtcaccgggcgctggaaat

SEQ ID NO: 424 - DNA, 25 bp, Homo sapiens
  source: /note="target seq for Familial hypertrophic cardiomyopathy 2"
ggctaaagtcaccgggcgctagaaa

SEQ ID NO: 425 - DNA, 25 bp, Homo sapiens
  source: /note="target seq for Familial hypertrophic cardiomyopathy 2"
gctaaagtcaccgggcgctagaaat

SEQ ID NO: 426 - DNA, 25 bp, Homo sapiens
  source: /note="target seq for Erythrocytosis, familial, 2"
gaaagagcaatgcctccaggttgtc

SEQ ID NO: 427 - DNA, 25 bp, Homo sapiens
  source: /note="target seq for Death in infancy"
gtattggaatccggagcatccacgt

SEQ ID NO: 428 - DNA, 20 bp, Homo sapiens
  source: /note="target seq for Muscular Diseases"
gcatcttccggatctttgag

SEQ ID NO: 429 - DNA, 25 bp, Homo sapiens
  source: /note="target seq for Familial hypercholesterolemia"
gctgcgagcatggggccctgaggct

SEQ ID NO: 430 - DNA, 20 bp, Homo sapiens
  source: /note="target seq for Familial cancer of breast"
ggcagcgttacccagtccga

SEQ ID NO: 431 - DNA, 25 bp, Homo sapiens
  source: /note="target seq for Hereditary cancer-predisposing syndrome"
gtgtaggcaacttctatagccacag

SEQ ID NO: 432 - DNA, 25 bp, Homo sapiens
  source: /note="target seq for Familial hypercholesterolemia"
ggaactcccgccaagatcaagaaag

SEQ ID NO: 433 - DNA, 25 bp, Homo sapiens
  source: /note="target seq for Familial hypercholesterolemia"
gcggctgccagtatctgtgcctccc

SEQ ID NO: 434 - DNA, 25 bp, Homo sapiens
  source: /note="target seq for Familial hypercholesterolemia"
gaatgatctgcaggtgagcgtcgcc

SEQ ID NO: 435 - DNA, 25 bp, Homo sapiens
  source: /note="target seq for Inclusion body myopathy 2"
gtgctgtagtgcaccaatgtaatct

SEQ ID NO: 436 - DNA, 20 bp, Homo sapiens
  source: /note="target seq for Ataxia-telangiectasia syndrome"
gctttgatgttaacaatcgc

SEQ ID NO: 437 - DNA, 25 bp, Homo sapiens
  source: /note="target seq for Benign familial neonatal-infantile seizures"
gtcagttctccgatcattccagctg

SEQ ID NO: 438 - DNA, 20 bp, Homo sapiens
  source: /note="target seq for Marfan Syndrome/Loeys-Dietz Syndrome/Familial Thoracic Aortic Aneurysms and Dissections"
gtatctccattgtctcctcg

SEQ ID NO: 439 - DNA, 25 bp, Homo sapiens
  source: /note="target seq for Dilated cardiomyopathy 1G"
gtttcagattcccctggcccacgtg

SEQ ID NO: 440 - DNA, 20 bp, Homo sapiens
  source: /note="target seq for Familial hypercholesterolemia"
gcggtgagtctcggtgcagg

SEQ ID NO: 441 - DNA, 20 bp, Homo sapiens
  source: /note="target seq for Breast-ovarian cancer, familial 2"
gatacagtattaattgactg

SEQ ID NO: 442 - DNA, 20 bp, Homo sapiens
  source: /note="target seq for Familial hypercholesterolemia"
gcgagtgcatccactccagc

SEQ ID NO: 443 - DNA, 25 bp, Homo sapiens
  source: /note="target seq for Familial hypercholesterolemia"
ggctacaagtgccagtgtgaggaag

SEQ ID NO: 444 - DNA, 25 bp, Homo sapiens
  source: /note="target seq for Familial hypercholesterolemia"
gggtggctacaagtgccagcgtgag

SEQ ID NO: 445 - DNA, 25 bp, Homo sapiens
  source: /note="target seq for Familial hypercholesterolemia"
gtacaccagcctcacccccaacctg

SEQ ID NO: 446 - DNA, 25 bp, Homo sapiens
  source: /note="target seq for Familial cancer of breast"
gcctgcccgatagacgagcctcccg

SEQ ID NO: 447 - DNA, 20 bp, Homo sapiens
  source: /note="target seq for Hereditary hemorrhagic telangiectasia type 2"
gatccgcagcgcggtgagtc

SEQ ID NO: 448 - DNA, 3 bp, Streptococcus pyogenes
  source: /note="SpyCas9 PAM"
  modified_base (1)..(1): a, c, t, g, unknown or other
ngg

SEQ ID NO: 449 - DNA, 5 bp, Staphylococcus aureus
  source: /note="SauCas9"
  modified_base (1)..(1): a, c, t, g, unknown or other
ngrrt

SEQ ID NO: 450 - protein, 415 aa, Artificial Sequence
  source: /note="Description of Artificial Sequence: Synthetic polypeptide"
  source: /note="ADAT"
MAKRPAATKKAGQAKKKKSEVEFSHEYWMRHALTLAKRAWDEREVPVGAVLVHNNRVIGEGWNRPIGRHDPTAHAEIMALRQGGLVMQNYRLIDATLYVTLEPCVMCAGAMIHSRIGRVVFGARDAKTGAAGSLMDVLHHPGMNHRVEITEGILADECAALLSDFFRMRRQEIKAQKKAQSSTDSGGSSGGSSGSETPGTSESATPESSGGSSGGSSEVEFSHEYWMRHALTLAKRARDEREVPVGAVLVLNNRVIGEGWNRAIGLHDPTAHAEIMALRQGGLVMQNYRLIDATLYVTFEPCVMCAGAMIHSRIGRVVFGVRNAKTGAAGSLMDVLHYPGMNHRVEITEGILADECAALLCYFFRMPRQVFNAQKKAQSSTDSGGSSGGSSGSETPGTSESATPESSGGSSGGSS

SEQ ID NO: 451 - protein, 1494 aa, Artificial Sequence
  source: /note="Description of Artificial Sequence: Synthetic polypeptide"
  source: /note="Nuc-ADAT-Linker-dAPG08290.1-Linker-SV40"
MAKRPAATKKAGQAKKKKSEVEFSHEYWMRHALTLAKRAWDEREVPVGAVLVHNNRVIGEGWNRPIGRHDPTAHAEIMALRQGGLVMQNYRLIDATLYVTLEPCVMCAGAMIHSRIGRVVFGARDAKTGAAGSLMDVLHHPGMNHRVEITEGILADECAALLSDFFRMRRQEIKAQKKAQSSTDSGGSSGGSSGSETPGTSESATPESSGGSSGGSSEVEFSHEYWMRHALTLAKRARDEREVPVGAVLVLNNRVIGEGWNRAIGLHDPTAHAEIMALRQGGLVMQNYRLIDATLYVTFEPCVMCAGAMIHSRIGRVVFGVRNAKTGAAGSLMDVLHYPGMNHRVEITEGILADECAALLCYFFRMPRQVFNAQKKAQSSTDSGGSSGGSSGSETPGTSESATPESSGGSSGGSSMSELDYRIGLAIGTNSIGWGVIELFWNKDRERYEKVRIVDKGVRMFDKAEIPNKGASLAEPRRIARSSRRRLNRKSQRKKEIRNLLVQHGMITQEELDLLYPLSKKSIDIWDIRLDGLDRLLNHLEWARLLIHLAQRRGFKSNRKSELKDAETGKVLSSIQVNEKRLFLYRTVGEMWIKDAEFSKYDRRRNSPNEYVFSVSRADLEKEIVTLFEAQRKFQSSYASKNLQETYLQIWAHQLPFASGNAILNKVGYCSLLKGKERRIPKATYTFQYFSALDQVNRTRLGPDFQPFTQEQKEIILDKMFQRTDYYKKKTIPEVSYYDIRKWLELDETIQFKGLNYDPNEELKKIEKKPFINLKAFYEIKKVVANYAERTNEAFSTLDYDAIAYALTVYKTDKDIRSYLKKSNNLSKRCYDDQLIEELFTLSYTKFGHLSFKAINHVLPIMQEGRTYQEAIHQLGYDTTNLKKENRSMFLPLIPDEITNPIVKRAITQARKVVNAIIRRYGSPNSVHIALARELSKSHDERKKIMTAHDENYKKNKGAISILIENGILNPTGYDIVRYKLWKEQGERCAYSLKEIPPDTFFNELKKERNGSPILEVDHILPYSQSFIDSYHNKVLVYSDENRNKGNRIPYTYFLETNKDWEAFERYVRSNKLFSKKKREYLLKKTYLPRESELIKERHLNDTRYASTFLKNFIEQNLQFKEVEVNLRKKRVQTVNGVITAHLRKRWGLEKNRQETYLHHAMDAIIVACTDHHMVTRITEYYQIKESNKSVKKPYFPMPWEGFRDELLSHLASQPIAKKISEELKAGYQSSDYIFVSRMPKRSVTGAAHDQTIRRKGGIDKKGKTIIIKRVRLKDIKFDENGDFKMVGKEQDLATYEAIKQRYLEHRKNSKKAFETPLYKPSKKGTGNLIKRVKIEGQTKAFVREVNGGVAQNSDLVRVDLFEKDDKYYMVPIYVPDTVCSELPKKVVKSGKGYEQWLTLDNSFTFKSSLYPYDLVRLVKGNEDRFLYFGTLDIDSDRLNFKDVNKPSKQNEYRYSLKTIENLEKYEVGVLGDLRLVKQETRRIFNRPKKKRKV

SEQ ID NO: 452 - protein, 1494 aa, Artificial Sequence
  source: /note="Description of Artificial Sequence: Synthetic polypeptide"
  source: /note="Nuc-ADAT-Linker-nAPG08290.1-Linker-SV40"
MAKRPAATKKAGQAKKKKSEVEFSHEYWMRHALTLAKRAWDEREVPVGAVLVHNNRVIGEGWNRPIGRHDPTAHAEIMALRQGGLVMQNYRLIDATLYVTLEPCVMCAGAMIHSRIGRVVFGARDAKTGAAGSLMDVLHHPGMNHRVEITEGILADECAALLSDFFRMRRQEIKAQKKAQSSTDSGGSSGGSSGSETPGTSESATPESSGGSSGGSSEVEFSHEYWMRHALTLAKRARDEREVPVGAVLVLNNRVIGEGWNRAIGLHDPTAHAEIMALRQGGLVMQNYRLIDATLYVTFEPCVMCAGAMIHSRIGRVVFGVRNAKTGAAGSLMDVLHYPGMNHRVEITEGILADECAALLCYFFRMPRQVFNAQKKAQSSTDSGGSSGGSSGSETPGTSESATPESSGGSSGGSSMSELDYRIGLAIGTNSIGWGVIELFWNKDRERYEKVRIVDKGVRMFDKAEIPNKGASLAEPRRIARSSRRRLNRKSQRKKEIRNLLVQHGMITQEELDLLYPLSKKSIDIWDIRLDGLDRLLNHLEWARLLIHLAQRRGFKSNRKSELKDAETGKVLSSIQVNEKRLFLYRTVGEMWIKDAEFSKYDRRRNSPNEYVFSVSRADLEKEIVTLFEAQRKFQSSYASKNLQETYLQIWAHQLPFASGNAILNKVGYCSLLKGKERRIPKATYTFQYFSALDQVNRTRLGPDFQPFTQEQKEIILDKMFQRTDYYKKKTIPEVSYYDIRKWLELDETIQFKGLNYDPNEELKKIEKKPFINLKAFYEIKKVVANYAERTNEAFSTLDYDAIAYALTVYKTDKDIRSYLKKSNNLSKRCYDDQLIEELFTLSYTKFGHLSFKAINHVLPIMQEGRTYQEAIHQLGYDTTNLKKENRSMFLPLIPDEITNPIVKRAITQARKVVNAIIRRYGSPNSVHIELARELSKSHDERKKIMTAHDENYKKNKGAISILIENGILNPTGYDIVRYKLWKEQGERCAYSLKEIPPDTFFNELKKERNGSPILEVDHILPYSQSFIDSYHNKVLVYSDENRNKGNRIPYTYFLETNKDWEAFERYVRSNKLFSKKKREYLLKKTYLPRESELIKERHLNDTRYASTFLKNFIEQNLQFKEVEVNLRKKRVQTVNGVITAHLRKRWGLEKNRQETYLHHAMDAIIVACTDHHMVTRITEYYQIKESNKSVKKPYFPMPWEGFRDELLSHLASQPIAKKISEELKAGYQSSDYIFVSRMPKRSVTGAAHDQTIRRKGGIDKKGKTIIIKRVRLKDIKFDENGDFKMVGKEQDLATYEAIKQRYLEHRKNSKKAFETPLYKPSKKGTGNLIKRVKIEGQTKAFVREVNGGVAQNSDLVRVDLFEKDDKYYMVPIYVPDTVCSELPKKVVKSGKGYEQWLTLDNSFTFKSSLYPYDLVRLVKGNEDRFLYFGTLDIDSDRLNFKDVNKPSKQNEYRYSLKTIENLEKYEVGVLGDLRLVKQETRRIFNRPKKKRKV

SEQ ID NO: 453 - DNA, 25 bp, Homo sapiens
  source: /note="Hurler target 1"
ggagcagctctaggccgaagtgtcg

SEQ ID NO: 454 - DNA, 25 bp, Homo sapiens
  source: /note="Hurler target 2"
taggccgaagtgtcgcaggccggga

SEQ ID NO: 455 - DNA, 25 bp, Homo sapiens
  source: /note="Hurler target 3"
gctctaggccgaagtgtcgcaggcc

SEQ ID NO: 456 - DNA, 135 bp, Artificial Sequence
  source: /note="Description of Artificial Sequence: Synthetic polynucleotide"
  source: /note="sgRNA Hurler target 1"
ggagcagctctaggccgaagtgtcggtcatagttccatgaaagccaaaagtggctttgatgtttctatgataagggtttcggcccgtggcgtcggggatcgcctgcccattccgatgggcttctccccatttatt

SEQ ID NO: 457 - DNA, 135 bp, Artificial Sequence
  source: /note="Description of Artificial Sequence: Synthetic polynucleotide"
  source: /note="sgRNA Hurler target 2"
taggccgaagtgtcgcaggccgggagtcatagttccatgaaagccaaaagtggctttgatgtttctatgataagggtttcggcccgtggcgtcggggatcgcctgcccattccgatgggcttctccccatttatt

SEQ ID NO: 458 - DNA, 135 bp, Artificial Sequence
  source: /note="Description of Artificial Sequence: Synthetic polynucleotide"
  source: /note="sgRNA Hurler target 3"
ggcctgcgacacttcggcctagagcgtcatagttccatgaaagccaaaagtggctttgatgtttctatgataagggtttcggcccgtggcgtcggggatcgcctgcccattccgatgggcttctccccatttatt

SEQ ID NO: 459 - DNA, 15 bp, Artificial Sequence
  source: /note="Description of Artificial Sequence: Synthetic oligonucleotide"
  source: /note="Hurler Forward Amplification Primer"
gactccttcaccaag

SEQ ID NO: 460 - DNA, 14 bp, Artificial Sequence
  source: /note="Description of Artificial Sequence: Synthetic oligonucleotide"
  source: /note="Hurler Reverse Amplification Primer"
gtagatcagcaccg

SEQ ID NO: 461 - DNA, 14 bp, Artificial Sequence
  source: /note="Description of Artificial Sequence: Synthetic oligonucleotide"
  source: /note="Hurler Wild Type Probe"
ctctgggccgaagt

SEQ ID NO: 462 - DNA, 14 bp, Artificial Sequence
  source: /note="Description of Artificial Sequence: Synthetic oligonucleotide"
  source: /note="Hurler W402X Probe-beta"
ctctaggccgaagt

SEQ ID NO: 463 - DNA, 13 bp, Artificial Sequence
  source: /note="Description of Artificial Sequence: Synthetic oligonucleotide"
  source: /note="Hurler NGS forward"
acttcctccagcc

SEQ ID NO: 464 - DNA, 13 bp, Artificial Sequence
  source: /note="Description of Artificial Sequence: Synthetic oligonucleotide"
  source: /note="Hurler NGS Reverse"
gaaccccggctta

SEQ ID NO: 465 - DNA, 31 bp, Homo sapiens
  source: /note="Human W402X"
ggagcagctctaggccgaagtgtcgcaggcc

SEQ ID NO: 466 - DNA, 31 bp, Mus musculus
  source: /note="Mouse W392X"
agaacaactctaggcagaggtctcaaaggct

SEQ ID NO: 467 - DNA, 31 bp, Artificial Sequence; identical to SEQ ID NO: 465
  source: /note="Description of Artificial Sequence: Synthetic oligonucleotide"
  source: /note="humanized mouse"

SEQ ID NO: 468 - DNA, 25 bp, Homo sapiens
  source: /note="FRDA target 1"
atcacctgaggtccggagttcaaga

SEQ ID NO: 469 - DNA, 25 bp, Homo sapiens
  source: /note="FRDA target 2"
gtcttgaactccggacctcaggtga

SEQ ID NO: 470 - DNA, 25 bp, Homo sapiens
  source: /note="FRDA target 3"
tgaactccggacctcaggtgatcca

SEQ ID NO: 471 - DNA, 25 bp, Homo sapiens
  source: /note="FRDA target 4"
gaaaagttagccgggcgtggtgtcg

SEQ ID NO: 472 - DNA, 500 bp, Artificial Sequence
  source: /note="Description of Artificial Sequence: Synthetic polynucleotide"
  source: /note="BCL11A enhancer region"
aaaaatggacaattatgaggaggggagagtgcagacaggggaagcttcacctcctttacaattttgggagtccacacggcatggcatacaaattatttcattcccattgagaaataaaatccaattctccatcaccaagagagccttccgaaagaggcccccctgggcaaacggccaccgatggagaggtctgccagtcctcttctaccccacccacgcccccaccctaatcagaggccaaacccttcctggagcctgtgataaaagcaactgttagcttgcactagactagcttcaaagttgtattgaccctggtgtgttatgtctaagagtagatgccatatctcttttctggcctatgttattacctgtatggactttgcactggaatcagctatctgctcttacttatgcacacctggggcatagagccagccctgtatcgcttttcagccatctcactacagataactcccaagtcctgtctagctgccttcctt

SEQ ID NO: 473 - DNA, 26 bp, Homo sapiens
  source: /note="SCD target seq 1"
gcactagactagcttcaaagttgtag

SEQ ID NO: 474 - DNA, 26 bp, Homo sapiens
  source: /note="SCD target seq 2"
cctaatcagaggccaaacccttcctg

SEQ ID NO: 475 - DNA, 26 bp, Homo sapiens
  source: /note="SCD target seq 3"
caagctaacagttgcttttatcacag

SEQ ID NO: 476 - DNA, 26 bp, Homo sapiens
  source: /note="SCD target seq 4"
gcactagactagcttcaaagttgtag

SEQ ID NO: 477 - DNA, 26 bp, Homo sapiens
  source: /note="SCD target seq 5"
cctaatcagaggccaaacccttcctg

SEQ ID NO: 478 - DNA, 26 bp, Homo sapiens
  source: /note="SCD target seq 6"
caagctaacagttgcttttatcacag

SEQ ID NO: 479 - DNA, 22 bp, Artificial Sequence
  source: /note="Description of Artificial Sequence: Synthetic oligonucleotide"
  source: /note="RelA FWD"
cttagtttcaccgcaggttcta

SEQ ID NO: 480 - DNA, 22 bp, Artificial Sequence
  source: /note="Description of Artificial Sequence: Synthetic oligonucleotide"
  source: /note="RelA REV"
ctgtgcactcaacactgatcta

SEQ ID NO: 481 - DNA, 21 bp, Artificial Sequence
  source: /note="Description of Artificial Sequence: Synthetic oligonucleotide"
  source: /note="AurkB FWD"
cccagccctaggttgtttatt

SEQ ID NO: 482 - DNA, 23 bp, Artificial Sequence
  source: /note="Description of Artificial Sequence: Synthetic oligonucleotide"
  source: /note="AurkB REV"
ctggctacatcttccttgactac

SEQ ID NO: 483 - DNA, 20 bp, Artificial Sequence
  source: /note="Description of Artificial Sequence: Synthetic oligonucleotide"
  source: /note="HPRT1 FWD"
gtggcagaagcagtgagtaa

SEQ ID NO: 484 - DNA, 22 bp, Artificial Sequence
  source: /note="Description of Artificial Sequence: Synthetic oligonucleotide"
  source: /note="HPRT1 REV"
tcccatctaggcactaggtaaa

SEQ ID NO: 485 - DNA, 54 bp, Artificial Sequence
  source: /note="Description of Artificial Sequence: Synthetic oligonucleotide"
  source: /note="FWD_Guide 134, Guide 135, Guide 136, Guide 137"
gtctcgtgggctcggagatgtgtataagagacagacaattctcctgcctcagcc

SEQ ID NO: 486 - DNA, 53 bp, Artificial Sequence
  source: /note="Description of Artificial Sequence: Synthetic oligonucleotide"
  source: /note="REV_Guide 134, Guide 135, Guide 136, Guide 137"
tcgtcggcagcgtcagatgtgtataagagacagactgccatgggaagaaggtg

SEQ ID NO: 487 - DNA, 54 bp, Artificial Sequence; identical to SEQ ID NO: 485
  source: /note="Description of Artificial Sequence: Synthetic oligonucleotide"
  source: /note="FWD_Guide 138, Guide 139, Guide 140, Guide 141"

SEQ ID NO: 488 - DNA, 53 bp, Artificial Sequence; identical to SEQ ID NO: 486
  source: /note="Description of Artificial Sequence: Synthetic oligonucleotide"
  source: /note="REV_Guide 138, Guide 139, Guide 140, Guide 141"

SEQ ID NO: 489 - DNA, 53 bp, Artificial Sequence
  source: /note="Description of Artificial Sequence: Synthetic oligonucleotide"
  source: /note="REV_Guide 142, Guide 143, Guide 144, Guide 145"
tcgtcggcagcgtcagatgtgtataagagacaggagctgcacatttgacgagc

SEQ ID NO: 490 - DNA, 54 bp, Artificial Sequence
  source: /note="Description of Artificial Sequence: Synthetic oligonucleotide"
  source: /note="FWD_Guide 142, Guide 143, Guide 144, Guide 145"
gtctcgtgggctcggagatgtgtataagagacagattacaggtgtgagccacgg

SEQ ID NO: 491 - DNA, 53 bp, Artificial Sequence
  source: /note="Description of Artificial Sequence: Synthetic oligonucleotide"
  source: /note="REV_Guide 164, Guide 165, Guide 166, Guide 167"
tcgtcggcagcgtcagatgtgtataagagacagctgacctcaggtgatacgcc

SEQ ID NO: 492 - DNA, 54 bp, Artificial Sequence
  source: /note="Description of Artificial Sequence: Synthetic oligonucleotide"
  source: /note="FWD_Guide 164, Guide 165, Guide 166, Guide 167"
gtctcgtgggctcggagatgtgtataagagacagctttgggaggctgagacagg

SEQ ID NO: 493 - DNA, 53 bp, Artificial Sequence
  source: /note="Description of Artificial Sequence: Synthetic oligonucleotide"
  source: /note="REV_Guide 168, Guide 169, Guide 170, Guide 171"
tcgtcggcagcgtcagatgtgtataagagacagtgctctattgtccaggctgg

SEQ ID NO: 494 - DNA, 54 bp, Artificial Sequence
  source: /note="Description of Artificial Sequence: Synthetic oligonucleotide"
  source: /note="FWD_Guide 168, Guide 169, Guide 170, Guide 171"
gtctcgtgggctcggagatgtgtataagagacagtccagcaggtcagcaaagaa

SEQ ID NO: 495 - DNA, 53 bp, Artificial Sequence
  source: /note="Description of Artificial Sequence: Synthetic oligonucleotide"
  source: /note="REV_Guide 172, Guide 173, Guide 174, Guide 175"
tcgtcggcagcgtcagatgtgtataagagacaggcagtataactggccagcct

SEQ ID NO: 496 - DNA, 56 bp, Artificial Sequence
  source: /note="Description of Artificial Sequence: Synthetic oligonucleotide"
  source: /note="FWD_Guide 172, Guide 173, Guide 174, Guide 175"
gtctcgtgggctcggagatgtgtataagagacagtcagttgaggagttcagcttaa

SEQ ID NO: 497 - DNA, 53 bp, Artificial Sequence
  source: /note="Description of Artificial Sequence: Synthetic oligonucleotide"
  source: /note="REV_Guide 185, Guide 186, Guide 187, Guide 188"
tcgtcggcagcgtcagatgtgtataagagacagtggcccctatgtggagatca

SEQ ID NO: 498 - DNA, 54 bp, Artificial Sequence
  source: /note="Description of Artificial Sequence: Synthetic oligonucleotide"
  source: /note="FWD_Guide 185, Guide 186, Guide 187, Guide 188"
gtctcgtgggctcggagatgtgtataagagacagggcagagctcagcctcatag

SEQ ID NO: 499 - DNA, 53 bp, Artificial Sequence
  source: /note="Description of Artificial Sequence: Synthetic oligonucleotide"
  source: /note="REV_Guide 189, Guide 190, Guide 191, Guide 192"
tcgtcggcagcgtcagatgtgtataagagacagatatccccacttcccctgct

SEQ ID NO: 500 - DNA, 54 bp, Artificial Sequence
  source: /note="Description of Artificial Sequence: Synthetic oligonucleotide"
  source: /note="FWD_Guide 189, Guide 190, Guide 191, Guide 192"
gtctcgtgggctcggagatgtgtataagagacagcacctcaaggacagctctgg

SEQ ID NO: 501 - DNA, 53 bp, Artificial Sequence; identical to SEQ ID NO: 499
  source: /note="Description of Artificial Sequence: Synthetic oligonucleotide"
  source: /note="REV_Guide 193, Guide 194, Guide 195, Guide 196"

SEQ ID NO: 502 - DNA, 54 bp, Artificial Sequence; identical to SEQ ID NO: 500
  source: /note="Description of Artificial Sequence: Synthetic oligonucleotide"
  source: /note="FWD_Guide 193, Guide 194, Guide 195, Guide 196"

SEQ ID NO: 503 - DNA, 54 bp, Artificial Sequence; identical to SEQ ID NO: 485
  source: /note="Description of Artificial Sequence: Synthetic oligonucleotide"
  source: /note="FWD_Guide 146"

SEQ ID NO: 504 - DNA, 53 bp, Artificial Sequence; identical to SEQ ID NO: 486
  source: /note="Description of Artificial Sequence: Synthetic oligonucleotide"
  source: /note="REV_Guide 146"

SEQ ID NO: 505 - DNA, 54 bp, Artificial Sequence; identical to SEQ ID NO: 485
  source: /note="Description of Artificial Sequence: Synthetic oligonucleotide"
  source: /note="FWD_Guide 147"

SEQ ID NO: 506 - DNA, 53 bp, Artificial Sequence; identical to SEQ ID NO: 486
  source: /note="Description of Artificial Sequence: Synthetic oligonucleotide"
  source: /note="REV_Guide 147"

SEQ ID NO: 507 - DNA, 53 bp, Artificial Sequence; identical to SEQ ID NO: 486
  source: /note="Description of Artificial Sequence: Synthetic oligonucleotide"
  source: /note="REV_Guide 148"

SEQ ID NO: 508 - DNA, 54 bp, Artificial Sequence; identical to SEQ ID NO: 485
  source: /note="Description of Artificial Sequence: Synthetic oligonucleotide"
  source: /note="FWD_Guide 148"

SEQ ID NO: 509 - DNA, 53 bp, Artificial Sequence
  source: /note="Description of Artificial Sequence: Synthetic oligonucleotide"
  source: /note="REV_Guide 176"
tcgtcggcagcgtcagatgtgtataagagacaggtagctcactgcagcctcaa

SEQ ID NO: 510 - DNA, 54 bp, Artificial Sequence
  source: /note="Description of Artificial Sequence: Synthetic oligonucleotide"
  source: /note="FWD_Guide 176"
gtctcgtgggctcggagatgtgtataagagacagtgggtgatgaacatacgggt

SEQ ID NO: 511 - DNA, 57 bp, Artificial Sequence
  source: /note="Description of Artificial Sequence: Synthetic oligonucleotide"
  source: /note="REV_Guide 177"
tcgtcggcagcgtcagatgtgtataagagacagtcagactgaagagctattgtgtga

SEQ ID NO: 512 - DNA, 54 bp, Artificial Sequence
  source: /note="Description of Artificial Sequence: Synthetic oligonucleotide"
  source: /note="FWD_Guide 177"
gtctcgtgggctcggagatgtgtataagagacagccccacaaaccgatgtagct

SEQ ID NO: 513 - DNA, 53 bp, Artificial Sequence
  source: /note="Description of Artificial Sequence: Synthetic oligonucleotide"
  source: /note="REV_Guide 209"
tcgtcggcagcgtcagatgtgtataagagacagtggagtgcagtggtgtgatc

SEQ ID NO: 514 - DNA, 54 bp, Artificial Sequence
  source: /note="Description of Artificial Sequence: Synthetic oligonucleotide"
  source: /note="FWD_Guide 209"
gtctcgtgggctcggagatgtgtataagagacagttgaggctgcagtgagctac

SEQ ID NO: 515 - DNA, 53 bp, Artificial Sequence; identical to SEQ ID NO: 497
  source: /note="Description of Artificial Sequence: Synthetic oligonucleotide"
  source: /note="REV_Guide 197"

SEQ ID NO: 516 - DNA, 54 bp, Artificial Sequence; identical to SEQ ID NO: 498
  source: /note="Description of Artificial Sequence: Synthetic oligonucleotide"
  source: /note="FWD_Guide 197"

SEQ ID NO: 517 - DNA, 53 bp, Artificial Sequence
  source: /note="Description of Artificial Sequence: Synthetic oligonucleotide"
  source: /note="REV_Guide 198"
tcgtcggcagcgtcagatgtgtataagagacagccaagccgaccaaacaagtg

SEQ ID NO: 518 - DNA, 54 bp, Artificial Sequence
  source: /note="Description of Artificial Sequence: Synthetic oligonucleotide"
  source: /note="FWD_Guide 198"
gtctcgtgggctcggagatgtgtataagagacaggatgcgctgactgatagcct

SEQ ID NO: 519 - DNA, 53 bp, Artificial Sequence; identical to SEQ ID NO: 497
  source: /note="Description of Artificial Sequence: Synthetic oligonucleotide"
  source: /note="REV_Guide 199"

SEQ ID NO: 520 - DNA, 54 bp, Artificial Sequence; identical to SEQ ID NO: 498
  source: /note="Description of Artificial Sequence: Synthetic oligonucleotide"
  source: /note="FWD_Guide 199"

SEQ ID NO: 521 - DNA, 54 bp, Artificial Sequence
  source: /note="Description of Artificial Sequence: Synthetic oligonucleotide"
  source: /note="FWD_Guide 149"
gtctcgtgggctcggagatgtgtataagagacagggtaaggggaaactggaggc

SEQ ID NO: 522 - DNA, 53 bp, Artificial Sequence
  source: /note="Description of Artificial Sequence: Synthetic oligonucleotide"
  source: /note="REV_Guide 149"
tcgtcggcagcgtcagatgtgtataagagacagtccactttctaagcaggcgg

SEQ ID NO: 523 - DNA, 54 bp, Artificial Sequence
  source: /note="Description of Artificial Sequence: Synthetic oligonucleotide"
  source: /note="FWD_Guide 150"
gtctcgtgggctcggagatgtgtataagagacaggtgggcctggatttcgatct

SEQ ID NO: 524 - DNA, 53 bp, Artificial Sequence
  source: /note="Description of Artificial Sequence: Synthetic oligonucleotide"
  source: /note="REV_Guide 150"
tcgtcggcagcgtcagatgtgtataagagacagatgaacaggcaggaagtcgg

SEQ ID NO: 525 - DNA, 53 bp, Artificial Sequence
  source: /note="Description of Artificial Sequence: Synthetic oligonucleotide"
  source: /note="REV_Guide 151"
tcgtcggcagcgtcagatgtgtataagagacagcggttctgagttgccttcct

SEQ ID NO: 526 - DNA, 54 bp, Artificial Sequence; identical to SEQ ID NO: 521
  source: /note="Description of Artificial Sequence: Synthetic oligonucleotide"
  source: /note="FWD_Guide 151"

SEQ ID NO: 527 - DNA, 53 bp, Artificial Sequence
  source: /note="Description of Artificial Sequence: Synthetic oligonucleotide"
  source: /note="REV_Guide 179"
tcgtcggcagcgtcagatgtgtataagagacagtcagtggtccacatgcaagt

SEQ ID NO: 528 - DNA, 54 bp, Artificial Sequence
  source: /note="Description of Artificial Sequence: Synthetic oligonucleotide"
  source: /note="FWD_Guide 179"
gtctcgtgggctcggagatgtgtataagagacagaaggcaagttgatcgctcga

SEQ ID NO: 529 - DNA, 53 bp, Artificial Sequence
  source: /note="Description of Artificial Sequence: Synthetic oligonucleotide"
  source: /note="REV_Guide 180"
tcgtcggcagcgtcagatgtgtataagagacagagtggttctgttgcacacgt

SEQ ID NO: 530 - DNA, 54 bp, Artificial Sequence
  source: /note="Description of Artificial Sequence: Synthetic oligonucleotide"
  source: /note="FWD_Guide 180"
gtctcgtgggctcggagatgtgtataagagacagtcgcttaagcccaggagttc

SEQ ID NO: 531 - DNA, 55 bp, Artificial Sequence
  source: /note="Description of Artificial Sequence: Synthetic oligonucleotide"
  source: /note="REV_Guide 181"
tcgtcggcagcgtcagatgtgtataagagacagtctggctgatccgtactaatcc

SEQ ID NO: 532 - DNA, 54 bp, Artificial Sequence
  source: /note="Description of Artificial Sequence: Synthetic oligonucleotide"
  source: /note="FWD_Guide 181"
gtctcgtgggctcggagatgtgtataagagacagtaggctcaagggatgctcct

SEQ ID NO: 533 - DNA, 53 bp, Artificial Sequence
  source: /note="Description of Artificial Sequence: Synthetic oligonucleotide"
  source: /note="REV_Guide 200"
tcgtcggcagcgtcagatgtgtataagagacagccagagctgtccttgaggtg

SEQ ID NO: 534 - DNA, 54 bp, Artificial Sequence
  source: /note="Description of Artificial Sequence: Synthetic oligonucleotide"
  source: /note="FWD_Guide 200"
gtctcgtgggctcggagatgtgtataagagacaggtccatacccaccttggcaa

SEQ ID NO: 535 - DNA, 53 bp, Artificial Sequence; identical to SEQ ID NO: 517
  source: /note="Description of Artificial Sequence: Synthetic oligonucleotide"
  source: /note="REV_Guide 201"

SEQ ID NO: 536 - DNA, 54 bp, Artificial Sequence; identical to SEQ ID NO: 518
  source: /note="Description of Artificial Sequence: Synthetic oligonucleotide"
  source: /note="FWD_Guide 201"

SEQ ID NO: 537 - DNA, 53 bp, Artificial Sequence
  source: /note="Description of Artificial Sequence: Synthetic oligonucleotide"
  source: /note="REV_Guide 202"
tcgtcggcagcgtcagatgtgtataagagacagaggctatcagtcagcgcatc

SEQ ID NO: 538 - DNA, 54 bp, Artificial Sequence
  source: /note="Description of Artificial Sequence: Synthetic oligonucleotide"
  source: /note="FWD_Guide 202"
gtctcgtgggctcggagatgtgtataagagacagagcaggggaagtggggatat

SEQ ID NO: 539 - DNA, 54 bp, Artificial Sequence; identical to SEQ ID NO: 490
  source: /note="Description of Artificial Sequence: Synthetic oligonucleotide"
  source: /note="FWD_Guide 152"

SEQ ID NO: 540 - DNA, 53 bp, Artificial Sequence; identical to SEQ ID NO: 489
  source: /note="Description of Artificial Sequence: Synthetic oligonucleotide"
  source: /note="REV_Guide 152"

SEQ ID NO: 541 - DNA, 54 bp, Artificial Sequence; identical to SEQ ID NO: 485
  source: /note="Description of Artificial Sequence: Synthetic oligonucleotide"
  source: /note="FWD_Guide 153"

SEQ ID NO: 542 - DNA, 53 bp, Artificial Sequence; identical to SEQ ID NO: 486
  source: /note="Description of Artificial Sequence: Synthetic oligonucleotide"
  source: /note="REV_Guide 153"

SEQ ID NO: 543 - DNA, 54 bp, Artificial Sequence; identical to SEQ ID NO: 490
  source: /note="Description of Artificial Sequence: Synthetic oligonucleotide"
  source: /note="FWD_Guide 154"

SEQ ID NO: 544 - DNA, 53 bp, Artificial Sequence; identical to SEQ ID NO: 489
  source: /note="Description of Artificial Sequence: Synthetic oligonucleotide"
  source: /note="REV_Guide 154"

SEQ ID NO: 545 - DNA, 54 bp, Artificial Sequence; identical to SEQ ID NO: 510
  source: /note="Description of Artificial Sequence: Synthetic oligonucleotide"
  source: /note="FWD_Guide 182"

SEQ ID NO: 546 - DNA, 53 bp, Artificial Sequence; identical to SEQ ID NO: 509
  source: /note="Description of Artificial Sequence: Synthetic oligonucleotide"
  source: /note="REV_Guide 182"

SEQ ID NO: 547 - DNA, 54 bp, Artificial Sequence
  source: /note="Description of Artificial Sequence: Synthetic oligonucleotide"
  source: /note="FWD_Guide 183"
gtctcgtgggctcggagatgtgtataagagacagtgcctgtagtcccagctact

SEQ ID NO: 548 - DNA, 53 bp, Artificial Sequence
  source: /note="Description of Artificial Sequence: Synthetic oligonucleotide"
  source: /note="REV_Guide 183"
tcgtcggcagcgtcagatgtgtataagagacagtcagctcagtgcaacctctg

SEQ ID NO: 549 - DNA, 54 bp, Artificial Sequence; identical to SEQ ID NO: 492
  source: /note="Description of Artificial Sequence: Synthetic oligonucleotide"
  source: /note="FWD_Guide 184"

SEQ ID NO: 550 - DNA, 53 bp, Artificial Sequence; identical to SEQ ID NO: 491
  source: /note="Description of Artificial Sequence: Synthetic oligonucleotide"
  source: /note="REV_Guide 184"

SEQ ID NO: 551 - DNA, 54 bp, Artificial Sequence; identical to SEQ ID NO: 518
  source: /note="Description of Artificial Sequence: Synthetic oligonucleotide"
  source: /note="FWD_Guide 203"

SEQ ID NO: 552 - DNA, 53 bp, Artificial Sequence; identical to SEQ ID NO: 517
  source: /note="Description of Artificial Sequence: Synthetic oligonucleotide"
  source: /note="REV_Guide 203"

SEQ ID NO: 553 - DNA, 54 bp, Artificial Sequence; identical to SEQ ID NO: 500
  source: /note="Description of Artificial Sequence: Synthetic oligonucleotide"
  source: /note="FWD_Guide 204"

SEQ ID NO: 554 - DNA, 53 bp, Artificial Sequence; identical to SEQ ID NO: 499
  source: /note="Description of Artificial Sequence: Synthetic oligonucleotide"
  source: /note="REV_Guide 204"

SEQ ID NO: 555 - DNA, 54 bp, Artificial Sequence; identical to SEQ ID NO: 498
  source: /note="Description of Artificial Sequence: Synthetic oligonucleotide"
  source: /note="FWD_Guide 205"

SEQ ID NO: 556 - DNA, 53 bp, Artificial Sequence; identical to SEQ ID NO: 497
  source: /note="Description of Artificial Sequence: Synthetic oligonucleotide"
  source: /note="REV_Guide 205"

SEQ ID NO: 557 - RNA, 6 nt, Artificial Sequence
  source: /note="Description of Artificial Sequence: Synthetic oligonucleotide"
  source: /note="seq in base of hairpin stem of tracrRNA"
  modified_base (2)..(2): a, c, u, g, unknown or other
  modified_base (4)..(5): a, c, u, g, unknown or other
unannu

SEQ ID NO: 558 - RNA, 6 nt, Artificial Sequence
  source: /note="Description of Artificial Sequence: Synthetic oligonucleotide"
  source: /note="seq in base of hairpin stem of tracrRNA"
  modified_base (2)..(2): a, c, u, g, unknown or other
  modified_base (4)..(5): a, c, u, g, unknown or other
unanna

SEQ ID NO: 559 - DNA, 30 bp, Artificial Sequence
  source: /note="Description of Artificial Sequence: Synthetic oligonucleotide"
  source: /note="sequence 2 for cleavage site assay"
ccatgatatagacgttgtggctgttgtagt

SEQ ID NO: 560 - protein, 6 aa, Artificial Sequence
  source: /note="Description of Artificial Sequence: Synthetic 6xHis tag"
HHHHHH

SEQ ID NO: 561 - protein, 10 aa, Artificial Sequence
  source: /note="Description of Artificial Sequence: Synthetic 10xHis tag"
HHHHHHHHHH

SEQ ID NO: 562 - DNA, 34 bp, Artificial Sequence
  source: /note="Description of Artificial Sequence: Synthetic oligonucleotide"
cctgggtgtgaggctgggccattaaaacctctcc

SEQ ID NO: 563 - DNA, 15 bp, Artificial Sequence
  source: /note="Description of Artificial Sequence: Synthetic oligonucleotide"
cctgaaaacctctcc

SEQ ID NO: 564 - DNA, 33 bp, Artificial Sequence
  source: /note="Description of Artificial Sequence: Synthetic oligonucleotide"
cctgggtgtgagctgggccattaaaacctctcc

SEQ ID NO: 565 - DNA, 22 bp, Artificial Sequence
  source: /note="Description of Artificial Sequence: Synthetic oligonucleotide"
cctgggccattaaaacctctcc

SEQ ID NO: 566 - DNA, 11 bp, Artificial Sequence
  source: /note="Description of Artificial Sequence: Synthetic oligonucleotide"
cctggctctcc

SEQ ID NO: 567 - DNA, 20 bp, Artificial Sequence
  source: /note="Description of Artificial Sequence: Synthetic oligonucleotide"
cgggccattaaaacctctcc

SEQ ID NO: 568 - DNA, 40 bp, Artificial Sequence
  source: /note="Description of Artificial Sequence: Synthetic oligonucleotide"
cctgggtgtgaggccagacctgggccattaaaacctctcc

SEQ ID NO: 569 - DNA, 79 bp, Artificial Sequence
  source: /note="Description of Artificial Sequence: Synthetic oligonucleotide"
cctgggtgtgaggggaagctgacgtcctttccatggctgctcgcctgtgttgccaccgctgggccattaaaacctctcc

SEQ ID NO: 570 - DNA, 33 bp, Artificial Sequence
  source: /note="Description of Artificial Sequence: Synthetic oligonucleotide"
cctgggtgtgacctgggccattaaaacctctcc

SEQ ID NO: 571 - DNA, 35 bp, Artificial Sequence
  source: /note="Description of Artificial Sequence: Synthetic oligonucleotide"
cctgggtgtgaggactgggccattaaaacctctcc

SEQ ID NO: 572 - DNA, 34 bp, Artificial Sequence
  source: /note="Description of Artificial Sequence: Synthetic oligonucleotide"
agttggcagatgctctaatgtactgccatgggaa

SEQ ID NO: 573 - DNA, 31 bp, Artificial Sequence
  source: /note="Description of Artificial Sequence: Synthetic oligonucleotide"
agttggcagatgcaatgtactgccatgggaa

SEQ ID NO: 574 - DNA, 30 bp, Artificial Sequence
  source: /note="Description of Artificial Sequence: Synthetic oligonucleotide"
agttggcagatgcatgtactgccatgggaa

SEQ ID NO: 575 - DNA, 31 bp, Artificial Sequence
  source: /note="Description of Artificial Sequence: Synthetic oligonucleotide"
agttggcagatgctatgtactgccatgggaa

SEQ ID NO: 576 - DNA, 32 bp, Artificial Sequence
  source: /note="Description of Artificial Sequence: Synthetic oligonucleotide"
agttggcagatgctaatgtactgccatgggaa

SEQ ID NO: 577 - DNA, 31 bp, Artificial Sequence
  source: /note="Description of Artificial Sequence: Synthetic oligonucleotide"
agttggcagatgctatgtaatgccatgggaa

SEQ ID NO: 578 - DNA, 33 bp, Artificial Sequence
  source: /note="Description of Artificial Sequence: Synthetic oligonucleotide"
agttggcagatgctctatgtactgccatgggaa

SEQ ID NO: 579 - DNA, 39 bp, Artificial Sequence
  source: /note="Description of Artificial Sequence: Synthetic oligonucleotide"
cgacctgaatgctgtgcggcgctctggcttcattcaatc

SEQ ID NO: 580 - DNA, 35 bp, Artificial Sequence
  source: /note="Description of Artificial Sequence: Synthetic oligonucleotide"
cgacctgaatgctgtgcggctctgcttccaggtga

SEQ ID NO: 581 - DNA, 36 bp, Artificial Sequence
  source: /note="Description of Artificial Sequence: Synthetic oligonucleotide"
cgacctgaatgctgtgcggcatctgcttccaggtga

SEQ ID NO: 582 - DNA, 25 bp, Artificial Sequence
  source: /note="Description of Artificial Sequence: Synthetic oligonucleotide"
cgacctgaatgctgcttccaggtga

SEQ ID NO: 583 - DNA, 28 bp, Artificial Sequence
  source: /note="Description of Artificial Sequence: Synthetic oligonucleotide"
cgacctgaatgcttctgcttccaggtga

SEQ ID NO: 584 - DNA, 22 bp, Artificial Sequence
  source: /note="Description of Artificial Sequence: Synthetic oligonucleotide"
cgacctgaatgcttccaggtga

SEQ ID NO: 585 - DNA, 35 bp, Artificial Sequence
  source: /note="Description of Artificial Sequence: Synthetic oligonucleotide"
gcgtggggactacgacctgaatgctgtgcggctct

SEQ ID NO: 586 - DNA, 24 bp, Artificial Sequence
  source: /note="Description of Artificial Sequence: Synthetic oligonucleotide"
gcgacctgaatgctgtgcggctct

SEQ ID NO: 587 - DNA, 28 bp, Artificial Sequence
  source: /note="Description of Artificial Sequence: Synthetic oligonucleotide"
gcgtggggactacgagctgtgcggctct

SEQ ID NO: 588 - DNA, 28 bp, Artificial Sequence
  source: /note="Description of Artificial Sequence: Synthetic oligonucleotide"
gcgtggggactgaatgctgtgcggctct

SEQ ID NO: 589 - DNA, 31 bp, Artificial Sequence
  source: /note="Description of Artificial Sequence: Synthetic oligonucleotide"
gcgtggggactcctgaatgctgtgcggctct

SEQ ID NO: 590 - DNA, 36 bp, Artificial Sequence
  source: /note="Description of Artificial Sequence: Synthetic oligonucleotide"
gcgtggggactacgaacctgaatgctgtgcggctct

SEQ ID NO: 591 - DNA, 30 bp, Artificial Sequence
  source: /note="Description of Artificial Sequence: Synthetic oligonucleotide"
gcgtggggactacgaatgctgtgcggctct

SEQ ID NO: 592 - DNA, 32 bp, Artificial Sequence
  source: /note="Description of Artificial Sequence: Synthetic oligonucleotide"
gcgtggggactacctgaatgctgtgcggctct

SEQ ID NO: 593 - DNA, 21 bp, Artificial Sequence
  source: /note="Description of Artificial Sequence: Synthetic oligonucleotide"
gcgtgaatgctgtgcggctct

SEQ ID NO: 594 - DNA, 24 bp, Artificial Sequence
  source: /note="Description of Artificial Sequence: Synthetic oligonucleotide"
gcgacctgactgctgtgcggctct

SEQ ID NO: 595 - DNA, 34 bp, Artificial Sequence
  source: /note="Description of Artificial Sequence: Synthetic oligonucleotide"
gcgtggggactacgcctgaatgctgtgcggctct

SEQ ID NO: 596 - DNA, 42 bp, Artificial Sequence
  source: /note="Description of Artificial Sequence: Synthetic oligonucleotide"
atggaggagttggcagatgctctaatgtactgccatgggaag

SEQ ID NO: 597 - DNA, 40 bp, Artificial Sequence
  source: /note="Description of Artificial Sequence: Synthetic oligonucleotide"
atggaggagttggcagatgctaatgtactgccatgggaag

SEQ ID NO: 598 - DNA, 34 bp, Artificial Sequence
  source: /note="Description of Artificial Sequence: Synthetic oligonucleotide"
atggaggagttggcagatgtactgccatgggaag

SEQ ID NO: 599 - DNA, 18 bp, Artificial Sequence
  source: /note="Description of Artificial Sequence: Synthetic oligonucleotide"
atgtactgccatgggaag

SEQ ID NO: 600 - DNA, 30 bp, Artificial Sequence
  source: /note="Description of Artificial Sequence: Synthetic oligonucleotide"
atggaggagttggtgtactgccatgggaag

SEQ ID NO: 601 - DNA, 43 bp, Artificial Sequence
  source: /note="Description of Artificial Sequence: Synthetic oligonucleotide"
atggaggagttggcagatgctctaaatgtactgccatgggaag

SEQ ID NO: 602 - DNA, 45 bp, Artificial Sequence
  source: /note="Description of Artificial Sequence: Synthetic oligonucleotide"
atggaggagttggcagatgctcttctaatgtactgccatgggaag

SEQ ID NO: 603 - DNA, 44 bp, Artificial Sequence
  source: /note="Description of Artificial Sequence: Synthetic oligonucleotide"
atggaggagttggcagatgccctctaatgtactgccatgggaag

SEQ ID NO: 604 - DNA, 40 bp, Artificial Sequence
  source: /note="Description of Artificial Sequence: Synthetic oligonucleotide"
atggaggagttggcagataatgtactgccatgggaagaag

SEQ ID NO: 605 - DNA, 24 bp, Artificial Sequence
  source: /note="Description of Artificial Sequence: Synthetic oligonucleotide"
atggcgtactgccatgggaagaag

SEQ ID NO: 606 - DNA, 46 bp, Artificial Sequence
  source: /note="Description of Artificial Sequence: Synthetic oligonucleotide"
atggaggagttggcagatgcttctaatgtactgccatgggaagaag

SEQ ID NO: 607 - DNA, 32 bp, Artificial Sequence
  source: /note="Description of Artificial Sequence: Synthetic oligonucleotide"
atggaggagttggcatctgccatgggaagaag

SEQ ID NO: 608 - DNA, 42 bp, Artificial Sequence
  source: /note="Description of Artificial Sequence: Synthetic oligonucleotide"
atggaggagttggcagatgcaatgtactgccatgggaagaag

SEQ ID NO: 609 - DNA, 124 bp, Artificial Sequence
  source: /note="Description of Artificial Sequence: Synthetic polynucleotide"
atggaggagttggcagatgccaaactgaaaaacaaatcaaagcactcttattgagtgctggcgatccccgacgccacgggccgaaacccttatcatagaaactctaatgtactgccatgggaag

SEQ ID NO: 610 - DNA, 84 bp, Artificial Sequence
  source: /note="Description of Artificial Sequence: Synthetic oligonucleotide"
atggaggagttggcagatgctgcttatatagacctcccaccgtacacgcctaccgcccattttctaatgtactgccatgggaag

SEQ ID NO: 611 - DNA, 34 bp, Artificial Sequence
  source: /note="Description of Artificial Sequence: Synthetic oligonucleotide"
atggaggagttgtctaatgtactgccatgggaag

SEQ ID NO: 612 - DNA, 16 bp, Artificial Sequence
  source: /note="Description of Artificial Sequence: Synthetic oligonucleotide"
ctgccatgggaagaag

SEQ ID NO: 613 - DNA, 90 bp, Artificial Sequence
  source: /note="Description of Artificial Sequence: Synthetic oligonucleotide"
atggaggagttggcagatgcgcggctgttcctgtacagaaccgtgggcgagatgtggatcaaggatgctctaatgtactgccatgggaag

SEQ ID NO: 614 - DNA, 41 bp, Artificial Sequence
  source: /note="Description of Artificial Sequence: Synthetic oligonucleotide"
atggaggagttggcagatgcctaatgtactgccatgggaag

SEQ ID NO: 615 - DNA, 97 bp, Artificial Sequence
  source: /note="Description of Artificial Sequence: Synthetic oligonucleotide"
atggaggagttggcagatgctgtcatgatctttttccgctcgtcgtgggacttgctcagttctctggccagctcgtctaatgtactgccatgggaag

SEQ ID NO: 616 - DNA, 41 bp, Artificial Sequence
  source: /note="Description of Artificial Sequence: Synthetic oligonucleotide"
atggaggagttggcagatgctctatgtactgccatgggaag

SEQ ID NO: 617 - DNA, 32 bp, Artificial Sequence
  source: /note="Description of Artificial Sequence: Synthetic oligonucleotide"
cagggacagtgcgcatctccctggtcaccaag

SEQ ID NO: 618 - DNA, 17 bp, Artificial Sequence
  source: /note="Description of Artificial Sequence: Synthetic oligonucleotide"
cagggacagtcaccaag

SEQ ID NO: 619 - DNA, 31 bp, Artificial Sequence
  source: /note="Description of Artificial Sequence: Synthetic oligonucleotide"
cagggacagtgcgcatctcctggtcaccaag

SEQ ID NO: 620 - DNA, 30 bp, Artificial Sequence
  source: /note="Description of Artificial Sequence: Synthetic oligonucleotide"
cagggacagtgcgcatctctggtcaccaag

SEQ ID NO: 621 - DNA, 33 bp, Artificial Sequence
  source: /note="Description of Artificial Sequence: Synthetic oligonucleotide"
cagggacagtgcgcatctcctctggtcaccaag

SEQ ID NO: 622 - DNA, 29 bp, Artificial Sequence
  source: /note="Description of Artificial Sequence: Synthetic oligonucleotide"
cagggacagtgcgcatcctggtcaccaag

SEQ ID NO: 623 - DNA, 17 bp, Artificial Sequence
  source: /note="Description of Artificial Sequence: Synthetic oligonucleotide"
cagggacggtcaccaag

SEQ ID NO: 624 - DNA, 31 bp, Artificial Sequence
  source: /note="Description of Artificial Sequence: Synthetic oligonucleotide"
cggggacagggcgcatctcctggtcaccaag

SEQ ID NO: 625 - DNA, 32 bp, Artificial Sequence
  source: /note="Description of Artificial Sequence: Synthetic oligonucleotide"
cgacctgaatgctgtgcggctctgcttccagg

SEQ ID NO: 626 - DNA, 33 bp, Artificial Sequence
  source: /note="Description of Artificial Sequence: Synthetic oligonucleotide"
cgacctgaatgctgtgcggcatctgcttccagg

SEQ ID NO: 627 - DNA, 33 bp, Artificial Sequence
  source: /note="Description of Artificial Sequence: Synthetic oligonucleotide"
cgacctgaatgctgtgcggcttctgcttccagg

SEQ ID NO: 628 - DNA, 28 bp, Artificial Sequence
  source: /note="Description of Artificial Sequence: Synthetic oligonucleotide"
cgacctgaatgctgtgtctgcttccagg

SEQ ID NO: 629 - DNA, 33 bp, Artificial Sequence
  source: /note="Description of Artificial Sequence: Synthetic oligonucleotide"
cgacctgcatgctgtgcggcatctgcttccagg

SEQ ID NO: 630 - DNA, 33 bp, Artificial Sequence
  source: /note="Description of Artificial Sequence: Synthetic oligonucleotide"
cgacctgcatgctgtgcggcttctgcttccagg

SEQ ID NO: 631 - DNA, 28 bp, Artificial Sequence
  source: /note="Description of Artificial Sequence: Synthetic oligonucleotide"
cgacctgcatgctgtgtctgcttccagg

SEQ ID NO: 632 - DNA, 33 bp, Artificial Sequence
  source: /note="Description of Artificial Sequence: Synthetic oligonucleotide"
cgacctgaatgctgtgcgacatctgcttccagg

SEQ ID NO: 633 - DNA, 32 bp, Artificial Sequence
  source: /note="Description of Artificial Sequence: Synthetic oligonucleotide"
tggggactacgacctgaatgctgtgcggctct

SEQ ID NO: 634 - DNA, 27 bp, Artificial Sequence
  source: /note="Description of Artificial Sequence: Synthetic oligonucleotide"
tggggactacgaatgctgtgcggctct

SEQ ID NO: 635 - DNA, 66 bp, Artificial Sequence
  source: /note="Description of Artificial Sequence: Synthetic oligonucleotide"
tggggactacgagcaggcagaagtatgcaaagcatgcatctcaattcctgaatgctgtgcggctct

SEQ ID NO: 636 - DNA, 72 bp, Artificial Sequence
  source: /note="Description of Artificial Sequence: Synthetic oligonucleotide"
tggggactacgaagaaggcgatagaaggccatgcgctgcgaatcgggagcggcctgaatgctgtgcggctct

SEQ ID NO: 637 - DNA, 99 bp, Artificial Sequence
  source: /note="Description of Artificial Sequence: Synthetic oligonucleotide"
tggggactacgatgactcgctgcgctcggtcgttcggctgcggcgagcggtatcagctcactcaaaggcggtaatacggcctgaatgctgtgcggctct

SEQ ID NO: 638 - DNA, 14 bp, Artificial Sequence
  source: /note="Description of Artificial Sequence: Synthetic oligonucleotide"
tggggtgcggctct

SEQ ID NO: 639 - DNA, 27 bp, Artificial Sequence
  source: /note="Description of Artificial Sequence: Synthetic oligonucleotide"
tggggactacgactgctgtgcggctct

SEQ ID NO: 640 - DNA, 39 bp, Artificial Sequence; identical to SEQ ID NO: 579
  source: /note="Description of Artificial Sequence: Synthetic oligonucleotide"

SEQ ID NO: 641 - DNA, 35 bp, Artificial Sequence; identical to SEQ ID NO: 580
  source: /note="Description of Artificial Sequence: Synthetic oligonucleotide"

SEQ ID NO: 642 - DNA, 36 bp, Artificial Sequence; identical to SEQ ID NO: 581
  source: /note="Description of Artificial Sequence: Synthetic oligonucleotide"

SEQ ID NO: 643 - DNA, 25 bp, Artificial Sequence
  source: /note="Description of Artificial Sequence: Synthetic oligonucleotide"
cgacctgaatgctgcttccaggtga

SEQ ID NO: 644 - DNA, 28 bp, Artificial Sequence
  source: /note="Description of Artificial Sequence: Synthetic oligonucleotide"
cgacctgaatgcttctgcttccaggtga

SEQ ID NO: 645 - DNA, 22 bp, Artificial Sequence
  source: /note="Description of Artificial Sequence: Synthetic oligonucleotide"
cgacctgaatgcttccaggtga

SEQ ID NO: 646 - protein, 4 aa, Homo sapiens
EEQL

SEQ ID NO: 647 - protein, 6 aa, Homo sapiens
AEVSQA

SEQ ID NO: 648 - protein, 4 aa, Mus musculus
GEQL

SEQ ID NO: 649 - protein, 6 aa, Mus musculus
AEVSKA

SEQ ID NO: 650 - protein, 4 aa, Artificial Sequence
  source: /note="Description of Artificial Sequence: Synthetic peptide"
GEQL

SEQ ID NO: 651 - protein, 6 aa, Artificial Sequence
  source: /note="Description of Artificial Sequence: Synthetic peptide"
AEVSQA